European Patent Application EP 4 582 146 A2, published July 9, 2025. Title: ENHANCED CHIMERIC ANTIGEN RECEPTORS AND USE THEREOF. Applicant: Board of Regents, The University of Texas System. The sequence listing filed with the application follows.

SEQUENCE LISTING (64 sequences)

SEQ ID NO: 1 - DNA, 1062 bp, Homo sapiens
  source 1..1062: mol_type = other DNA
ctggaagagaagaaaggcaattacgtcgtgaccgaccacggcagctgtgtgcgggcttgtggcgccgatagctacgagatggaagaggacggcgtgcggaagtgcaagaagtgcgagggcccctgcagaaaagtgtgcaacggcatcggcatcggagagttcaaggatagcctgagcatcaacgccaccaacatcaagcacttcaagaactgcaccagcatcagcggcgacctgcacatcctgcccgtggcctttagaggcgacagcttcacccacacccccccactggatccccaggaactggacatcctgaaaaccgtgaaagagatcacaggctttctgctgattcaggcctggcccgagaaccggacagacctgcacgccttcgagaacctggaaatcatcagaggccggaccaagcagcacggccagttttctctggccgtggtgtccctgaacatcaccagcctgggcctgcggagcctgaaagaaatcagcgacggcgacgtgatcatctccggcaacaagaacctgtgctacgccaacaccatcaattggaagaagctgttcggcacctccggccagaaaacaaagatcatctctaaccggggcgagaacagctgcaaagccaccggacaagtgtgccacgccctgtgtagccctgagggctgttggggacccgagcccagagattgcgtgtcctgccggaatgtgtccagaggccgcgagtgcgtggacaagtgcaacctgctggaaggcgagccccgcgagtttgtggaaaacagcgagtgcatccagtgccaccccgagtgtctgccccaggccatgaacattacctgcaccggcagaggccccgacaactgtatccagtgcgcccactacatcgacggcccccactgcgtgaaaacctgtccagctggcgtgatgggagagaacaacaccctcgtgtggaagtacgccgacgccggccatgtgtgccacctgtgtcaccccaattgcacctacggctgtaccggccctggcctggaaggctgtcctaccaacggccccaagatcccttct

SEQ ID NO: 2 - protein, 354 aa, Homo sapiens
LEEKKGNYVVTDHGSCVRACGADSYEMEEDGVRKCKKCEGPCRKVCNGIGIGEFKDSLSINATNIKHFKNCTSISGDLHILPVAFRGDSFTHTPPLDPQELDILKTVKEITGFLLIQAWPENRTDLHAFENLEIIRGRTKQHGQFSLAVVSLNITSLGLRSLKEISDGDVIISGNKNLCYANTINWKKLFGTSGQKTKIISNRGENSCKATGQVCHALCSPEGCWGPEPRDCVSCRNVSRGRECVDKCNLLEGEPREFVENSECIQCHPECLPQAMNITCTGRGPDNCIQCAHYIDGPHCVKTCPAGVMGENNTLVWKYADAGHVCHLCHPNCTYGCTGPGLEGCPTNGPKIPS

SEQ ID NO: 3 - DNA, 801 bp, synthetic construct
  misc_feature 1..801: note = hCD19-scFv
  source 1..801: mol_type = other DNA
atggagttcggtttgagctggctctttcttgttgctatcctcaagggggtgcagtgttcaagggatatccagatgactcagagccctagctcccttagcgcgtccgtcggcgaccgggttacaattacttgtcgcgcatcacaagacataagtaaatacttgaactggtatcaacaaaagccaggaaaggttccaaaactcctcatctatcacacgagtagactccattccggggtccctgatcggttctcaggctctggttctggaactgacttcactctcacgatctctagtctgcaacctgaggatgtcgctacctattattgccaacagggaaacaccctcccttacacatttggccaaggtaccaaagttgagatcaagaggggctccacatctgggagcgggaaaccgggaagtggagaaggctcaaccaaaggtgaggtgcaacttgtagagagtggtggaggcctggttcagccgggagggtccctcagacttagttgcgcggcttctggcgtttcactgccggactacggggtcagttgggttaggcaggcgcctgggaaaggacttgagtggatcggcgtgatatggggtagtgaaacaacctactacaatagtgctcttaaatcaaaattcattatcagccgagacaatgctaagaactccctctatctccaaatgaatagtcttagagcagaagacacagccgtttattactgtgcccgccattattactatgggggcagctacgcaatggattattggggccaagggaccctggtcacggtatcaagc

SEQ ID NO: 4 - DNA, 324 bp, synthetic construct
  misc_feature 1..324: note = hCD19-scFv VL
  source 1..324: mol_type = other DNA
gatatccagatgactcagagccctagctcccttagcgcgtccgtcggcgaccgggttacaattacttgtcgcgcatcacaagacataagtaaatacttgaactggtatcaacaaaagccaggaaaggttccaaaactcctcatctatcacacgagtagactccattccggggtccctgatcggttctcaggctctggttctggaactgacttcactctcacgatctctagtctgcaacctgaggatgtcgctacctattattgccaacagggaaacaccctcccttacacatttggccaaggtaccaaagttgagatcaagagg

SEQ ID NO: 5 - DNA, 360 bp, synthetic construct
  misc_feature 1..360: note = hCD19-scFv VH
  source 1..360: mol_type = other DNA
gaggtgcaacttgtagagagtggtggaggcctggttcagccgggagggtccctcagacttagttgcgcggcttctggcgtttcactgccggactacggggtcagttgggttaggcaggcgcctgggaaaggacttgagtggatcggcgtgatatggggtagtgaaacaacctactacaatagtgctcttaaatcaaaattcattatcagccgagacaatgctaagaactccctctatctccaaatgaatagtcttagagcagaagacacagccgtttattactgtgcccgccattattactatgggggcagctacgcaatggattattggggccaagggaccctggtcacggtatcaagc

SEQ ID NO: 6 - protein, 267 aa, synthetic construct
  REGION 1..267: note = hCD19-scFv
MEFGLSWLFLVAILKGVQCSRDIQMTQSPSSLSASVGDRVTITCRASQDISKYLNWYQQKPGKVPKLLIYHTSRLHSGVPDRFSGSGSGTDFTLTISSLQPEDVATYYCQQGNTLPYTFGQGTKVEIKRGSTSGSGKPGSGEGSTKGEVQLVESGGGLVQPGGSLRLSCAASGVSLPDYGVSWVRQAPGKGLEWIGVIWGSETTYYNSALKSKFIISRDNAKNSLYLQMNSLRAEDTAVYYCARHYYYGGSYAMDYWGQGTLVTVSS

SEQ ID NO: 7 - protein, 108 aa, synthetic construct
  REGION 1..108: note = hCD19-scFv VL
DIQMTQSPSSLSASVGDRVTITCRASQDISKYLNWYQQKPGKVPKLLIYHTSRLHSGVPDRFSGSGSGTDFTLTISSLQPEDVATYYCQQGNTLPYTFGQGTKVEIKR

SEQ ID NO: 8 - protein, 120 aa, synthetic construct
  REGION 1..120: note = hCD19-scFv VH
EVQLVESGGGLVQPGGSLRLSCAASGVSLPDYGVSWVRQAPGKGLEWIGVIWGSETTYYNSALKSKFIISRDNAKNSLYLQMNSLRAEDTAVYYCARHYYYGGSYAMDYWGQGTLVTVSS

SEQ ID NO: 9 - DNA, 786 bp, synthetic construct
  misc_feature 1..786: note = hCD123-scFv
  source 1..786: mol_type = other DNA
atggaattcgggctttcatggttgttcctcgttgcgatacttaaaggcgttcagtgcagtagagacattcagatgacccaaagccctagtagcctctccgccagtgtgggtgaccgcgtgactattacgtgccgagcaagcaagagtattagcaaagatttggcatggtaccagcagaaaccaggcaaggtccctaagttgcttatatatagcgggtctacactccaatctggagtgccggatcgcttctcaggttccggatcaggaaccgatttcactcttacaatttcctctctgcaaccggaggacgtggcaacatactattgccagcagcataacaaatatccctatactttcggtcaaggtacaaaagtagaaataaaacgaggttccacctccgggagtgggaagcccggctccggcgaaggatccaccaaaggcgaggtacagctcgttgaaagcgggggcggtctcgtccaaccaggagggtctcttcgactttcttgtgctgcaagtgggtacacgtttacttcctattggatgaattgggttcggcaagcccccggtaaagggcttgaatggatagggaggatagacccctacgattctgagacgcattataatcagaaattcaaagataagttcataataagcagagacaatgcaaaaaatagtttgtacctccagatgaatagtcttcgggcagaagacacagcggtatattactgtgctcggggtaactgggatgattactggggtcagggaactctggttactgtgtctagc

SEQ ID NO: 10 - DNA, 324 bp, synthetic construct
  misc_feature 1..324: note = hCD123-scFv VL
  source 1..324: mol_type = other DNA
gacattcagatgacccaaagccctagtagcctctccgccagtgtgggtgaccgcgtgactattacgtgccgagcaagcaagagtattagcaaagatttggcatggtaccagcagaaaccaggcaaggtccctaagttgcttatatatagcgggtctacactccaatctggagtgccggatcgcttctcaggttccggatcaggaaccgatttcactcttacaatttcctctctgcaaccggaggacgtggcaacatactattgccagcagcataacaaatatccctatactttcggtcaaggtacaaaagtagaaataaaacga

SEQ ID NO: 11 - DNA, 345 bp, synthetic construct
  misc_feature 1..345: note = hCD123-scFv VH
  source 1..345: mol_type = other DNA
gaggtacagctcgttgaaagcgggggcggtctcgtccaaccaggagggtctcttcgactttcttgtgctgcaagtgggtacacgtttacttcctattggatgaattgggttcggcaagcccccggtaaagggcttgaatggatagggaggatagacccctacgattctgagacgcattataatcagaaattcaaagataagttcataataagcagagacaatgcaaaaaatagtttgtacctccagatgaatagtcttcgggcagaagacacagcggtatattactgtgctcggggtaactgggatgattactggggtcagggaactctggttactgtgtctagc

SEQ ID NO: 12 - protein, 262 aa, synthetic construct
  REGION 1..262: note = hCD123-scFv
MEFGLSWLFLVAILKGVQCSRDIQMTQSPSSLSASVGDRVTITCRASKSISKDLAWYQQKPGKVPKLLIYSGSTLQSGVPDRFSGSGSGTDFTLTISSLQPEDVATYYCQQHNKYPYTFGQGTKVEIKRGSTSGSGKPGSGEGSTKGEVQLVESGGGLVQPGGSLRLSCAASGYTFTSYWMNWVRQAPGKGLEWIGRIDPYDSETHYNQKFKDKFIISRDNAKNSLYLQMNSLRAEDTAVYYCARGNWDDYWGQGTLVTVSS

SEQ ID NO: 13 - protein, 108 aa, synthetic construct
  REGION 1..108: note = hCD123-scFv VL
DIQMTQSPSSLSASVGDRVTITCRASKSISKDLAWYQQKPGKVPKLLIYSGSTLQSGVPDRFSGSGSGTDFTLTISSLQPEDVATYYCQQHNKYPYTFGQGTKVEIKR

SEQ ID NO: 14 - protein, 115 aa, synthetic construct
  REGION 1..115: note = hCD123-scFv VH
EVQLVESGGGLVQPGGSLRLSCAASGYTFTSYWMNWVRQAPGKGLEWIGRIDPYDSETHYNQKFKDKFIISRDNAKNSLYLQMNSLRAEDTAVYYCARGNWDDYWGQGTLVTVSS

SEQ ID NO: 15 - DNA, 777 bp, synthetic construct
  misc_feature 1..777: note = hMeso-scFv
  source 1..777: mol_type = other DNA
atggagttcggcctttcttggctgtttttggtcgcaatattgaagggcgttcagtgttcaagggacatacagatgacgcagtcacctagctctctttcagcctctgtgggagaccgcgttacaattacgtgttctgcttctagttcagtgtcttacatgcattggtaccagcaaaaacccggcaaggttccaaagctccttatatacgatacgtccaaactggcttcaggcgtgccagacaggtttagtggatctgggagcggcactgacttcacacttacaatatccagtctgcaacccgaagatgttgcgacatactattgtcagcaatggagcggctatccgctcaccggacaggggacaaaagtggagataaagcggggctccaccagtggttccgggaagcctggtagtggtgagggttctacgaaaggcgaagtgcagttggtggagtctggtggcgggcttgttcaacccggtggttctctcaggcttagctgtgcagcctctgggtacacaatgaattgggtaaggcaagcgcctggaaagggccttgagtggatcggtttgataaccccatacaacggagcttcaagttacaaccaaaagttccgcgggaagtttattataagcagggataacgcaaagaacagcctctatcttcaaatgaactcactccgggctgaagacacagccgtctattattgtgcccgggggggctacgacggacgagggttcgattactggggtcagggcacactcgtgaccgtgtcaagc

SEQ ID NO: 16 - DNA, 318 bp, synthetic construct
  misc_feature 1..318: note = hMeso-scFv VL
  source 1..318: mol_type = other DNA
gacatacagatgacgcagtcacctagctctctttcagcctctgtgggagaccgcgttacaattacgtgttctgcttctagttcagtgtcttacatgcattggtaccagcaaaaacccggcaaggttccaaagctccttatatacgatacgtccaaactggcttcaggcgtgccagacaggtttagtggatctgggagcggcactgacttcacacttacaatatccagtctgcaacccgaagatgttgcgacatactattgtcagcaatggagcggctatccgctcaccggacaggggacaaaagtggagataaagcgg

SEQ ID NO: 17 - DNA, 342 bp, synthetic construct
  misc_feature 1..342: note = hMeso-scFv VH
  source 1..342: mol_type = other DNA
gaagtgcagttggtggagtctggtggcgggcttgttcaacccggtggttctctcaggcttagctgtgcagcctctgggtacacaatgaattgggtaaggcaagcgcctggaaagggccttgagtggatcggtttgataaccccatacaacggagcttcaagttacaaccaaaagttccgcgggaagtttattataagcagggataacgcaaagaacagcctctatcttcaaatgaactcactccgggctgaagacacagccgtctattattgtgcccgggggggctacgacggacgagggttcgattactggggtcagggcacactcgtgaccgtgtcaagc

SEQ ID NO: 18 - protein, 259 aa, synthetic construct
  REGION 1..259: note = hMeso-scFv
MEFGLSWLFLVAILKGVQCSRDIQMTQSPSSLSASVGDRVTITCSASSSVSYMHWYQQKPGKVPKLLIYDTSKLASGVPDRFSGSGSGTDFTLTISSLQPEDVATYYCQQWSGYPLTGQGTKVEIKRGSTSGSGKPGSGEGSTKGEVQLVESGGGLVQPGGSLRLSCAASGYTMNWVRQAPGKGLEWIGLITPYNGASSYNQKFRGKFIISRDNAKNSLYLQMNSLRAEDTAVYYCARGGYDGRGFDYWGQGTLVTVSS

SEQ ID NO: 19 - protein, 106 aa, synthetic construct
  REGION 1..106: note = hMeso-scFv VL
DIQMTQSPSSLSASVGDRVTITCSASSSVSYMHWYQQKPGKVPKLLIYDTSKLASGVPDRFSGSGSGTDFTLTISSLQPEDVATYYCQQWSGYPLTGQGTKVEIKR

SEQ ID NO: 20 - protein, 114 aa, synthetic construct
  REGION 1..114: note = hMeso-scFv VH
EVQLVESGGGLVQPGGSLRLSCAASGYTMNWVRQAPGKGLEWIGLITPYNGASSYNQKFRGKFIISRDNAKNSLYLQMNSLRAEDTAVYYCARGGYDGRGFDYWGQGTLVTVSS

SEQ ID NO: 21 - DNA, 798 bp, synthetic construct
  misc_feature 1..798: note = hROR1-scFv
  source 1..798: mol_type = other DNA
atggagttcggacttagttggcttttcctcgtcgccatactcaaaggtgtacaatgctcacgcgatatacaaatgacgcagagtccatcctcactgtctgcctcagtaggcgacagggtcacaataacctgtaaagcaagcccggatatcaactcttacctcagttggttccaacagaaaccaggaaaggtgccgaagttgttgatttaccgcgcaaaccgcctcgttgacggcgtgccagataggttttctggcagcgggagcggcactgactttacgctcactatatcaagcctgcagccggaggacgtagcaacttactattgcctccaatacgacgaattcccttacacgttcgggcaaggaactaaagttgaaataaaaagaggaagcacaagtggttctggaaaacccggttccggtgagggcagtaccaaaggagaggtgcagttggtagagtctggtgggggtttggtgcaacccggagggtctctgaggttgtcttgcgcggcatccggctttactttttcctcatatgcgatgtcatgggtacgacaggccccaggcaagggactggagtggatcgcatctatttcacgaggagggacgacatattacccggattcagtgaagggcaaattcataatttcacgcgataacgccaagaactccctctacctgcaaatgaacagtcttagagcggaagatacggctgtgtattactgtgcgcgatatgactacgatggatattacgcgatggattattggggacaaggtacactggtaaccgtttccagc

SEQ ID NO: 22 - DNA, 324 bp, synthetic construct
  misc_feature 1..324: note = hROR1-scFv VL
  source 1..324: mol_type = other DNA
gatatacaaatgacgcagagtccatcctcactgtctgcctcagtaggcgacagggtcacaataacctgtaaagcaagcccggatatcaactcttacctcagttggttccaacagaaaccaggaaaggtgccgaagttgttgatttaccgcgcaaaccgcctcgttgacggcgtgccagataggttttctggcagcgggagcggcactgactttacgctcactatatcaagcctgcagccggaggacgtagcaacttactattgcctccaatacgacgaattcccttacacgttcgggcaaggaactaaagttgaaataaaaaga

SEQ ID NO: 23 - DNA, 357 bp, synthetic construct
  misc_feature 1..357: note = hROR1-scFv VH
  source 1..357: mol_type = other DNA
gaggtgcagttggtagagtctggtgggggtttggtgcaacccggagggtctctgaggttgtcttgcgcggcatccggctttactttttcctcatatgcgatgtcatgggtacgacaggccccaggcaagggactggagtggatcgcatctatttcacgaggagggacgacatattacccggattcagtgaagggcaaattcataatttcacgcgataacgccaagaactccctctacctgcaaatgaacagtcttagagcggaagatacggctgtgtattactgtgcgcgatatgactacgatggatattacgcgatggattattggggacaaggtacactggtaaccgtttccagc

SEQ ID NO: 24 - protein, 266 aa, synthetic construct
  REGION 1..266: note = hROR1-scFv
MEFGLSWLFLVAILKGVQCSRDIQMTQSPSSLSASVGDRVTITCKASPDINSYLSWFQQKPGKVPKLLIYRANRLVDGVPDRFSGSGSGTDFTLTISSLQPEDVATYYCLQYDEFPYTFGQGTKVEIKRGSTSGSGKPGSGEGSTKGEVQLVESGGGLVQPGGSLRLSCAASGFTFSSYAMSWVRQAPGKGLEWIASISRGGTTYYPDSVKGKFIISRDNAKNSLYLQMNSLRAEDTAVYYCARYDYDGYYAMDYWGQGTLVTVSS

SEQ ID NO: 25 - protein, 108 aa, synthetic construct
  REGION 1..108: note = hROR1-scFv VL
DIQMTQSPSSLSASVGDRVTITCKASPDINSYLSWFQQKPGKVPKLLIYRANRLVDGVPDRFSGSGSGTDFTLTISSLQPEDVATYYCLQYDEFPYTFGQGTKVEIKR

SEQ ID NO: 26 - protein, 119 aa, synthetic construct
  REGION 1..119: note = hROR1-scFv VH
EVQLVESGGGLVQPGGSLRLSCAASGFTFSSYAMSWVRQAPGKGLEWIASISRGGTTYYPDSVKGKFIISRDNAKNSLYLQMNSLRAEDTAVYYCARYDYDGYYAMDYWGQGTLVTVSS

SEQ ID NO: 27 - DNA, 792 bp, synthetic construct
  misc_feature 1..792: note = hCD5-scFv
  source 1..792: mol_type = other DNA
atggagttcggtctcagttggctgtttttggttgctatcttgaagggcgtccaatgcagccgggacatccagatgacccagtctccctctagcatgtcagcgagtcttggtgatcgagtgacgattacctgcagagcctctcaagatataaacagctatctttcatggttccaacagaagccggggaagtccccaaaaactctcatatacagggcgaatcgactcgtagacggtgtgccttcaaggttttccgggagtggtagtggcacagattacacacttacaatctcttcattgcagtatgaggatttcgggatctactactgtcaacagtacgacgaatccccatggacgtttgggggcgggaccaaacttgagataaaagggagcacatctggaagtggtaaacctgggtcaggggagggttccacaaaaggacaaattcaacttgtccaaagcggtcctggtcttaagaagcctggagggtctgtcaggataagttgtgcggcatccggctacaccttcaccaactatgggatgaactgggtgaaacaagcgcctgggaaaggtcttcgatggatgggctggattaatacccacactggagagcccacttacgctgatgatttcaaaggacgatttaccttctccttggatacttccaagagtaccgcgtacttgcaaatcaacagtctccgggctgaagacacggccacatacttctgtacgcggagagggtatgactggtattttgatgtgtggggtcagggaacaaccgtgactgtttcaagc

SEQ ID NO: 28 - DNA, 321 bp, synthetic construct
  misc_feature 1..321: note = hCD5-scFv VL
  source 1..321: mol_type = other DNA
gacatccagatgacccagtctccctctagcatgtcagcgagtcttggtgatcgagtgacgattacctgcagagcctctcaagatataaacagctatctttcatggttccaacagaagccggggaagtccccaaaaactctcatatacagggcgaatcgactcgtagacggtgtgccttcaaggttttccgggagtggtagtggcacagattacacacttacaatctcttcattgcagtatgaggatttcgggatctactactgtcaacagtacgacgaatccccatggacgtttgggggcgggaccaaacttgagataaaa

SEQ ID NO: 29 - DNA, 354 bp, synthetic construct
  misc_feature 1..354: note = hCD5-scFv VH
  source 1..354: mol_type = other DNA
caaattcaacttgtccaaagcggtcctggtcttaagaagcctggagggtctgtcaggataagttgtgcggcatccggctacaccttcaccaactatgggatgaactgggtgaaacaagcgcctgggaaaggtcttcgatggatgggctggattaatacccacactggagagcccacttacgctgatgatttcaaaggacgatttaccttctccttggatacttccaagagtaccgcgtacttgcaaatcaacagtctccgggctgaagacacggccacatacttctgtacgcggagagggtatgactggtattttgatgtgtggggtcagggaacaaccgtgactgtttcaagc

SEQ ID NO: 30 - protein, 264 aa, synthetic construct
  REGION 1..264: note = hCD5-scFv
MEFGLSWLFLVAILKGVQCSRDIQMTQSPSSMSASLGDRVTITCRASQDINSYLSWFQQKPGKSPKTLIYRANRLVDGVPSRFSGSGSGTDYTLTISSLQYEDFGIYYCQQYDESPWTFGGGTKLEIKGSTSGSGKPGSGEGSTKGQIQLVQSGPGLKKPGGSVRISCAASGYTFTNYGMNWVKQAPGKGLRWMGWINTHTGEPTYADDFKGRFTFSLDTSKSTAYLQINSLRAEDTATYFCTRRGYDWYFDVWGQGTTVTVSS

SEQ ID NO: 31 - protein, 107 aa, synthetic construct
  REGION 1..107: note = hCD5-scFv VL
DIQMTQSPSSMSASLGDRVTITCRASQDINSYLSWFQQKPGKSPKTLIYRANRLVDGVPSRFSGSGSGTDYTLTISSLQYEDFGIYYCQQYDESPWTFGGGTKLEIK

SEQ ID NO: 32 - protein, 118 aa, synthetic construct
  REGION 1..118: note = hCD5-scFv VH
QIQLVQSGPGLKKPGGSVRISCAASGYTFTNYGMNWVKQAPGKGLRWMGWINTHTGEPTYADDFKGRFTFSLDTSKSTAYLQINSLRAEDTATYFCTRRGYDWYFDVWGQGTTVTVSS

SEQ ID NO: 33 - DNA, 10253 bp, synthetic construct
  misc_feature 1..10253: note = hCD19-CAR
  source 1..10253: mol_type = other DNA
aatgaaagaccccacctgtaggtttggcaagctagcttaagtaacgccattttgcaaggcatggaaaaatacataactgagaatagaaaagttcagatcaaggtcaggaacagatggaacagctgaatatgggccaaacaggatatctgtggtaagcagttcctgccccggctcagggccaagaacagatggaacagctgaatatgggccaaacaggatatctgtggtaagcagttcctgccccggctcagggccaagaacagatggtccccagatgcggtccagccctcagcagtttctagagaaccatcagatgtttccagggtgccccaaggacctgaaatgaccctgtgccttatttgaactaaccaatcagttcgcttctcgcttctgttcgcgcgcttatgctccccgagctcaataaaagagcccacaacccctcactcggggcgccagtcctccgattgactgagtcgcccgggtacccgtgtatccaataaaccctcttgcagttgcatccgacttgtggtctcgctgttccttgggagggtctcctctgagtgattgactacccgtcagcgggggtctttcatttgggggctcgtccgggatcgggagacccctgcccagggaccaccgacccaccaccgggaggtaagctggccagcaacttatctgtgtctgtccgattgtctagtgtctatgactgattttatgcgcctgcgtcggtactagttagctaactagctctgtatctggcggacccgtggtggaactgacgagttcggaacacccggccgcaaccctgggagacgtcccagggacttcgggggccgtttttgtggcccgacctgagtcctaaaatcccgatcgtttaggactctttggtgcaccccccttagaggagggatatgtggttctggtaggagacgagaacctaaaacagttcccgcctccgtctgaatttttgctttcggtttgggaccgaagccgcgccgcgcgtcttgtctgctgcagcatcgttctgtgttgtctctgtctgactgtgtttctgtatttgtctgaaaatatgggcccgggctagcctgttaccactcccttaagtttgaccttaggtcactggaaagatgtcgagcggatcgctcacaaccagtcggtagatgtcaagaagagacgttgggttaccttctgctctgcagaatggccaacctttaacgtcggatggccgcgagacggcacctttaaccgagacctcatcacccaggttaagatcaaggtcttttcacctggcccgcatggacacccagaccaggtggggtacatcgtgacctgggaagccttggcttttgacccccctccctgggtcaagccctttgtacaccctaagcctccgcctcctcttcctccatccgccccgtctctcccccttgaacctcctcgttcgaccccgcctcgatcctccctttatccagccctcactccttctctaggcgcccccatatggccatatgagatcttatatggggcacccccgccccttgtaaacttccctgaccctgacatgacaagagttactaacagcccctctctccaagctcacttacaggctctctacttagtccagcacgaagtctggagacctctggcggcagcctaccaagaacaactggaccgaccggtggtacctcacccttaccgagtcggcgacacagtgtgggtccgccgacaccagactaagaacctagaacctcgctggaaaggaccttacacagtcctgctgaccacccccaccgccctcaaagtagacggcatcgcagcttggatacacgccgcccacgtgaaggctgccgaccccgggggtggaccatcctctagactgccatgctcgagggagtgcaggtggaaaccatctccccaggagacgggcgcaccttccccaagcgcggccagacctgcgtggtgcactacaccgggatgcttgaagatggaaagaaagttgattcctcccgggacagaaacaagccctttaagtttatgctaggcaagcaggaggtgatccgaggctgggaagaaggggttgcccagatgagtgtgggtcagagagccaaactgactatatctccagattatgcctatggtgccactgggcacccaggcatcatcccaccacatgccactctcgtcttcgatgtggagcttctaaaactggaatctggcggtggatccggagtcgacggatttggtgatgtcggtgctcttgagagtttgaggggaaatgcagatttggcttacatcctgagcatggagccctgtggccactgcctcattatcaacaatgtgaacttctgccgtgagtccgggctccgcacccgcactggctccaacatcgactgtgagaagttgcggcgtcgcttctcctcgctgcatttcatggtggaggtgaagggcgacctgactgccaagaaaatggtgctggctttgctggagctggcgcagcaggaccacggtgctctggactgctgcgtggtggtcattctctctcacggctgtcaggccagccacctgcagttcccaggggctgtctacggcacagatggatgccctgtgtcggtcgagaagattgtgaacatcttcaatgggaccagctgccccagcctgggagggaagcccaagctctttttcatccaggcctgtggtggggagcagaaagaccatgggtttgaggtggcctccacttcccctgaagacgagtcccctggcagtaaccccgagccagatgccaccccgttccaggaaggtttgaggaccttcgaccagctggacgccatatctagtttgcccacacccagtgacatctttgtgtcctactctactttcccaggttttgtttcctggagggaccccaagagtggctcctggtacgttgagaccctggacgacatctttgagcagtgggctcactctgaagacctgcagtccctcctgcttagggtcgctaatgctgtttcggtgaaagggatttataaacagatgcctggttgctttaatttcctccggaaaaaacttttctttaaaacatcagctagcagagccgagggcaggggaagtcttctaacatgcggggacgtggaggaaaatcccgggcccatggagttcggtttgagctggctctttcttgttgctatcctcaagggggtgcagtgttcaagggatatccagatgactcagagccctagctcccttagcgcgtccgtcggcgaccgggttacaattacttgtcgcgcatcacaagacataagtaaatacttgaactggtatcaacaaaagccaggaaaggttccaaaactcctcatctatcacacgagtagactccattccggggtccctgatcggttctcaggctctggttctggaactgacttcactctcacgatctctagtctgcaacctgaggatgtcgctacctattattgccaacagggaaacaccctcccttacacatttggccaaggtaccaaagttgagatcaagaggggctccacatctgggagcgggaaaccgggaagtggagaaggctcaaccaaaggtgaggtgcaacttgtagagagtggtggaggcctggttcagccgggagggtccctcagacttagttgcgcggcttctggcgtttcactgccggactacggggtcagttgggttaggcaggcgcctgggaaaggacttgagtggatcggcgtgatatggggtagtgaaacaacctactacaatagtgctcttaaatcaaaattcattatcagccgagacaatgctaagaactccctctatctccaaatgaatagtcttagagcagaagacacagccgtttattactgtgcccgccattattactatgggggcagctacgcaatggattattggggccaagggaccctggtcacggtatcaagctacgtcaccgtctcttcacaggatcccgccgagcccaaatctcctgacaaaactcacacatgcccaccgtgcccagcacctgaactcctggggggaccgtcagtcttcctcttccccccaaaacccaaggacaccctcatgatctcccggacccctgaggtcacatgcgtggtggtggacgtgagccacgaagaccctgaggtcaagttcaactggtacgtggacggcgtggaggtgcataatgccaagacaaagccgcgggaggagcagtacaacagcacgtaccgtgtggtcagcgtcctcaccgtcctgcaccaggactggctgaatggcaaggagtacaagtgcaaggtctccaacaaagccctcccagcccccatcgagaaaaccatctccaaagccaaagggcagccccgagaaccacaggtgtacaccctgcccccatcccgggatgagctgaccaagaaccaggtcagcctgacctgcctggtcaaaggcttctatcccagcgacatcgccgtggagtgggagagcaatgggcaaccggagaacaactacaagaccacgcctcccgtgctggactccgacggctccttcttcctctacagcaagctcaccgtggacaagagcaggtggcagcaggggaacgtcttctcatgctccgtgatgcatgaggctctgcacaaccactacacgcagaagagcctctccctgtctccgggtaaaaaagatcccaaattttgggtgctggtggtggttggtggagtcctggcttgctatagcttgctagtaacagtggcctttattattttctgggtgaggagtaagaggagcaggctcctgcacagtgactacatgaacatgactccccgccgccccgggcccacccgcaagcattaccagccctatgccccaccacgcgacttcgcagcctatcgctccagagtgaagttcagcaggagcgcagacgcccccgcgtaccagcagggccagaaccagctctataacgagctcaatctaggacgaagagaggagtacgatgttttggacaagagacgtggccgggaccctgagatggggggaaagccgagaaggaagaaccctcaggaaggcctgtacaatgaactgcagaaagataagatggcggaggcctacagtgagattgggatgaaaggcgagcgccggaggggcaaggggcacgatggcctttaccagggtctcagtacagccaccaaggacacctacgacgcccttcacatgcaggccctgccccctcgcggaccgcagtgtactaattatgctctcttgaaattggctggagatgttgagagcaatcccgggcccatgcggatcagcaagccccacctgcggagcatcagcatccagtgctacctgtgcctgctgctgaacagccacttcctgaccgaggccggcatccacgtgttcatcctgggctgcttcagcgccggactgcccaagaccgaggccaactgggtgaacgtgatcagcgacctgaagaagatcgaggacctgatccagagcatgcacatcgacgccaccctgtacaccgagagcgacgtgcaccccagctgcaaggtgaccgccatgaagtgctttctgctggaactgcaggtgatcagcctggaaagcggcgacgccagcatccacgacaccgtggagaacctgatcatcctggccaacaacagcctgagcagcaacggcaacgtgaccgagagcggctgcaaagagtgcgaggaactggaagagaagaacatcaaagagtttctgcagagcttcgtgcacatcgtgcagatgttcatcaacaccagctgacgcgtcatcatcgatccggattagtccaatttgttaaagacaggatatcagtggtccaggctctagttttgactcaacaatatcaccagctgaagcctatagagtacgagccatagataaaataaaagattttatttagtctccagaaaaaggggggaatgaaagaccccacctgtaggtttggcaagctagcttaagtaacgccattttgcaaggcatggaaaaatacataactgagaatagagaagttcagatcaaggtcaggaacagatggaacagctgaatatgggccaaacaggatatctgtggtaagcagttcctgccccggctcagggccaagaacagatggaacagctgaatatgggccaaacaggatatctgtggtaagcagttcctgccccggctcagggccaagaacagatggtccccagatgcggtccagccctcagcagtttctagagaaccatcagatgtttccagggtgccccaaggacctgaaatgaccctgtgccttatttgaactaaccaatcagttcgcttctcgcttctgttcgcgcgcttctgctccccgagctcaataaaagagcccacaacccctcactcggggcgccagtcctccgattgactgagtcgcccgggtacccgtgtatccaataaaccctcttgcagttgcatccgacttgtggtctcgctgttccttgggagggtctcctctgagtgattgactacccgtcagcgggggtctttcacacatgcagcatgtatcaaaattaatttggttttttttcttaagtatttacattaaatggccatagtacttaaagttacattggcttccttgaaataaacatggagtattcagaatgtgtcataaatatttctaattttaagatagtatctccattggctttctactttttcttttatttttttttgtcctctgtcttccatttgttgttgttgttgtttgtttgtttgtttgttggttggttggttaatttttttttaaagatcctacactatagttcaagctagactattagctactctgtaacccagggtgaccttgaagtcatgggtagcctgctgttttagccttcccacatctaagattacaggtatgagctatcatttttggtatattgattgattgattgattgatgtgtgtgtgtgtgattgtgtttgtgtgtgtgactgtgaaaatgtgtgtatgggtgtgtgtgaatgtgtgtatgtatgtgtgtgtgtgagtgtgtgtgtgtgtgtgtgcatgtgtgtgtgtgtgactgtgtctatgtgtatgactgtgtgtgtgtgtgtgtgtgtgtgtgtgtgtgtgtgtgtgtgtgtgttgtgaaaaaatattctatggtagtgagagccaacgctccggctcaggtgtcaggttggtttttgagacagagtctttcacttagcttggaattcactggccgtcgttttacaacgtcgtgactgggaaaaccctggcgttacccaacttaatcgccttgcagcacatccccctttcgccagctggcgtaatagcgaagaggcccgcaccgatcgcccttcccaacagttgcgcagcctgaatggcgaatggcgcctgatgcggtattttctccttacgcatctgtgcggtatttcacaccgcatatggtgcactctcagtacaatctgctctgatgccgcatagttaagccagccccgacacccgccaacacccgctgacgcgccctgacgggcttgtctgctcccggcatccgcttacagacaagctgtgaccgtctccgggagctgcatgtgtcagaggttttcaccgtcatcaccgaaacgcgcgagacgaaagggcctcgtgatacgcctatttttataggttaatgtcatgataataatggtttcttagacgtcaggtggcacttttcggggaaatgtgcgcggaacccctatttgtttatttttctaaatacattcaaatatgtatccgctcatgagacaataaccctgataaatgcttcaataatattgaaaaaggaagagtatgagtattcaacatttccgtgtcgcccttattcccttttttgcggcattttgccttcctgtttttgctcacccagaaacgctggtgaaagtaaaagatgctgaagatcagttgggtgcacgagtgggttacatcgaactggatctcaacagcggtaagatccttgagagttttcgccccgaagaacgttttccaatgatgagcacttttaaagttctgctatgtggcgcggtattatcccgtattgacgccgggcaagagcaactcggtcgccgcatacactattctcagaatgacttggttgagtactcaccagtcacagaaaagcatcttacggatggcatgacagtaagagaattatgcagtgctgccataaccatgagtgataacactgcggccaacttacttctgacaacgatcggaggaccgaaggagctaaccgcttttttgcacaacatgggggatcatgtaactcgccttgatcgttgggaaccggagctgaatgaagccataccaaacgacgagcgtgacaccacgatgcctgtagcaatggcaacaacgttgcgcaaactattaactggcgaactacttactctagcttcccggcaacaattaatagactggatggaggcggataaagttgcaggaccacttctgcgctcggcccttccggctggctggtttattgctgataaatctggagccggtgagcgtgggtctcgcggtatcattgcagcactggggccagatggtaagccctcccgtatcgtagttatctacacgacggggagtcaggcaactatggatgaacgaaatagacagatcgctgagataggtgcctcactgattaagcattggtaactgtcagaccaagtttactcatatatactttagattgatttaaaacttcatttttaatttaaaaggatctaggtgaagatcctttttgataatctcatgaccaaaatcccttaacgtgagttttcgttccactgagcgtcagaccccgtagaaaagatcaaaggatcttcttgagatcctttttttctgcgcgtaatctgctgcttgcaaacaaaaaaaccaccgctaccagcggtggtttgtttgccggatcaagagctaccaactctttttccgaaggtaactggcttcagcagagcgcagataccaaatactgttcttctagtgtagccgtagttaggccaccacttcaagaactctgtagcaccgcctacatacctcgctctgctaatcctgttaccagtggctgctgccagtggcgataagtcgtgtcttaccgggttggactcaagacgatagttaccggataaggcgcagcggtcgggctgaacggggggttcgtgcacacagcccagcttggagcgaacgacctacaccgaactgagatacctacagcgtgagctatgagaaagcgccacgcttcccgaagggagaaaggcggacaggtatccggtaagcggcagggtcggaacaggagagcgcacgagggagcttccagggggaaacgcctggtatctttatagtcctgtcgggtttcgccacctctgacttgagcgtcgatttttgtgatgctcgtcaggggggcggagcctatggaaaaacgccagcaacgcggcctttttacggttcctggccttttgctggccttttgctcacatgttctttcctgcgttatcccctgattctgtggataaccgtattaccgcctttgagtgagctgataccgctcgccgcagccgaacgaccgagcgcagcgagtcagtgagcgaggaagcggaagagcgcccaatacgcaaaccgcctctccccgcgcgttggccgattcattaatgcagctggcacgacaggtttcccgactggaaagcgggcagtgagcgcaacgcaattaatgtgagttagctcactcattaggcaccccaggctttacactttatgcttccggctcgtatgttgtgtggaattgtgagcggataacaatttcacacaggaaacagctatgaccatgattacgccaagctttgctcttaggagtttcctaatacatcccaaactcaaatatataaagcatttgacttgttctatgccctagggggcggggggaagctaagccagctttttttaacatttaaaatgttaattccattttaaatgcacagatgtttttatttcataagggtttcaatgtgcatgaatgctgcaatattcctgttaccaaagctagtataaataaaaatagataaacgtggaaattacttagagtttctgtcattaacgtttccttcctcagttgacaacataaatgcgctgctgagcaagccagtttgcatctgtcaggatcaatttcccattatgccagtcatattaattactagtcaattagttgatttttatttttgacatatacatgtg

SEQ ID NO: 34 - DNA, 10238 bp, synthetic construct
  misc_feature 1..10238: note = hCD123-CAR
  source 1..10238: mol_type = other DNA
aatgaaagaccccacctgtaggtttggcaagctagcttaagtaacgccattttgcaaggcatggaaaaatacataactgagaatagaaaagttcagatcaaggtcaggaacagatggaacagctgaatatgggccaaacaggatatctgtggtaagcagttcctgccccggctcagggccaagaacagatggaacagctgaatatgggccaaacaggatatctgtggtaagcagttcctgccccggctcagggccaagaacagatggtccccagatgcggtccagccctcagcagtttctagagaaccatcagatgtttccagggtgccccaaggacctgaaatgaccctgtgccttatttgaactaaccaatcagttcgcttctcgcttctgttcgcgcgcttatgctccccgagctcaataaaagagcccacaacccctcactcggggcgccagtcctccgattgactgagtcgcccgggtacccgtgtatccaataaaccctcttgcagttgcatccgacttgtggtctcgctgttccttgggagggtctcctctgagtgattgactacccgtcagcgggggtctttcatttgggggctcgtccgggatcgggagacccctgcccagggaccaccgacccaccaccgggaggtaagctggccagcaacttatctgtgtctgtccgattgtctagtgtctatgactgattttatgcgcctgcgtcggtactagttagctaactagctctgtatctggcggacccgtggtggaactgacgagttcggaacacccggccgcaaccctgggagacgtcccagggacttcgggggccgtttttgtggcccgacctgagtcctaaaatcccgatcgtttaggactctttggtgcaccccccttagaggagggatatgtggttctggtaggagacgagaacctaaaacagttcccgcctccgtctgaatttttgctttcggtttgggaccgaagccgcgccgcgcgtcttgtctgctgcagcatcgttctgtgttgtctctgtctgactgtgtttctgtatttgtctgaaaatatgggcccgggctagcctgttaccactcccttaagtttgaccttaggtcactggaaagatgtcgagcggatcgctcacaaccagtcggtagatgtcaagaagagacgttgggttaccttctgctctgcagaatggccaacctttaacgtcggatggccgcgagacggcacctttaaccgagacctcatcacccaggttaagatcaaggtcttttcacctggcccgcatggacacccagaccaggtggggtacatcgtgacctgggaagccttggcttttgacccccctccctgggtcaagccctttgtacaccctaagcctccgcctcctcttcctccatccgccccgtctctcccccttgaacctcctcgttcgaccccgcctcgatcctccctttatccagccctcactccttctctaggcgcccccatatggccatatgagatcttatatggggcacccccgccccttgtaaacttccctgaccctgacatgacaagagttactaacagcccctctctccaagctcacttacaggctctctacttagtccagcacgaagtctggagacctctggcggcagcctaccaagaacaactggaccgaccggtggtacctcacccttaccgagtcggcgacacagtgtgggtccgccgacaccagactaagaacctagaacctcgctggaaaggaccttacacagtcctgctgaccacccccaccgccctcaaagtagacggcatcgcagcttggatacacgccgcccacgtgaaggctgccgaccccgggggtggaccatcctctagactgccatgctcgagggagtgcaggtggaaaccatctccccaggagacgggcgcaccttccccaagcgcggccagacctgcgtggtgcactacaccgggatgcttgaagatggaaagaaagttgattcctcccgggacagaaacaagccctttaagtttatgctaggcaagcaggaggtgatccgaggctgggaagaaggggttgcccagatgagtgtgggtcagagagccaaactgactatatctccagattatgcctatggtgccactgggcacccaggcatcatcccaccacatgccactctcgtcttcgatgtggagcttctaaaactggaatctggcggtggatccggagtcgacggatttggtgatgtcggtgctcttgagagtttgaggggaaatgcagatttggcttacatcctgagcatggagccctgtggccactgcctcattatcaacaatgtgaacttctgccgtgagtccgggctccgcacccgcactggctccaacatcgactgtgagaagttgcggcgtcgcttctcctcgctgcatttcatggtggaggtgaagggcgacctgactgccaagaaaatggtgctggctttgctggagctggcgcagcaggaccacggtgctctggactgctgcgtggtggtcattctctctcacggctgtcaggccagccacctgcagttcccaggggctgtctacggcacagatggatgccctgtgtcggtcgagaagattgtgaacatcttcaatgggaccagctgccccagcctgggagggaagcccaagctctttttcatccaggcctgtggtggggagcagaaagaccatgggtttgaggtggcctccacttcccctgaagacgagtcccctggcagtaaccccgagccagatgccaccccgttccaggaaggtttgaggaccttcgaccagctggacgccatatctagtttgcccacacccagtgacatctttgtgtcctactctactttcccaggttttgtttcctggagggaccccaagagtggctcctggtacgttgagaccctggacgacatctttgagcagtgggctcactctgaagacctgcagtccctcctgcttagggtcgctaatgctgtttcggtgaaagggatttataaacagatgcctggttgctttaatttcctccggaaaaaacttttctttaaaacatcagctagcagagccgagggcaggggaagtcttctaacatgcggggacgtggaggaaaatcccgggcccatggaattcgggctttcatggttgttcctcgttgcgatacttaaaggcgttcagtgcagtagagacattcagatgacccaaagccctagtagcctctccgccagtgtgggtgaccgcgtgactattacgtgccgagcaagcaagagtattagcaaagatttggcatggtaccagcagaaaccaggcaaggtccctaagttgcttatatatagcgggtctacactccaatctggagtgccggatcgcttctcaggttccggatcaggaaccgatttcactcttacaatttcctctctgcaaccggaggacgtggcaacatactattgccagcagcataacaaatatccctatactttcggtcaaggtacaaaagtagaaataaaacgaggttccacctccgggagtgggaagcccggctccggcgaaggatccaccaaaggcgaggtacagctcgttgaaagcgggggcggtctcgtccaaccaggagggtctcttcgactttcttgtgctgcaagtgggtacacgtttacttcctattggatgaattgggttcggcaagcccccggtaaagggcttgaatggatagggaggatagacccctacgattctgagacgcattataatcagaaattcaaagataagttcataataagcagagacaatgcaaaaaatagtttgtacctccagatgaatagtcttcgggcagaagacacagcggtatattactgtgctcggggtaactgggatgattactggggtcagggaactctggttactgtgtctagctacgtcaccgtctcttcacaggatcccgccgagcccaaatctcctgacaaaactcacacatgcccaccgtgcccagcacctgaactcctggggggaccgtcagtcttcctcttccccccaaaacccaaggacaccctcatgatctcccggacccctgaggtcacatgcgtggtggtggacgtgagccacgaagaccctgaggtcaagttcaactggtacgtggacggcgtggaggtgcataatgccaagacaaagccgcgggaggagcagtacaacagcacgtaccgtgtggtcagcgtcctcaccgtcctgcaccaggactggctgaatggcaaggagtacaagtgcaaggtctccaacaaagccctcccagcccccatcgagaaaaccatctccaaagccaaagggcagccccgagaaccacaggtgtacaccctgcccccatcccgggatgagctgaccaagaaccaggtcagcctgacctgcctggtcaaaggcttctatcccagcgacatcgccgtggagtgggagagcaatgggcaaccggagaacaactacaagaccacgcctcccgtgctggactccgacggctccttcttcctctacagcaagctcaccgtggacaagagcaggtggcagcaggggaacgtcttctcatgctccgtgatgcatgaggctctgcacaaccactacacgcagaagagcctctccctgtctccgggtaaaaaagatcccaaattttgggtgctggtggtggttggtggagtcctggcttgctatagcttgctagtaacagtggcctttattattttctgggtgaggagtaagaggagcaggctcctgcacagtgactacatgaacatgactccccgccgccccgggcccacccgcaagcattaccagccctatgccccaccacgcgacttcgcagcctatcgctccagagtgaagttcagcaggagcgcagacgcccccgcgtaccagcagggccagaaccagctctataacgagctcaatctaggacgaagagaggagtacgatgttttggacaagagacgtggccgggaccctgagatggggggaaagccgagaaggaagaaccctcaggaaggcctgtacaatgaactgcagaaagataagatggcggaggcctacagtgagattgggatgaaaggcgagcgccggaggggcaaggggcacgatggcctttaccagggtctcagtacagccaccaaggacacctacgacgcccttcacatgcaggccctgccccctcgcggaccgcagtgtactaattatgctctcttgaaattggctggagatgttgagagcaatcccgggcccatgcggatcagcaagccccacctgcggagcatcagcatccagtgctacctgtgcctgctgctgaacagccacttcctgaccgaggccggcatccacgtgttcatcctgggctgcttcagcgccggactgcccaagaccgaggccaactgggtgaacgtgatcagcgacctgaagaagatcgaggacctgatccagagcatgcacatcgacgccaccctgtacaccgagagcgacgtgcaccccagctgcaaggtgaccgccatgaagtgctttctgctggaactgcaggtgatcagcctggaaagcggcgacgccagcatccacgacaccgtggagaacctgatcatcctggccaacaacagcctgagcagcaacggcaacgtgaccgagagcggctgcaaagagtgcgaggaactggaagagaagaacatcaaagagtttctgcagagcttcgtgcacatcgtgcagatgttcatcaacaccagctgacgcgtcatcatcgatccggattagtccaatttgttaaagacaggatatcagtggtccaggctctagttttgactcaacaatatcaccagctgaagcctatagagtacgagccatagataaaataaaagattttatttagtctccagaaaaaggggggaatgaaagaccccacctgtaggtttggcaagctagcttaagtaacgccattttgcaaggcatggaaaaatacataactgagaatagagaagttcagatcaaggtcaggaacagatggaacagctgaatatgggccaaacaggatatctgtggtaagcagttcctgccccggctcagggccaagaacagatggaacagctgaatatgggccaaacaggatatctgtggtaagcagttcctgccccggctcagggccaagaacagatggtccccagatgcggtccagccctcagcagtttctagagaaccatcagatgtttccagggtgccccaaggacctgaaatgaccctgtgccttatttgaactaaccaatcagttcgcttctcgcttctgttcgcgcgcttctgctccccgagctcaataaaagagcccacaacccctcactcggggcgccagtcctccgattgactgagtcgcccgggtacccgtgtatccaataaaccctcttgcagttgcatccgacttgtggtctcgctgttccttgggagggtctcctctgagtgattgactacccgtcagcgggggtctttcacacatgcagcatgtatcaaaattaatttggttttttttcttaagtatttacattaaatggccatagtacttaaagttacattggcttccttgaaataaacatggagtattcagaatgtgtcataaatatttctaattttaagatagtatctccattggctttctactttttcttttatttttttttgtcctctgtcttccatttgttgttgttgttgtttgtttgtttgtttgttggttggttggttaatttttttttaaagatcctacactatagttcaagctagactattagctactctgtaacccagggtgaccttgaagtcatgggtagcctgctgttttagccttcccacatctaagattacaggtatgagctatcatttttggtatattgattgattgattgattgatgtgtgtgtgtgtgattgtgtttgtgtgtgtgactgtgaaaatgtgtgtatgggtgtgtgtgaatgtgtgtatgtatgtgtgtgtgtgagtgtgtgtgtgtgtgtgtgcatgtgtgtgtgtgtgactgtgtctatgtgtatgactgtgtgtgtgtgtgtgtgtgtgtgtgtgtgtgtgtgtgtgtgtgtgttgtgaaaaaatattctatggtagtgagagccaacgctccggctcaggtgtcaggttggtttttgagacagagtctttcacttagcttggaattcactggccgtcgttttacaacgtcgtgactgggaaaaccctggcgttacccaacttaatcgccttgcagcacatccccctttcgccagctggcgtaatagcgaagaggcccgcaccgatcgcccttcccaacagttgcgcagcctgaatggcgaatggcgcctgatgcggtattttctccttacgcatctgtgcggtatttcacaccgcatatggtgcactctcagtacaatctgctctgatgccgcatagttaagccagccccgacacccgccaacacccgctgacgcgccctgacgggcttgtctgctcccggcatccgcttacagacaagctgtgaccgtctccgggagctgcatgtgtcagaggttttcaccgtcatcaccgaaacgcgcgagacgaaagggcctcgtgatacgcctatttttataggttaatgtcatgataataatggtttcttagacgtcaggtggcacttttcggggaaatgtgcgcggaacccctatttgtttatttttctaaatacattcaaatatgtatccgctcatgagacaataaccctgataaatgcttcaataatattgaaaaaggaagagtatgagtattcaacatttccgtgtcgcccttattcccttttttgcggcattttgccttcctgtttttgctcacccagaaacgctggtgaaagtaaaagatgctgaagatcagttgggtgcacgagtgggttacatcgaactggatctcaacagcggtaagatccttgagagttttcgccccgaagaacgttttccaatgatgagcacttttaaagttctgctatgtggcgcggtattatcccgtattgacgccgggcaagagcaactcggtcgccgcatacactattctcagaatgacttggttgagtactcaccagtcacagaaaagcatcttacggatggcatgacagtaagagaattatgcagtgctgccataaccatgagtgataacactgcggccaacttacttctgacaacgatcggaggaccgaaggagctaaccgcttttttgcacaacatgggggatcatgtaactcgccttgatcgttgggaaccggagctgaatgaagccataccaaacgacgagcgtgacaccacgatgcctgtagcaatggcaacaacgttgcgcaaactattaactggcgaactacttactctagcttcccggcaacaattaatagactggatggaggcggataaagttgcaggaccacttctgcgctcggcccttccggctggctggtttattgctgataaatctggagccggtgagcgtgggtctcgcggtatcattgcagcactggggccagatggtaagccctcccgtatcgtagttatctacacgacggggagtcaggcaactatggatgaacgaaatagacagatcgctgagataggtgcctcactgattaagcattggtaactgtcagaccaagtttactcatatatactttagattgatttaaaacttcatttttaatttaaaaggatctaggtgaagatcctttttgataatctcatgaccaaaatcccttaacgtgagttttcgttccactgagcgtcagaccccgtagaaaagatcaaaggatcttcttgagatcctttttttctgcgcgtaatctgctgcttgcaaacaaaaaaaccaccgctaccagcggtggtttgtttgccggatcaagagctaccaactctttttccgaaggtaactggcttcagcagagcgcagataccaaatactgttcttctagtgtagccgtagttaggccaccacttcaagaactctgtagcaccgcctacatacctcgctctgctaatcctgttaccagtggctgctgccagtggcgataagtcgtgtcttaccgggttggactcaagacgatagttaccggataaggcgcagcggtcgggctgaacggggggttcgtgcacacagcccagcttggagcgaacgacctacaccgaactgagatacctacagcgtgagctatgagaaagcgccacgcttcccgaagggagaaaggcggacaggtatccggtaagcggcagggtcggaacaggagagcgcacgagggagcttccagggggaaacgcctggtatctttatagtcctgtcgggtttcgccacctctgacttgagcgtcgatttttgtgatgctcgtcaggggggcggagcctatggaaaaacgccagcaacgcggcctttttacggttcctggccttttgctggccttttgctcacatgttctttcctgcgttatcccctgattctgtggataaccgtattaccgcctttgagtgagctgataccgctcgccgcagccgaacgaccgagcgcagcgagtcagtgagcgaggaagcggaagagcgcccaatacgcaaaccgcctctccccgcgcgttggccgattcattaatgcagctggcacgacaggtttcccgactggaaagcgggcagtgagcgcaacgcaattaatgtgagttagctcactcattaggcaccccaggctttacactttatgcttccggctcgtatgttgtgtggaattgtgagcggataacaatttcacacaggaaacagctatgaccatgattacgccaagctttgctcttaggagtttcctaatacatcccaaactcaaatatataaagcatttgacttgttctatgccctagggggcggggggaagctaagccagctttttttaacatttaaaatgttaattccattttaaatgcacagatgtttttatttcataagggtttcaatgtgcatgaatgctgcaatattcctgttaccaaagctagtataaataaaaatagataaacgtggaaattacttagagtttctgtcattaacgtttccttcctcagttgacaacataaatgcgctgctgagcaagccagtttgcatctgtcaggatcaatttcccattatgccagtcatattaattactagtcaattagttgatttttatttttgacatatacatgtg

SEQ ID NO: 35 - DNA, 10229 bp, synthetic construct
  misc_feature 1..10229: note = hMeso-CAR
  source 1..10229: mol_type = other DNA
aatgaaagaccccacctgtaggtttggcaagctagcttaagtaacgccattttgcaaggcatggaaaaatacataactgagaatagaaaagttcagatcaaggtcaggaacagatggaacagctgaatatgggccaaacaggatatctgtggtaagcagttcctgccccggctcagggccaagaacagatggaacagctgaatatgggccaaacaggatatctgtggtaagcagttcctgccccggctcagggccaagaacagatggtccccagatgcggtccagccctcagcagtttctagagaaccatcagatgtttccagggtgccccaaggacctgaaatgaccctgtgccttatttgaactaaccaatcagttcgcttctcgcttctgttcgcgcgcttatgctccccgagctcaataaaagagcccacaacccctcactcggggcgccagtcctccgattgactgagtcgcccgggtacccgtgtatccaataaaccctcttgcagttgcatccgacttgtggtctcgctgttccttgggagggtctcctctgagtgattgactacccgtcagcgggggtctttcatttgggggctcgtccgggatcgggagacccctgcccagggaccaccgacccaccaccgggaggtaagctggccagcaacttatctgtgtctgtccgattgtctagtgtctatgactgattttatgcgcctgcgtcggtactagttagctaactagctctgtatctggcggacccgtggtggaactgacgagttcggaacacccggccgcaaccctgggagacgtcccagggacttcgggggccgtttttgtggcccgacctgagtcctaaaatcccgatcgtttaggactctttggtgcaccccccttagaggagggatatgtggttctggtaggagacgagaacctaaaacagttcccgcctccgtctgaatttttgctttcggtttgggaccgaagccgcgccgcgcgtcttgtctgctgcagcatcgttctgtgttgtctctgtctgactgtgtttctgtatttgtctgaaaatatgggcccgggctagcctgttaccactcccttaagtttgaccttaggtcactggaaagatgtcgagcggatcgctcacaaccagtcggtagatgtcaagaagagacgttgggttaccttctgctctgcagaatggccaacctttaacgtcggatggccgcgagacggcacctttaaccgagacctcatcacccaggttaagatcaaggtcttttcacctggcccgcatggacacccagaccaggtggggtacatcgtgacctgggaagccttggcttttgacccccctccctgggtcaagccctttgtacaccctaagcctccgcctcctcttcctccatccgccccgtctctcccccttgaacctcctcgttcgaccccgcctcgatcctccctttatccagccctcactccttctctaggcgcccccatatggccatatgagatcttatatggggcacccccgccccttgtaaacttccctgaccctgacatgacaagagttactaacagcccctctctccaagctcacttacaggctctctacttagtccagcacgaagtctggagacctctggcggcagcctaccaagaacaactggaccgaccggtggtacctcacccttaccgagtcggcgacacagtgtgggtccgccgacaccagactaagaacctagaacctcgctggaaaggaccttacacagtcctgctgaccacccccaccgccctcaaagtagacggcatcgcagcttggatacacgccgcccacgtgaaggctgccgaccccgggggtggaccatcctctagactgccatgctcgagggagtgcaggtggaaaccatctccccaggagacgggcgcaccttccccaagcgcggccagacctgcgtggtgcactacaccgggatgcttgaagatggaaagaaagttgattcctcccgggacagaaacaagccctttaagtttatgctaggcaagcaggaggtgatccgaggctgggaagaaggggttgcccagatgagtgtgggtcagagagccaaactgactatatctccagattatgcctatggtgccactgggcacccaggcatcatcccaccacatgccactctcgtcttcgatgtggagcttctaaaactggaatctggcggtggatccggagtcgacggatttggtgatgtcggtgctcttgagagtttgaggggaaatgcagatttggcttacatcctgagcatggagccctgtggccactgcctcattatcaacaatgtgaacttctgccgtgagtccgggctccgcacccgcactggctccaacatcgactgtgagaagttgcggcgtcgcttctcctcgctgcatttcatggtggaggtgaagggcgacctgactgccaagaaaatggtgctggctttgctggagctggcgcagcaggaccacggtgctctggactgctgcgtggtggtcattctctctcacggctgtcaggccagccacctgcagttcccaggggctgtctacggcacagatggatgccctgtgtcggtcgagaagattgtgaacatcttcaatgggaccagctgccccagcctgggagggaagcccaagctctttttcatccaggcctgtggtggggagcagaaagaccatgggtttgaggtggcctccacttcccctgaagacgagtcccctggcagtaaccccgagccagatgccaccccgttccaggaaggtttgaggaccttcgaccagctggacgccatatctagtttgcccacacccagtgacatctttgtgtcctactctactttcccaggttttgtttcctggagggaccccaagagtggctcctggtacgttgagaccctggacgacatctttgagcagtgggctcactctgaagacctgcagtccctcctgcttagggtcgctaatgctgtttcggtgaaagggatttataaacagatgcctggttgctttaatttcctccggaaaaaacttttctttaaaacatcagctagcagagccgagggcaggggaagtcttctaacatgcggggacgtggaggaaaatcccgggcccatggagttcggcctttcttggctgtttttggtcgcaatattgaagggcgttcagtgttcaagggacatacagatgacgcagtcacctagctctctttcagcctctgtgggagaccgcgttacaattacgtgttctgcttctagttcagtgtcttacatgcattggtaccagcaaaaacccggcaaggttccaaagctccttatatacgatacgtccaaactggcttcaggcgtgccagacaggtttagtggatctgggagcggcactgacttcacacttacaatatccagtctgcaacccgaagatgttgcgacatactattgtcagcaatggagcggctatccgctcaccggacaggggacaaaagtggagataaagcggggctccaccagtggttccgggaagcctggtagtggtgagggttctacgaaaggcgaagtgcagttggtggagtctggtggcgggcttgttcaacccggtggttctctcaggcttagctgtgcagcctctgggtacacaatgaattgggtaaggcaagcgcctggaaagggccttgagtggatcggtttgataaccccatacaacggagcttcaagttacaaccaaaagttccgcgggaagtttattataagcagggataacgcaaagaacagcctctatcttcaaatgaactcactccgggctgaagacacagccgtctattattgtgcccgggggggctacgacggacgagggttcgattactggggtcagggcacactcgtgaccgtgtcaagctacgtcaccgtctcttcacaggatcccgccgagcccaaatctcctgacaaaactcacacatgcccaccgtgcccagcacctgaactcctggggggaccgtcagtcttcctcttccccccaaaacccaaggacaccctcatgatctcccggacccctgaggtcacatgcgtggtggtggacgtgagccacgaagaccctgaggtcaagttcaactggtacgtggacggcgtggaggtgcataatgccaagacaaagccgcgggaggagcagtacaacagcacgtaccgtgtggtcagcgtcctcaccgtcctgcaccaggactggctgaatggcaaggagtacaagtgcaaggtctccaacaaagccctcccagcccccatcgagaaaaccatctccaaagccaaagggcagccccgagaaccacaggtgtacaccctgcccccatcccgggatgagctgaccaagaaccaggtcagcctgacctgcctggtcaaaggcttctatcccagcgacatcgccgtggagtgggagagcaatgggcaaccggagaacaactacaagaccacgcctcccgtgctggactccgacggctccttcttcctctacagcaagctcaccgtggacaagagcaggtggcagcaggggaacgtcttctcatgctccgtgatgcatgaggctctgcacaaccactacacgcagaagagcctctccctgtctccgggtaaaaaagatcccaaattttgggtgctggtggtggttggtggagtcctggcttgctatagcttgctagtaacagtggcctttattattttctgggtgaggagtaagaggagcaggctcctgcacagtgactacatgaacatgactccccgccgccccgggcccacccgcaagcattaccagccctatgccccaccacgcgacttcgcagcctatcgctccagagtgaagttcagcaggagcgcagacgcccccgcgtaccagcagggccagaaccagctctataacgagctcaatctaggacgaagagaggagtacgatgttttggacaagagacgtggccgggaccctgagatggggggaaagccgagaaggaagaaccctcaggaaggcctgtacaatgaactgcagaaagataagatggcggaggcctacagtgagattgggatgaaaggcgagcgccggaggggcaaggggcacgatggcctttaccagggtctcagtacagccaccaaggacacctacgacgcccttcacatgcaggccctgccccctcgcggaccgcagtgtactaattatgctctcttgaaattggctggagatgttgagagcaatcccgggcccatgcggatcagcaagccccacctgcggagcatcagcatccagtgctacctgtgcctgctgctgaacagccacttcctgaccgaggccggcatccacgtgttcatcctgggctgcttcagcgccggactgcccaagaccgaggccaactgggtgaacgtgatcagcgacctgaagaagatcgaggacctgatccagagcatgcacatcgacgccaccctgtacaccgagagcgacgtgcaccccagctgcaaggtgaccgccatgaagtgctttctgctggaactgcaggtgatcagcctggaaagcggcgacgccagcatccacgacaccgtggagaacctgatcatcctggccaacaacagcctgagcagcaacggcaacgtgaccgagagcggctgcaaagagtgcgaggaactggaagagaagaacatcaaagagtttctgcagagcttcgtgcacatcgtgcagatgttcatcaacaccagctgacgcgtcatcatcgatccggattagtccaatttgttaaagacaggatatcagtggtccaggctctagttttgactcaacaatatcaccagctgaagcctatagagtacgagccatagataaaataaaagattttatttagtctccagaaaaaggggggaatgaaagaccccacctgtaggtttggcaagctagcttaagtaacgccattttgcaaggcatggaaaaatacataactgagaatagagaagttcagatcaaggtcaggaacagatggaacagctgaatatgggccaaacaggatatctgtggtaagcagttcctgccccggctcagggccaagaacagatggaacagctgaatatgggccaaacaggatatctgtggtaagcagttcctgccccggctcagggccaagaacagatggtccccagatgcggtccagccctcagcagtttctagagaaccatcagatgtttccagggtgccccaaggacctgaaatgaccctgtgccttatttgaactaaccaatcagttcgcttctcgcttctgttcgcgcgcttctgctccccgagctcaataaaagagcccacaacccctcactcggggcgccagtcctccgattgactgagtcgcccgggtacccgtgtatccaataaaccctcttgcagttgcatccgacttgtggtctcgctgttccttgggagggtctcctctgagtgattgactacccgtcagcgggggtctttcacacatgcagcatgtatcaaaattaatttggttttttttcttaagtatttacattaaatggccatagtacttaaagttacattggcttccttgaaataaacatggagtattcagaatgtgtcataaatatttctaattttaagatagtatctccattggctttctactttttcttttatttttttttgtcctctgtcttccatttgttgttgttgttgtttgtttgtttgtttgttggttggttggttaatttttttttaaagatcctacactatagttcaagctagactattagctactctgtaacccagggtgaccttgaagtcatgggtagcctgctgttttagccttcccacatctaagattacaggtatgagctatcatttttggtatattgattgattgattgattgatgtgtgtgtgtgtgattgtgtttgtgtgtgtgactgtgaaaatgtgtgtatgggtgtgtgtgaatgtgtgtatgtatgtgtgtgtgtgagtgtgtgtgtgtgtgtgtgcatgtgtgtgtgtgtgactgtgtctatgtgtatgactgtgtgtgtgtgtgtgtgtgtgtgtgtgtgtgtgtgtgtgtgtgtgttgtgaaaaaatattctatggtagtgagagccaacgctccggctcaggtgtcaggttggtttttgagacagagtctttcacttagcttggaattcactggccgtcgttttacaacgtcgtgactgggaaaaccctggcgttacccaacttaatcgccttgcagcacatccccctttcgccagctggcgtaatagcgaagaggcccgcaccgatcgcccttcccaacagttgcgcagcctgaatggcgaatggcgcctgatgcggtattttctccttacgcatctgtgcggtatttcacaccgcatatggtgcactctcagtacaatctgctctgatgccgcatagttaagccagccccgacacccgccaacacccgctgacgcgccctgacgggcttgtctgctcccggcatccgcttacagacaagctgtgaccgtctccgggagctgcatgtgtcagaggttttcaccgtcatcaccgaaacgcgcgagacgaaagggcctcgtgatacgcctatttttataggttaatgtcatgataataatggtttcttagacgtcaggtggcacttttcggggaaatgtgcgcggaacccctatttgtttatttttctaaatacattcaaatatgtatccgctcatgagacaataaccctgataaatgcttcaataatattgaaaaaggaagagtatgagtattcaacatttccgtgtcgcccttattcccttttttgcggcattttgccttcctgtttttgctcacccagaaacgctggtgaaagtaaaagatgctgaagatcagttgggtgcacgagtgggttacatcgaactggatctcaacagcggtaagatccttgagagttttcgccccgaagaacgttttccaatgatgagcacttttaaagttctgctatgtggcgcggtattatcccgtattgacgccgggcaagagcaactcggtcgccgcatacactattctcagaatgacttggttgagtactcaccagtcacagaaaagcatcttacggatggcatgacagtaagagaattatgcagtgctgccataaccatgagtgataacactgcggccaacttacttctgacaacgatcggaggaccgaaggagctaaccgcttttttgcacaacatgggggatcatgtaactcgccttgatcgttgggaaccggagctgaatgaagccataccaaacgacgagcgtgacaccacgatgcctgtagcaatggcaacaacgttgcgcaaactattaactggcgaactacttactctagcttcccggcaacaattaatagactggatggaggcggataaagttgcaggaccacttctgcgctcggcccttccggctggctggtttattgctgataaatctggagccggtgagcgtgggtctcgcggtatcattgcagcactggggccagatggtaagccctcccgtatcgtagttatctacacgacggggagtcaggcaactatggatgaacgaaatagacagatcgctgagataggtgcctcactgattaagcattggtaactgtcagaccaagtttactcatatatactttagattgatttaaaacttcatttttaatttaaaaggatctaggtgaagatcctttttgataatctcatgaccaaaatcccttaacgtgagttttcgttccactgagcgtcagaccccgtagaaaagatcaaaggatcttcttgagatcctttttttctgcgcgtaatctgctgcttgcaaacaaaaaaaccaccgctaccagcggtggtttgtttgccggatcaagagctaccaactctttttccgaaggtaactggcttcagcagagcgcagataccaaatactgttcttctagtgtagccgtagttaggccaccacttcaagaactctgtagcaccgcctacatacctcgctctgctaatcctgttaccagtggctgctgccagtggcgataagtcgtgtcttaccgggttggactcaagacgatagttaccggataaggcgcagcggtcgggctgaacggggggttcgtgcacacagcccagcttggagcgaacgacctacaccgaactgagatacctacagcgtgagctatgagaaagcgccacgcttcccgaagggagaaaggcggacaggtatccggtaagcggcagggtcggaacaggagagcgcacgagggagcttccagggggaaacgcctggtatctttatagtcctgtcgggtttcgccacctctgacttgagcgtcgatttttgtgatgctcgtcaggggggcggagcctatggaaaaacgccagcaacgcggcctttttacggttcctggccttttgctggccttttgctcacatgttctttcctgcgttatcccctgattctgtggataaccgtattaccgcctttgagtgagctgataccgctcgccgcagccgaacgaccgagcgcagcgagtcagtgagcgaggaagcggaagagcgcccaatacgcaaaccgcctctccccgcgcgttggccgattcattaatgcagctggcacgacaggtttcccgactggaaagcgggcagtgagcgcaacgcaattaatgtgagttagctcactcattaggcaccccaggctttacactttatgcttccggctcgtatgttgtgtggaattgtgagcggataacaatttcacacaggaaacagctatgaccatgattacgccaagctttgctcttaggagtttcctaatacatcccaaactcaaatatataaagcatttgacttgttctatgccctagggggcggggggaagctaagccagctttttttaacatttaaaatgttaattccattttaaatgcacagatgtttttatttcataagggtttcaatgtgcatgaatgctgcaatattcctgttaccaaagctagtataaataaaaatagataaacgtggaaattacttagagtttctgtcattaacgtttccttcctcagttgacaacataaatgcgctgctgagcaagccagtttgcatctgtcaggatcaatttcccattatgccagtcatattaattactagtcaattagttgatttttatttttgacatatacatgtg

SEQ ID NO: 36 - DNA, 10250 bp, synthetic construct
  misc_feature 1..10250: note = hROR1-CAR
  source 1..10250: mol_type = other DNA
aatgaaagaccccacctgtaggtttggcaagctagcttaagtaacgccattttgcaaggcatggaaaaatacataactgagaatagaaaagttcagatcaaggtcaggaacagatggaacagctgaatatgggccaaacaggatatctgtggtaagcagttcctgccccggctcagggccaagaacagatggaacagctgaatatgggccaaacaggatatctgtggtaagcagttcctgccccggctcagggccaagaacagatggtccccagatgcggtccagccctcagcagtttctagagaaccatcagatgtttccagggtgccccaaggacctgaaatgaccctgtgccttatttgaactaaccaatcagttcgcttctcgcttctgttcgcgcgcttatgctccccgagctcaataaaagagcccacaacccctcactcggggcgccagtcctccgattgactgagtcgcccgggtacccgtgtatccaataaaccctcttgcagttgcatccgacttgtggtctcgctgttccttgggagggtctcctctgagtgattgactacccgtcagcgggggtctttcatttgggggctcgtccgggatcgggagacccctgcccagggaccaccgacccaccaccgggaggtaagctggccagcaacttatctgtgtctgtccgattgtctagtgtctatgactgattttatgcgcctgcgtcggtactagttagctaactagctctgtatctggcggacccgtggtggaactgacgagttcggaacacccggccgcaaccctgggagacgtcccagggacttcgggggccgtttttgtggcccgacctgagtcctaaaatcccgatcgtttaggactctttggtgcaccccccttagaggagggatatgtggttctggtaggagacgagaacctaaaacagttcccgcctccgtctgaatttttgctttcggtttgggaccgaagccgcgccgcgcgtcttgtctgctgcagcatcgttctgtgttgtctctgtctgactgtgtttctgtatttgtctgaaaatatgggcccgggctagcctgttaccactcccttaagtttgaccttaggtcactggaaagatgtcgagcggatcgctcacaaccagtcggtagatgtcaagaagagacgttgggttaccttctgctctgcagaatggccaacctttaacgtcggatggccgcgagacggcacctttaaccgagacctcatcacccaggttaagatcaaggtcttttcacctggcccgcatggacacccagaccaggtggggtacatcgtgacctgggaagccttggcttttgacccccctccctgggtcaagccctttgtacaccctaagcctccgcctcctcttcctccatccgccccgtctctcccccttgaacctcctcgttcgaccccgcctcgatcctccctttatccagccctcactccttctctaggcgcccccatatggccatatgagatcttatatggggcacccccgccccttgtaaacttccctgaccctgacatgacaagagttactaacagcccctctctccaagctcacttacaggctctctacttagtccagcacgaagtctggagacctctggcggcagcctaccaagaacaactggaccgaccggtggtacctcacccttaccgagtcggcgacacagtgtgggtccgccgacaccagactaagaacctagaacctcgctggaaaggaccttacacagtcctgctgaccacccccaccgccctcaaagtagacggcatcgcagcttggatacacgccgcccacgtgaaggctgccgaccccgggggtggaccatcctctagactgccatgctcgagggagtgcaggtggaaaccatctccccaggagacgggcgcaccttccccaagcgcggccagacctgcgtggtgcactacaccgggatgcttgaagatggaaagaaagttgattcctcccgggacagaaacaagccctttaagtttatgctaggcaagcaggaggtgatccgaggctgggaagaaggggttgcccagatgagtgtgggtcagagagccaaactgactatatctccagattatgcctatggtgccactgggcacccaggcatcatcccaccacatgccactctcgtcttcgatgtggagcttctaaaactggaatctggcggtggatccggagtcgacggatttggtgatgtcggtgctcttgagagtttgaggggaaatgcagatttggcttacatcctgagcatggagccctgtggccactgcctcattatcaacaatgtgaacttctgccgtgagtccgggctccgcacccgcactggctccaacatcgactgtgagaagttgcggcgtcgcttctcctcgctgcatttcatggtggaggtgaagggcgacctgactgccaagaaaatggtgctggctttgctggagctggcgcagcaggaccacggtgctctggactgctgcgtggtggtcattctctctcacggctgtcaggccagccacctgcagttcccaggggctgtctacggcacagatggatgccctgtgtcggtcgagaagattgtgaacatcttcaatgggaccagctgccccagcctgggagggaagcccaagctctttttcatccaggcctgtggtggggagcagaaagaccatgggtttgaggtggcctccacttcccctgaagacgagtcccctggcagtaaccccgagccagatgccaccccgttccaggaaggtttgaggaccttcgaccagctggacgccatatctagtttgcccacacccagtgacatctttgtgtcctactctactttcccaggttttgtttcctggagggaccccaagagtggctcctggtacgttgagaccctggacgacatctttgagcagtgggctcactctgaagacctgcagtccctcctgcttagggtcgctaatgctgtttcggtgaaagggatttataaacagatgcctggttgctttaatttcctccggaaaaaacttttctttaaaacatcagctagcagagccgagggcaggggaagtcttctaacatgcggggacgtggaggaaaatcccgggcccatggagttcggacttagttggcttttcctcgtcgccatactcaaaggtgtacaatgctcacgcgatatacaaatgacgcagagtccatcctcactgtctgcctcagtaggcgacagggtcacaataacctgtaaagcaagcccggatatcaactcttacctcagttggttccaacagaaaccaggaaaggtgccgaagttgttgatttaccgcgcaaaccgcctcgttgacggcgtgccagataggttttctggcagcgggagcggcactgactttacgctcactatatcaagcctgcagccggaggacgtagcaacttactattgcctccaatacgacgaattcccttacacgttcgggcaaggaactaaagttgaaataaaaagaggaagcacaagtggttctggaaaacccggttccggtgagggcagtaccaaaggagaggtgcagttggtagagtctggtgggggtttggtgcaacccggagggtctctgaggttgtcttgcgcggcatccggctttactttttcctcatatgcgatgtcatgggtacgacaggccccaggcaagggactggagtggatcgcatctatttcacgaggagggacgacatattacccggattcagtgaagggcaaattcataatttcacgcgataacgccaagaactccctctacctgcaaatgaacagtcttagagcggaagatacggctgtgtattactgtgcgcgatatgactacgatggatattacgcgatggattattggggacaaggtacactggtaaccgtttccagctacgtcaccgtctcttcacaggatcccgccgagcccaaatctcctgacaaaactcacacatgcccaccgtgcccagcacctgaactcctggggggaccgtcagtcttcctcttccccccaaaacccaaggacaccctcatgatctcccggacccctgaggtcacatgcgtggtggtggacgtgagccacgaagaccctgaggtcaagttcaactggtacgtggacggcgtggaggtgcataatgccaagacaaagccgcgggaggagcagtacaacagcacgtaccgtgtggtcagcgtcctcaccgtcctgcaccaggactggctgaatggcaaggagtacaagtgcaaggtctccaacaaagccctcccagcccccatcgagaaaaccatctccaaagccaaagggcagccccgagaaccacaggtgtacaccctgcccccatcccgggatgagctgaccaagaaccaggtcagcctgacctgcctggtcaaaggcttctatcccagcgacatcgccgtggagtgggagagcaatgggcaaccggagaacaactacaagaccacgcctcccgtgctggactccgacggctccttcttcctctacagcaagctcaccgtggacaagagcaggtggcagcaggggaacgtcttctcatgctccgtgatgcatgaggctctgcacaaccactacacgcagaagagcctctccctgtctccgggtaaaaaagatcccaaattttgggtgctggtggtggttggtggagtcctggcttgctatagcttgctagtaacagtggcctttattattttctgggtgaggagtaagaggagcaggctcctgcacagtgactacatgaacatgactccccgccgccccgggcccacccgcaagcattaccagccctatgccccaccacgcgacttcgcagcctatcgctccagagtgaagttcagcaggagcgcagacgcccccgcgtaccagcagggccagaaccagctctataacgagctcaatctaggacgaagagaggagtacgatgttttggacaagagacgtggccgggaccctgagatggggggaaagccgagaaggaagaaccctcaggaaggcctgtacaatgaactgcagaaagataagatggcggaggcctacagtgagattgggatgaaaggcgagcgccggaggggcaaggggcacgatggcctttaccagggtctcagtacagccaccaaggacacctacgacgcccttcacatgcaggccctgccccctcgcggaccgcagtgtactaattatgctctcttgaaattggctggagatgttgagagcaatcccgggcccatgcggatcagcaagccccacctgcggagcatcagcatccagtgctacctgtgcctgctgctgaacagccacttcctgaccgaggccggcatccacgtgttcatcctgggctgcttcagcgccggactgcccaagaccgaggccaactgggtgaacgtgatcagcgacctgaagaagatcgaggacctgatccagagcatgcacatcgacgccaccctgtacaccgagagcgacgtgcaccccagctgcaaggtgaccgccatgaagtgctttctgctggaactgcaggtgatcagcctggaaagcggcgacgccagcatccacgacaccgtggagaacctgatcatcctggccaacaacagcctgagcagcaacggcaacgtgaccgagagcggctgcaaagagtgcgaggaactggaagagaagaacatcaaagagtttctgcagagcttcgtgcacatcgtgcagatgttcatcaacaccagctgacgcgtcatcatcgatccggattagtccaatttgttaaagacaggatatcagtggtccaggctctagttttgactcaacaatatcaccagctgaagcctatagagtacgagccatagataaaataaaagattttatttagtctccagaaaaaggggggaatgaaagaccccacctgtaggtttggcaagctagcttaagtaacgccattttgcaaggcatggaaaaatacataactgagaatagagaagttcagatcaaggtcaggaacagatggaacagctgaatatgggccaaacaggatatctgtggtaagcagttcctgccccggctcagggccaagaacagatggaacagctgaatatgggccaaacaggatatctgtggtaagcagttcctgccccggctcagggccaagaacagatggtccccagatgcggtccagccctcagcagtttctagagaaccatcagatgtttccagggtgccccaaggacctgaaatgaccctgtgccttatttgaactaaccaatcagttcgcttctcgcttctgttcgcgcgcttctgctccccgagctcaataaaagagcccacaacccctcactcggggcgccagtcctccgattgactgagtcgcccgggtacccgtgtatccaataaaccctcttgcagttgcatccgacttgtggtctcgctgttccttgggagggtctcctctgagtgattgactacccgtcagcgggggtctttcacacatgcagcatgtatcaaaattaatttggttttttttcttaagtatttacattaaatggccatagtacttaaagttacattggcttccttgaaataaacatggagtattcagaatgtgtcataaatatttctaattttaagatagtatctccattggctttctactttttcttttatttttttttgtcctctgtcttccatttgttgttgttgttgtttgtttgtttgtttgttggttggttggttaatttttttttaaagatcctacactatagttcaagctagactattagctactctgtaacccagggtgaccttgaagtcatgggtagcctgctgttttagccttcccacatctaagattacaggtatgagctatcatttttggtatattgattgattgattgattgatgtgtgtgtgtgtgattgtgtttgtgtgtgtgactgtgaaaatgtgtgtatgggtgtgtgtgaatgtgtgtatgtatgtgtgtgtgtgagtgtgtgtgtgtgtgtgtgcatgtgtgtgtgtgtgactgtgtctatgtgtatgactgtgtgtgtgtgtgtgtgtgtgtgtgtgtgtgtgtgtgtgtgtgtgttgtgaaaaaatattctatggtagtgagagccaacgctccggctcaggtgtcaggttggtttttgagacagagtctttcacttagcttggaattcactggccgtcgttttacaacgtcgtgactgggaaaaccctggcgttacccaacttaatcgccttgcagcacatccccctttcgccagctggcgtaatagcgaagaggcccgcaccgatcgcccttcccaacagttgcgcagcctgaatggcgaatggcgcctgatgcggtattttctccttacgcatctgtgcggtatttcacaccgcatatggtgcactctcagtacaatctgctctgatgccgcatagttaagccagccccgacacccgccaacacccgctgacgcgccctgacgggcttgtctgctcccggcatccgcttacagacaagctgtgaccgtctccgggagctgcatgtgtcagaggttttcaccgtcatcaccgaaacgcgcgagacgaaagggcctcgtgatacgcctatttttataggttaatgtcatgataataatggtttcttagacgtcaggtggcacttttcggggaaatgtgcgcggaacccctatttgtttatttttctaaatacattcaaatatgtatccgctcatgagacaataaccctgataaatgcttcaataatattgaaaaaggaagagtatgagtattcaacatttccgtgtcgcccttattcccttttttgcggcattttgccttcctgtttttgctcacccagaaacgctggtgaaagtaaaagatgctgaagatcagttgggtgcacgagtgggttacatcgaactggatctcaacagcggtaagatccttgagagttttcgccccgaagaacgttttccaatgatgagcacttttaaagttctgctatgtggcgcggtattatcccgtattgacgccgggcaagagcaactcggtcgccgcatacactattctcagaatgacttggttgagtactcaccagtcacagaaaagcatcttacggatggcatgacagtaagagaattatgcagtgctgccataaccatgagtgataacactgcggccaacttacttctgacaacgatcggaggaccgaaggagctaaccgcttttttgcacaacatgggggatcatgtaactcgccttgatcgttgggaaccggagctgaatgaagccataccaaacgacgagcgtgacaccacgatgcctgtagcaatggcaacaacgttgcgcaaactattaactggcgaactacttactctagcttcccggcaacaattaatagactggatggaggcggataaagttgcaggaccacttctgcgctcggcccttccggctggctggtttattgctgataaatctggagccggtgagcgtgggtctcgcggtatcattgcagcactggggccagatggtaagccctcccgtatcgtagttatctacacgacggggagtcaggcaactatggatgaacgaaatagacagatcgctgagataggtgcctcactgattaagcattggtaactgtcagaccaagtttactcatatatactttagattgatttaaaacttcatttttaatttaaaaggatctaggtgaagatcctttttgataatctcatgaccaaaatcccttaacgtgagttttcgttccactgagcgtcagaccccgtagaaaagatcaaaggatcttcttgagatcctttttttctgcgcgtaatctgctgcttgcaaacaaaaaaaccaccgctaccagcggtggtttgtttgccggatcaagagctaccaactctttttccgaaggtaactggcttcagcagagcgcagataccaaatactgttcttctagtgtagccgtagttaggccaccacttcaagaactctgtagcaccgcctacatacctcgctctgctaatcctgttaccagtggctgctgccagtggcgataagtcgtgtcttaccgggttggactcaagacgatagttaccggataaggcgcagcggtcgggctgaacggggggttcgtgcacacagcccagcttggagcgaacgacctacaccgaactgagatacctacagcgtgagctatgagaaagcgccacgcttcccgaagggagaaaggcggacaggtatccggtaagcggcagggtcggaacaggagagcgcacgagggagcttccagggggaaacgcctggtatctttatagtcctgtcgggtttcgccacctctgacttgagcgtcgatttttgtgatgctcgtcaggggggcggagcctatggaaaaacgccagcaacgcggcctttttacggttcctggccttttgctggccttttgctcacatgttctttcctgcgttatcccctgattctgtggataaccgtattaccgcctttgagtgagctgataccgctcgccgcagccgaacgaccgagcgcagcgagtcagtgagcgaggaagcggaagagcgcccaatacgcaaaccgcctctccccgcgcgttggccgattcattaatgcagctggcacgacaggtttcccgactggaaagcgggcagtgagcgcaacgcaattaatgtgagttagctcactcattaggcaccccaggctttacactttatgcttccggctcgtatgttgtgtggaattgtgagcggataacaatttcacacaggaaacagctatgaccatgattacgccaagctttgctcttaggagtttcctaatacatcccaaactcaaatatataaagcatttgacttgttctatgccctagggggcggggggaagctaagccagctttttttaacatttaaaatgttaattccattttaaatgcacagatgtttttatttcataagggtttcaatgtgcatgaatgctgcaatattcctgttaccaaagctagtataaataaaaatagataaacgtggaaattacttagagtttctgtcattaacgtttccttcctcagttgacaacataaatgcgctgctgagcaagccagtttgcatctgtcaggatcaatttcccattatgccagtcatattaattactagtcaattagttgatttttatttttgacatatacatgtg

SEQ ID NO: 37 - DNA, 10244 bp, synthetic construct
  misc_feature 1..10244: note = hCD5-CAR
  source 1..10244: mol_type = other DNA
aatgaaagaccccacctgtaggtttggcaagctagcttaagtaacgccattttgcaaggcatggaaaaatacataactgagaatagaaaagttcagatcaaggtcaggaacagatggaacagctgaatatgggccaaacaggatatctgtggtaagcagttcctgccccggctcagggccaagaacagatggaacagctgaatatgggccaaacaggatatctgtggtaagcagttcctgccccggctcagggccaagaacagatggtccccagatgcggtccagccctcagcagtttctagagaaccatcagatgtttccagggtgccccaaggacctgaaatgaccctgtgccttatttgaactaaccaatcagttcgcttctcgcttctgttcgcgcgcttatgctccccgagctcaataaaagagcccacaacccctcactcggggcgccagtcctccgattgactgagtcgcccgggtacccgtgtatccaataaaccctcttgcagttgcatccgacttgtggtctcgctgttccttgggagggtctcctctgagtgattgactacccgtcagcgggggtctttcatttgggggctcgtccgggatcgggagacccctgcccagggaccaccgacccaccaccgggaggtaagctggccagcaacttatctgtgtctgtccgattgtctagtgtctatgactgattttatgcgcctgcgtcggtactagttagctaactagctctgtatctggcggacccgtggtggaactgacgagttcggaacacccggccgcaaccctgggagacgtcccagggacttcgggggccgtttttgtggcccgacctgagtcctaaaatcccgatcgtttaggactctttggtgcaccccccttagaggagggatatgtggttctggtaggagacgagaacctaaaacagttcccgcctccgtctgaatttttgctttcggtttgggaccgaagccgcgccgcgcgtcttgtctgctgcagcatcgttctgtgttgtctctgtctgactgtgtttctgtatttgtctgaaaatatgggcccgggctagcctgttaccactcccttaagtttgaccttaggtcactggaaagatgtcgagcggatcgctcacaaccagtcggtagatgtcaagaagagacgttgggttaccttctgctctgcagaatggccaacctttaacgtcggatggccgcgagacggcacctttaaccgagacctcatcacccaggttaagatcaaggtcttttcacctggcccgcatggacacccagaccaggtggggtacatcgtgacctgggaagccttggcttttgacccccctccctgggtcaagccctttgtacaccctaagcctccgcctcctcttcctccatccgccccgtctctcccccttgaacctcctcgttcgaccccgcctcgatcctccctttatccagccctcactccttctctaggcgcccccatatggccatatgagatcttatatggggcacccccgccccttgtaaacttccctgaccctgacatgacaagagttactaacagcccctctctccaagctcacttacaggctctctacttagtccagcacgaagtctggagacctctggcggcagcctaccaagaacaactggaccgaccggtggtacctcacccttaccgagtcggcgacacagtgtgggtccgccgacaccagactaagaacctagaacctcgctggaaaggaccttacacagtcctgctgaccacccccaccgccctcaaagtagacggcatcgcagcttggatacacgccgcccacgtgaaggctgccgaccccgggggtggaccatcctctagactgccatgctcgagggagtgcaggtggaaaccatctccccaggagacgggcgcaccttccccaagcgcggccagacctgcgtggtgcactacaccgggatgcttgaagatggaaagaaagttgattcctcccgggacagaaacaagccctttaagtttatgctaggcaagcaggaggtgatccgaggctgggaagaaggggttgcccagatgagtgtgggtcagagagccaaactgactatatctccagattatgcctatggtgccactgggcacccaggcatcatcccaccacatgccactctcgtcttcgatgtggagcttctaaaactggaatctggcggtggatccggagtcgacggatttggtgatgtcggtgctcttgagagtttgaggggaaatgcagatttggcttacatcctgagcatggagccctgtggccactgcctcattatcaacaatgtgaacttctgccgtgagtccgggctccgcacccgcactggctccaacatcgactgtgagaagttgcggcgtcgcttctcctcgctgcatttcatggtggaggtgaagggcgacctgactgccaagaaaatggtgctggctttgctggagctggcgcagcaggaccacggtgctctggactgctgcgtggtggtcattctctctcacggctgtcaggccagccacctgcagttcccaggggctgtctacggcacagatggatgccctgtgtcggtcgagaagattgtgaacatcttcaatgggaccagctgccccagcctgggagggaagcccaagctctttttcatccaggcctgtggtggggagcagaaagaccatgggtttgaggtggcctccacttcccctgaagacgagtcccctggcagtaaccccgagccagatgccaccccgttccaggaaggtttgaggaccttcgaccagctggacgccatatctagtttgcccacacccagtgacatctttgtgtcctactctactttcccaggttttgtttcctggagggaccccaagagtggctcctggtacgttgagaccctggacgacatctttgagcagtgggctcactctgaagacctgcagtccctcctgcttagggtcgctaatgctgtttcggtgaaagggatttataaacagatgcctggttgctttaatttcctccggaaaaaacttttctttaaaacatcagctagcagagccgagggcaggggaagtcttctaacatgcggggacgtggaggaaaatcccgggcccatggagttcggtctcagttggctgtttttggttgctatcttgaagggcgtccaatgcagccgggacatccagatgacccagtctccctctagcatgtcagcgagtcttggtgatcgagtgacgattacctgcagagcctctcaagatataaacagctatctttcatggttccaacagaagccggggaagtccccaaaaactctcatatacagggcgaatcgactcgtagacggtgtgccttcaaggttttccgggagtggtagtggcacagattacacacttacaatctcttcattgcagtatgaggatttcgggatctactactgtcaacagtacgacgaatccccatggacgtttgggggcgggaccaaacttgagataaaagggagcacatctggaagtggtaaacctgggtcaggggagggttccacaaaaggacaaattcaacttgtccaaagcggtcctggtcttaagaagcctggagggtctgtcaggataagttgtgcggcatccggctacaccttcaccaactatgggatgaactgggtgaaacaagcgcctgggaaaggtcttcgatggatgggctggattaatacccacactggagagcccacttacgctgatgatttcaaaggacgatttaccttctccttggatacttccaagagtaccgcgtacttgcaaatcaacagtctccgggctgaagacacggccacatacttctgtacgcggagagggtatgactggtattttgatgtgtggggtcagggaacaaccgtgactgtttcaagctacgtcaccgtctcttcacaggatcccgccgagcccaaatctcctgacaaaactcacacatgcccaccgtgcccagcacctgaactcctggggggaccgtcagtcttcctcttccccccaaaacccaaggacaccctcatgatctcccggacccctgaggtcacatgcgtggtggtggacgtgagccacgaagaccctgaggtcaagttcaactggtacgtggacggcgtggaggtgcataatgccaagacaaagccgcgggaggagcagtacaacagcacgtaccgtgtggtcagcgtcctcaccgtcctgcaccaggactggctgaatggcaaggagtacaagtgcaaggtctccaacaaagccctcccagcccccatcgagaaaaccatctccaaagccaaagggcagccccgagaaccacaggtgtacaccctgcccccatcccgggatgagctgaccaagaaccaggtcagcctgacctgcctggtcaaaggcttctatcccagcgacatcgccgtggagtgggagagcaatgggcaaccggagaacaactacaagaccacgcctcccgtgctggactccgacggctccttcttcctctacagcaagctcaccgtggacaagagcaggtggcagcaggggaacgtcttctcatgctccgtgatgcatgaggctctgcacaaccactacacgcagaagagcctctccctgtctccgggtaaaaaagatcccaaattttgggtgctggtggtggttggtggagtcctggcttgctatagcttgctagtaacagtggcctttattattttctgggtgaggagtaagaggagcaggctcctgcacagtgactacatgaacatgactccccgccgccccgggcccacccgcaagcattaccagccctatgccccaccacgcgacttcgcagcctatcgctccagagtgaagttcagcaggagcgcagacgcccccgcgtaccagcagggccagaaccagctctataacgagctcaatctaggacgaagagaggagtacgatgttttggacaagagacgtggccgggaccctgagatggggggaaagccgagaaggaagaaccctcaggaaggcctgtacaatgaactgcagaaagataagatggcggaggcctacagtgagattgggatgaaaggcgagcgccggaggggcaaggggcacgatggcctttaccagggtctcagtacagccaccaaggacacctacgacgcccttcacatgcaggccctgccccctcgcggaccgcagtgtactaattatgctctcttgaaattggctggagatgttgagagcaatcccgggcccatgcggatcagcaagccccacctgcggagcatcagcatccagtgctacctgtgcctgctgctgaacagccacttcctgaccgaggccggcatccacgtgttcatcctgggctgcttcagcgccggactgcccaagaccgaggccaactgggtgaacgtgatcagcgacctgaagaagatcgaggacctgatccagagcatgcacatcgacgccaccctgtacaccgagagcgacgtgcaccccagctgcaaggtgaccgccatgaagtgctttctgctggaactgcaggtgatcagcctggaaagcggcgacgccagcatccacgacaccgtggagaacctgatcatcctggccaacaacagcctgagcagcaacggcaacgtgaccgagagcggctgcaaagagtgcgaggaactggaagagaagaacatcaaagagtttctgcagagcttcgtgcacatcgtgcagatgttcatcaacaccagctgacgcgtcatcatcgatccggattagtccaatttgttaaagacaggatatcagtggtccaggctctagttttgactcaacaatatcaccagctgaagcctatagagtacgagccatagataaaataaaagattttatttagtctccagaaaaaggggggaatgaaagaccccacctgtaggtttggcaagctagcttaagtaacgccattttgcaaggcatggaaaaatacataactgagaatagagaagttcagatcaaggtcaggaacagatggaacagctgaatatgggccaaacaggatatctgtggtaagcagttcctgccccggctcagggccaagaacagatggaacagctgaatatgggccaaacaggatatctgtggtaagcagttcctgccccggctcagggccaagaacagatggtccccagatgcggtccagccctcagcagtttctagagaaccatcagatgtttccagggtgccccaaggacctgaaatgaccctgtgccttatttgaactaaccaatcagttcgcttctcgcttctgttcgcgcgcttctgctccccgagctcaataaaagagcccacaacccctcactcggggcgccagtcctccgattgactgagtcgcccgggtacccgtgtatccaataaaccctcttgcagttgcatccgacttgtggtctcgctgttccttgggagggtctcctctgagtgattgactacccgtcagcgggggtctttcacacatgcagcatgtatcaaaattaatttggttttttttcttaagtatttacattaaatggccatagtacttaaagttacattggcttccttgaaataaacatggagtattcagaatgtgtcataaatatttctaattttaagatagtatctccattggctttctactttttcttttatttttttttgtcctctgtcttccatttgttgttgttgttgtttgtttgtttgtttgttggttggttggttaatttttttttaaagatcctacactatagttcaagctagactattagctactctgtaacccagggtgaccttgaagtcatgggtagcctgctgttttagccttcccacatctaagattacaggtatgagctatcatttttggtatattgattgattgattgattgatgtgtgtgtgtgtgattgtgtttgtgtgtgtgactgtgaaaatgtgtgtatgggtgtgtgtgaatgtgtgtatgtatgtgtgtgtgtgagtgtgtgtgtgtgtgtgtgcatgtgtgtgtgtgtgactgtgtctatgtgtatgactgtgtgtgtgtgtgtgtgtgtgtgtgtgtgtgtgtgtgtgtgtgtgttgtgaaaaaatattctatggtagtgagagccaacgctccggctcaggtgtcaggttggtttttgagacagagtctttcacttagcttggaattcactggccgtcgttttacaacgtcgtgactgggaaaaccctggcgttacccaacttaatcgccttgcagcacatccccctttcgccagctggcgtaatagcgaagaggcccgcaccgatcgcccttcccaacagttgcgcagcctgaatggcgaatggcgcctgatgcggtattttctccttacgcatctgtgcggtatttcacaccgcatatggtgcactctcagtacaatctgctctgatgccgcatagttaagccagccccgacacccgccaacacccgctgacgcgccctgacgggcttgtctgctcccggcatccgcttacagacaagctgtgaccgtctccgggagctgcatgtgtcagaggttttcaccgtcatcaccgaaacgcgcgagacgaaagggcctcgtgatacgcctatttttataggttaatgtcatgataataatggtttcttagacgtcaggtggcacttttcggggaaatgtgcgcggaacccctatttgtttatttttctaaatacattcaaatatgtatccgctcatgagacaataaccctgataaatgcttcaataatattgaaaaaggaagagtatgagtattcaacatttccgtgtcgcccttattcccttttttgcggcattttgccttcctgtttttgctcacccagaaacgctggtgaaagtaaaagatgctgaagatcagttgggtgcacgagtgggttacatcgaactggatctcaacagcggtaagatccttgagagttttcgccccgaagaacgttttccaatgatgagcacttttaaagttctgctatgtggcgcggtattatcccgtattgacgccgggcaagagcaactcggtcgccgcatacactattctcagaatgacttggttgagtactcaccagtcacagaaaagcatcttacggatggcatgacagtaagagaattatgcagtgctgccataaccatgagtgataacactgcggccaacttacttctgacaacgatcggaggaccgaaggagctaaccgcttttttgcacaacatgggggatcatgtaactcgccttgatcgttgggaaccggagctgaatgaagccataccaaacgacgagcgtgacaccacgatgcctgtagcaatggcaacaacgttgcgcaaactattaactggcgaactacttactctagcttcccggcaacaattaatagactggatggaggcggataaagttgcaggaccacttctgcgctcggcccttccggctggctggtttattgctgataaatctggagccggtgagcgtgggtctcgcggtatcattgcagcactggggccagatggtaagccctcccgtatcgtagttatctacacgacggggagtcaggcaactatggatgaacgaaatagacagatcgctgagataggtgcctcactgattaagcattggtaactgtcagaccaagtttactcatatatactttagattgatttaaaacttcatttttaatttaaaaggatctaggtgaagatcctttttgataatctcatgaccaaaatcccttaacgtgagttttcgttccactgagcgtcagaccccgtagaaaagatcaaaggatcttcttgagatcctttttttctgcgcgtaatctgctgcttgcaaacaaaaaaaccaccgctaccagcggtggtttgtttgccggatcaagagctaccaactctttttccgaaggtaactggcttcagcagagcgcagataccaaatactgttcttctagtgtagccgtagttaggccaccacttcaagaactctgtagcaccgcctacatacctcgctctgctaatcctgttaccagtggctgctgccagtggcgataagtcgtgtcttaccgggttggactcaagacgatagttaccggataaggcgcagcggtcgggctgaacggggggttcgtgcacacagcccagcttggagcgaacgacctacaccgaactgagatacctacagcgtgagctatgagaaagcgccacgcttcccgaagggagaaaggcggacaggtatccggtaagcggcagggtcggaacaggagagcgcacgagggagcttccagggggaaacgcctggtatctttatagtcctgtcgggtttcgccacctctgacttgagcgtcgatttttgtgatgctcgtcaggggggcggagcctatggaaaaacgccagcaacgcggcctttttacggttcctggccttttgctggccttttgctcacatgttctttcctgcgttatcccctgattctgtggataaccgtattaccgcctttgagtgagctgataccgctcgccgcagccgaacgaccgagcgcagcgagtcagtgagcgaggaagcggaagagcgcccaatacgcaaaccgcctctccccgcgcgttggccgattcattaatgcagctggcacgacaggtttcccgactggaaagcgggcagtgagcgcaacgcaattaatgtgagttagctcactcattaggcaccccaggctttacactttatgcttccggctcgtatgttgtgtggaattgtgagcggataacaatttcacacaggaaacagctatgaccatgattacgccaagctttgctcttaggagtttcctaatacatcccaaactcaaatatataaagcatttgacttgttctatgccctagggggcggggggaagctaagccagctttttttaacatttaaaatgttaattccattttaaatgcacagatgtttttatttcataagggtttcaatgtgcatgaatgctgcaatattcctgttaccaaagctagtataaataaaaatagataaacgtggaaattacttagagtttctgtcattaacgtttccttcctcagttgacaacataaatgcgctgctgagcaagccagtttgcatctgtcaggatcaatttcccattatgccagtcatattaattactagtcaattagttgatttttatttttgacatatacatgtg

SEQ ID NO: 38 - DNA, 10625 bp, synthetic construct
  misc_feature 1..10625: note = pSFG4-CD19CAR-Ev3
  source 1..10625: mol_type = other DNA
aatgaaagaccccacctgtaggtttggcaagctagcttaagtaacgccattttgcaaggcatggaaaaatacataactgagaatagaaaagttcagatcaaggtcaggaacagatggaacagctgaatatgggccaaacaggatatctgtggtaagcagttcctgccccggctcagggccaagaacagatggaacagctgaatatgggccaaacaggatatctgtggtaagcagttcctgccccggctcagggccaagaacagatggtccccagatgcggtccagccctcagcagtttctagagaaccatcagatgtttccagggtgccccaaggacctgaaatgaccctgtgccttatttgaactaaccaatcagttcgcttctcgcttctgttcgcgcgcttatgctccccgagctcaataaaagagcccacaacccctcactcggggcgccagtcctccgattgactgagtcgcccgggtacccgtgtatccaataaaccctcttgcagttgcatccgacttgtggtctcgctgttccttgggagggtctcctctgagtgattgactacccgtcagcgggggtctttcatttgggggctcgtccgggatcgggagacccctgcccagggaccaccgacccaccaccgggaggtaagctggccagcaacttatctgtgtctgtccgattgtctagtgtctatgactgattttatgcgcctgcgtcggtactagttagctaactagctctgtatctggcggacccgtggtggaactgacgagttcggaacacccggccgcaaccctgggagacgtcccagggacttcgggggccgtttttgtggcccgacctgagtcctaaaatcccgatcgtttaggactctttggtgcaccccccttagaggagggatatgtggttctggtaggagacgagaacctaaaacagttcccgcctccgtctgaatttttgctttcggtttgggaccgaagccgcgccgcgcgtcttgtctgctgcagcatcgttctgtgttgtctctgtctgactgtgtttctgtatttgtctgaaaatatgggcccgggctagcctgttaccactcccttaagtttgaccttaggtcactggaaagatgtcgagcggatcgctcacaaccagtcggtagatgtcaagaagagacgttgggttaccttctgctctgcagaatggccaacctttaacgtcggatggccgcgagacggcacctttaaccgagacctcatcacccaggttaagatcaaggtcttttcacctggcccgcatggacacccagaccaggtggggtacatcgtgacctgggaagccttggcttttgacccccctccctgggtcaagccctttgtacaccctaagcctccgcctcctcttcctccatccgccccgtctctcccccttgaacctcctcgttcgaccccgcctcgatcctccctttatccagccctcactccttctctaggcgcccccatatggccatatgagatcttatatggggcacccccgccccttgtaaacttccctgaccctgacatgacaagagttactaacagcccctctctccaagctcacttacaggctctctacttagtccagcacgaagtctggagacctctggcggcagcctaccaagaacaactggaccgaccggtggtacctcacccttaccgagtcggcgacacagtgtgggtccgccgacaccagactaagaacctagaacctcgctggaaaggaccttacacagtcctgctgaccacccccaccgccctcaaagtagacggcatcgcagcttggatacacgccgcccacgtgaaggctgccgaccccgggggtggaccatcctctagactgccatgctcgagggagtgcaggtggaaaccatctccccaggagacgggcgcaccttccccaagcgcggccagacctgcgtggtgcactacaccgggatgcttgaagatggaaagaaagttgattcctcccgggacagaaacaagccctttaagtttatgctaggcaagcaggaggtgatccgaggctgggaagaaggggttgcccagatgagtgtgggtcagagagccaaactgactatatctccagattatgcctatggtgccactgggcacccaggcatcatcccaccacatgccactctcgtcttcgatgtggagcttctaaaactggaatctggcggtggatccggagtcgacggatttggtgatgtcggtgctcttgagagtttgaggggaaatgcagatttggcttacatcctgagcatggagccctgtggccactgcctcattatcaacaatgtgaacttctgccgtgagtccgggctccgcacccgcactggctccaacatcgactgtgagaagttgcggcgtcgcttctcctcgctgcatttcatggtggaggtgaagggcgacctgactgccaagaaaatggtgctggctttgctggagctggcgcagcaggaccacggtgctctggactgctgcgtggtggtcattctctctcacggctgtcaggccagccacctgcagttcccaggggctgtctacggcacagatggatgccctgtgtcggtcgagaagattgtgaacatcttcaatgggaccagctgccccagcctgggagggaagcccaagctctttttcatccaggcctgtggtggggagcagaaagaccatgggtttgaggtggcctccacttcccctgaagacgagtcccctggcagtaaccccgagccagatgccaccccgttccaggaaggtttgaggaccttcgaccagctggacgccatatctagtttgcccacacccagtgacatctttgtgtcctactctactttcccaggttttgtttcctggagggaccccaagagtggctcctggtacgttgagaccctggacgacatctttgagcagtgggctcactctgaagacctgcagtccctcctgcttagggtcgctaatgctgtttcggtgaaagggatttataaacagatgcctggttgctttaatttcctccggaaaaaacttttctttaaaacatcagctagcagagccgagggcaggggaagtcttctaacatgcggggacgtggaggaaaatcccgggcccatggagtttgggctgagctggctttttcttgtggctattttaaaaggtgtccagtgctctagagacatccagatgacacagactacatcctccctgtctgcctctctgggagacagagtcaccatcagttgcagggcaagtcaggacattagtaaatatttaaattggtatcagcagaaaccagatggaactgttaaactcctgatctaccatacatcaagattacactcaggagtcccatcaaggttcagtggcagtgggtctggaacagattattctctcaccattagcaacctggagcaagaagatattgccacttacttttgccaacagggtaatacgcttccgtacacgttcggaggggggaccaagctggagctgaaacgtggtggtggtggttctggtggtggtggttctggcggcggcggctccggtggtggtggatccgaggtgcagctgcagcagtctggacctggcctggtggcgccctcacagagcctgtccgtcacatgcactgtctcaggggtctcattacccgactatggtgtaagctggattcgccagcctccacgaaagggtctggagtggctgggagtaatatggggtagtgaaaccacatactataattcagctctcaaatccagactgaccatcatcaaggacaactccaagagccaagttttcttaaaaatgaacagtctgcaaactgatgacacagccatttactactgtgccaaacattattactacggtggtagctatgctatggactactggggccaagggaccacggtcaccgtctcctcgtacgtcaccgtctcttcacaggatcccgccctggaagagaagaaaggcaattacgtcgtgaccgaccacggcagctgtgtgcgggcttgtggcgccgatagctacgagatggaagaggacggcgtgcggaagtgcaagaagtgcgagggcccctgcagaaaagtgtgcaacggcatcggcatcggagagttcaaggatagcctgagcatcaacgccaccaacatcaagcacttcaagaactgcaccagcatcagcggcgacctgcacatcctgcccgtggcctttagaggcgacagcttcacccacacccccccactggatccccaggaactggacatcctgaaaaccgtgaaagagatcacaggctttctgctgattcaggcctggcccgagaaccggacagacctgcacgccttcgagaacctggaaatcatcagaggccggaccaagcagcacggccagttttctctggccgtggtgtccctgaacatcaccagcctgggcctgcggagcctgaaagaaatcagcgacggcgacgtgatcatctccggcaacaagaacctgtgctacgccaacaccatcaattggaagaagctgttcggcacctccggccagaaaacaaagatcatctctaaccggggcgagaacagctgcaaagccaccggacaagtgtgccacgccctgtgtagccctgagggctgttggggacccgagcccagagattgcgtgtcctgccggaatgtgtccagaggccgcgagtgcgtggacaagtgcaacctgctggaaggcgagccccgcgagtttgtggaaaacagcgagtgcatccagtgccaccccgagtgtctgccccaggccatgaacattacctgcaccggcagaggccccgacaactgtatccagtgcgcccactacatcgacggcccccactgcgtgaaaacctgtccagctggcgtgatgggagagaacaacaccctcgtgtggaagtacgccgacgccggccatgtgtgccacctgtgtcaccccaattgcacctacggctgtaccggccctggcctggaaggctgtcctaccaacggccccaagatcccttctaaagatcccaaattttgggtgctggtggtggttggtggagtcctggcttgctatagcttgctagtaacagtggcctttattattttctgggtgaggagtaagaggagcaggctcctgcacagtgactacatgaacatgactccccgccgccccgggcccacccgcaagcattaccagccctatgccccaccacgcgacttcgcagcctatcgctccagagtgaagttcagcaggagcgcagacgcccccgcgtaccagcagggccagaaccagctctataacgagctcaatctaggacgaagagaggagtacgatgttttggacaagagacgtggccgggaccctgagatggggggaaagccgagaaggaagaaccctcaggaaggcctgtacaatgaactgcagaaagataagatggcggaggcctacagtgagattgggatgaaaggcgagcgccggaggggcaaggggcacgatggcctttaccagggtctcagtacagccaccaaggacacctacgacgcccttcacatgcaggccctgccccctcgcggaccgcagtgtactaattatgctctcttgaaattggctggagatgttgagagcaatcccgggcccatgcggatcagcaagccccacctgcggagcatcagcatccagtgctacctgtgcctgctgctgaacagccacttcctgaccgaggccggcatccacgtgttcatcctgggctgcttcagcgccggactgcccaagaccgaggccaactgggtgaacgtgatcagcgacctgaagaagatcgaggacctgatccagagcatgcacatcgacgccaccctgtacaccgagagcgacgtgcaccccagctgcaaggtgaccgccatgaagtgctttctgctggaactgcaggtgatcagcctggaaagcggcgacgccagcatccacgacaccgtggagaacctgatcatcctggccaacaacagcctgagcagcaacggcaacgtgaccgagagcggctgcaaagagtgcgaggaactggaagagaagaacatcaaagagtttctgcagagcttcgtgcacatcgtgcagatgttcatcaacaccagctgacgcgtcatcatcgatccggattagtccaatttgttaaagacaggatatcagtggtccaggctctagttttgactcaacaatatcaccagctgaagcctatagagtacgagccatagataaaataaaagattttatttagtctccagaaaaaggggggaatgaaagaccccacctgtaggtttggcaagctagcttaagtaacgccattttgcaaggcatggaaaaatacataactgagaatagagaagttcagatcaaggtcaggaacagatggaacagctgaatatgggccaaacaggatatctgtggtaagcagttcctgccccggctcagggccaagaacagatggaacagctgaatatgggccaaacaggatatctgtggtaagcagttcctgccccggctcagggccaagaacagatggtccccagatgcggtccagccctcagcagtttctagagaaccatcagatgtttccagggtgccccaaggacctgaaatgaccctgtgccttatttgaactaaccaatcagttcgcttctcgcttctgttcgcgcgcttctgctccccgagctcaataaaagagcccacaacccctcactcggggcgccagtcctccgattgactgagtcgcccgggtacccgtgtatccaataaaccctcttgcagttgcatccgacttgtggtctcgctgttccttgggagggtctcctctgagtgattgactacccgtcagcgggggtctttcacacatgcagcatgtatcaaaattaatttggttttttttcttaagtatttacattaaatggccatagtacttaaagttacattggcttccttgaaataaacatggagtattcagaatgtgtcataaatatttctaattttaagatagtatctccattggctttctactttttcttttatttttttttgtcctctgtcttccatttgttgttgttgttgtttgtttgtttgtttgttggttggttggttaatttttttttaaagatcctacactatagttcaagctagactattagctactctgtaacccagggtgaccttgaagtcatgggtagcctgctgttttagccttcccacatctaagattacaggtatgagctatcatttttggtatattgattgattgattgattgatgtgtgtgtgtgtgattgtgtttgtgtgtgtgactgtgaaaatgtgtgtatgggtgtgtgtgaatgtgtgtatgtatgtgtgtgtgtgagtgtgtgtgtgtgtgtgtgcatgtgtgtgtgtgtgactgtgtctatgtgtatgactgtgtgtgtgtgtgtgtgtgtgtgtgtgtgtgtgtgtgtgtgtgtgttgtgaaaaaatattctatggtagtgagagccaacgctccggctcaggtgtcaggttggtttttgagacagagtctttcacttagcttggaattcactggccgtcgttttacaacgtcgtgactgggaaaaccctggcgttacccaacttaatcgccttgcagcacatccccctttcgccagctggcgtaatagcgaagaggcccgcaccgatcgcccttcccaacagttgcgcagcctgaatggcgaatggcgcctgatgcggtattttctccttacgcatctgtgcggtatttcacaccgcatatggtgcactctcagtacaatctgctctgatgccgcatagttaagccagccccgacacccgccaacacccgctgacgcgccctgacgggcttgtctgctcccggcatccgcttacagacaagctgtgaccgtctccgggagctgcatgtgtcagaggttttcaccgtcatcaccgaaacgcgcgagacgaaagggcctcgtgatacgcctatttttataggttaatgtcatgataataatggtttcttagacgtcaggtggcacttttcggggaaatgtgcgcggaacccctatttgtttatttttctaaatacattcaaatatgtatccgctcatgagacaataaccctgataaatgcttcaataatattgaaaaaggaagagtatgagtattcaacatttccgtgtcgcccttattcccttttttgcggcattttgccttcctgtttttgctcacccagaaacgctggtgaaagtaaaagatgctgaagatcagttgggtgcacgagtgggttacatcgaactggatctcaacagcggtaagatccttgagagttttcgccccgaagaacgttttccaatgatgagcacttttaaagttctgctatgtggcgcggtattatcccgtattgacgccgggcaagagcaactcggtcgccgcatacactattctcagaatgacttggttgagtactcaccagtcacagaaaagcatcttacggatggcatgacagtaagagaattatgcagtgctgccataaccatgagtgataacactgcggccaacttacttctgacaacgatcggaggaccgaaggagctaaccgcttttttgcacaacatgggggatcatgtaactcgccttgatcgttgggaaccggagctgaatgaagccataccaaacgacgagcgtgacaccacgatgcctgtagcaatggcaacaacgttgcgcaaactattaactggcgaactacttactctagcttcccggcaacaattaatagactggatggaggcggataaagttgcaggaccacttctgcgctcggcccttccggctggctggtttattgctgataaatctggagccggtgagcgtgggtctcgcggtatcattgcagcactggggccagatggtaagccctcccgtatcgtagttatctacacgacggggagtcaggcaactatggatgaacgaaatagacagatcgctgagataggtgcctcactgattaagcattggtaactgtcagaccaagtttactcatatatactttagattgatttaaaacttcatttttaatttaaaaggatctaggtgaagatcctttttgataatctcatgaccaaaatcccttaacgtgagttttcgttccactgagcgtcagaccccgtagaaaagatcaaaggatcttcttgagatcctttttttctgcgcgtaatctgctgcttgcaaacaaaaaaaccaccgctaccagcggtggtttgtttgccggatcaagagctaccaactctttttccgaaggtaactggcttcagcagagcgcagataccaaatactgttcttctagtgtagccgtagttaggccaccacttcaagaactctgtagcaccgcctacatacctcgctctgctaatcctgttaccagtggctgctgccagtggcgataagtcgtgtcttaccgggttggactcaagacgatagttaccggataaggcgcagcggtcgggctgaacggggggttcgtgcacacagcccagcttggagcgaacgacctacaccgaactgagatacctacagcgtgagctatgagaaagcgccacgcttcccgaagggagaaaggcggacaggtatccggtaagcggcagggtcggaacaggagagcgcacgagggagcttccagggggaaacgcctggtatctttatagtcctgtcgggtttcgccacctctgacttgagcgtcgatttttgtgatgctcgtcaggggggcggagcctatggaaaaacgccagcaacgcggcctttttacggttcctggccttttgctggccttttgctcacatgttctttcctgcgttatcccctgattctgtggataaccgtattaccgcctttgagtgagctgataccgctcgccgcagccgaacgaccgagcgcagcgagtcagtgagcgaggaagcggaagagcgcccaatacgcaaaccgcctctccccgcgcgttggccgattcattaatgcagctggcacgacaggtttcccgactggaaagcgggcagtgagcgcaacgcaattaatgtgagttagctcactcattaggcaccccaggctttacactttatgcttccggctcgtatgttgtgtggaattgtgagcggataacaatttcacacaggaaacagctatgaccatgattacgccaagctttgctcttaggagtttcctaatacatcccaaactcaaatatataaagcatttgacttgttctatgccctagggggcggggggaagctaagccagctttttttaacatttaaaatgttaattccattttaaatgcacagatgtttttatttcataagggtttcaatgtgcatgaatgctgcaatattcctgttaccaaagctagtataaataaaaatagataaacgtggaaattacttagagtttctgtcattaacgtttccttcctcagttgacaacataaatgcgctgctgagcaagccagtttgcatctgtcaggatcaatttcccattatgccagtcatattaattactagtcaattagttgatttttatttttgacatatacatgtg

SEQ ID NO: 39 - DNA, 10619 bp, synthetic construct
  misc_feature 1..10619: note = pSFG4-hCD19-Ev3-CAR
  source 1..10619: mol_type = other DNA
aatgaaagaccccacctgtaggtttggcaagctagcttaagtaacgccattttgcaaggcatggaaaaatacataactgagaatagaaaagttcagatcaaggtcaggaacagatggaacagctgaatatgggccaaacaggatatctgtggtaagcagttcctgccccggctcagggccaagaacagatggaacagctgaatatgggccaaacaggatatctgtggtaagcagttcctgccccggctcagggccaagaacagatggtccccagatgcggtccagccctcagcagtttctagagaaccatcagatgtttccagggtgccccaaggacctgaaatgaccctgtgccttatttgaactaaccaatcagttcgcttctcgcttctgttcgcgcgcttatgctccccgagctcaataaaagagcccacaacccctcactcggggcgccagtcctccgattgactgagtcgcccgggtacccgtgtatccaataaaccctcttgcagttgcatccgacttgtggtctcgctgttccttgggagggtctcctctgagtgattgactacccgtcagcgggggtctttcatttgggggctcgtccgggatcgggagacccctgcccagggaccaccgacccaccaccgggaggtaagctggccagcaacttatctgtgtctgtccgattgtctagtgtctatgactgattttatgcgcctgcgtcggtactagttagctaactagctctgtatctggcggacccgtggtggaactgacgagttcggaacacccggccgcaaccctgggagacgtcccagggacttcgggggccgtttttgtggcccgacctgagtcctaaaatcccgatcgtttaggactctttggtgcaccccccttagaggagggatatgtggttctggtaggagacgagaacctaaaacagttcccgcctccgtctgaatttttgctttcggtttgggaccgaagccgcgccgcgcgtcttgtctgctgcagcatcgttctgtgttgtctctgtctgactgtgtttctgtatttgtctgaaaatatgggcccgggctagcctgttaccactcccttaagtttgaccttaggtcactggaaagatgtcgagcggatcgctcacaaccagtcggtagatgtcaagaagagacgttgggttaccttctgctctgcagaatggccaacctttaacgtcggatggccgcgagacggcacctttaaccgagacctcatcacccaggttaagatcaaggtcttttcacctggcccgcatggacacccagaccaggtggggtacatcgtgacctgggaagccttggcttttgacccccctccctgggtcaagccctttgtacaccctaagcctccgcctcctcttcctccatccgccccgtctctcccccttgaacctcctcgttcgaccccgcctcgatcctccctttatccagccctcactccttctctaggcgcccccatatggccatatgagatcttatatggggcacccccgccccttgtaaacttccctgaccctgacatgacaagagttactaacagcccctctctccaagctcacttacaggctctctacttagtccagcacgaagtctggagacctctggcggcagcctaccaagaacaactggaccgaccggtggtacctcacccttaccgagtcggcgacacagtgtgggtccgccgacaccagactaagaacctagaacctcgctggaaaggaccttacacagtcctgctgaccacccccaccgccctcaaagtagacggcatcgcagcttggatacacgccgcccacgtgaaggctgccgaccccgggggtggaccatcctctagactgccatgctcgagggagtgcaggtggaaaccatctccccaggagacgggcgcaccttccccaagcgcggccagacctgcgtggtgcactacaccgggatgcttgaagatggaaagaaagttgattcctcccgggacagaaacaagccctttaagtttatgctaggcaagcaggaggtgatccgaggctgggaagaaggggttgcccagatgagtgtgggtcagagagccaaactgactatatctccagattatgcctatggtgccactgggcacccaggcatcatcccaccacatgccactctcgtcttcgatgtggagcttctaaaactggaatctggcggtggatccggagtcgacggatttggtgatgtcggtgctcttgagagtttgaggggaaatgcagatttggcttacatcctgagcatggagccctgtggccactgcctcattatcaacaatgtgaacttctgccgtgagtccgggctccgcacccgcactggctccaacatcgactgtgagaagttgcggcgtcgcttctcctcgctgcatttcatggtggaggtgaagggcgacctgactgccaagaaaatggtgctggctttgctggagctggcgcagcaggaccacggtgctctggactgctgcgtggtggtcattctctctcacggctgtcaggccagccacctgcagttcccaggggctgtctacggcacagatggatgccctgtgtcggtcgagaagattgtgaacatcttcaatgggaccagctgccccagcctgggagggaagcccaagctctttttcatccaggcctgtggtggggagcagaaagaccatgggtttgaggtggcctccacttcccctgaagacgagtcccctggcagtaaccccgagccagatgccaccccgttccaggaaggtttgaggaccttcgaccagctggacgccatatctagtttgcccacacccagtgacatctttgtgtcctactctactttcccaggttttgtttcctggagggaccccaagagtggctcctggtacgttgagaccctggacgacatctttgagcagtgggctcactctgaagacctgcagtccctcctgcttagggtcgctaatgctgtttcggtgaaagggatttataaacagatgcctggttgctttaatttcctccggaaaaaacttttctttaaaacatcagctagcagagccgagggcaggggaagtcttctaacatgcggggacgtggaggaaaatcccgggcccatggagttcggtttgagctggctctttcttgttgctatcctcaagggggtgcagtgttcaagggatatccagatgactcagagccctagctcccttagcgcgtccgtcggcgaccgggttacaattacttgtcgcgcatcacaagacataagtaaatacttgaactggtatcaacaaaagccaggaaaggttccaaaactcctcatctatcacacgagtagactccattccggggtccctgatcggttctcaggctctggttctggaactgacttcactctcacgatctctagtctgcaacctgaggatgtcgctacctattattgccaacagggaaacaccctcccttacacatttggccaaggtaccaaagttgagatcaagaggggctccacatctgggagcgggaaaccgggaagtggagaaggctcaaccaaaggtgaggtgcaacttgtagagagtggtggaggcctggttcagccgggagggtccctcagacttagttgcgcggcttctggcgtttcactgccggactacggggtcagttgggttaggcaggcgcctgggaaaggacttgagtggatcggcgtgatatggggtagtgaaacaacctactacaatagtgctcttaaatcaaaattcattatcagccgagacaatgctaagaactccctctatctccaaatgaatagtcttagagcagaagacacagccgtttattactgtgcccgccattattactatgggggcagctacgcaatggattattggggccaagggaccctggtcacggtatcaagctacgtcaccgtctcttcacaggatcccgccctggaagagaagaaaggcaattacgtcgtgaccgaccacggcagctgtgtgcgggcttgtggcgccgatagctacgagatggaagaggacggcgtgcggaagtgcaagaagtgcgagggcccctgcagaaaagtgtgcaacggcatcggcatcggagagttcaaggatagcctgagcatcaacgccaccaacatcaagcacttcaagaactgcaccagcatcagcggcgacctgcacatcctgcccgtggcctttagaggcgacagcttcacccacacccccccactggatccccaggaactggacatcctgaaaaccgtgaaagagatcacaggctttctgctgattcaggcctggcccgagaaccggacagacctgcacgccttcgagaacctggaaatcatcagaggccggaccaagcagcacggccagttttctctggccgtggtgtccctgaacatcaccagcctgggcctgcggagcctgaaagaaatcagcgacggcgacgtgatcatctccggcaacaagaacctgtgctacgccaacaccatcaattggaagaagctgttcggcacctccggccagaaaacaaagatcatctctaaccggggcgagaacagctgcaaagccaccggacaagtgtgccacgccctgtgtagccctgagggctgttggggacccgagcccagagattgcgtgtcctgccggaatgtgtccagaggccgcgagtgcgtggacaagtgcaacctgctggaaggcgagccccgcgagtttgtggaaaacagcgagtgcatccagtgccaccccgagtgtctgccccaggccatgaacattacctgcaccggcagaggccccgacaactgtatccagtgcgcccactacatcgacggcccccactgcgtgaaaacctgtccagctggcgtgatgggagagaacaacaccctcgtgtggaagtacgccgacgccggccatgtgtgccacctgtgtcaccccaattgcacctacggctgtaccggccctggcctggaaggctgtcctaccaacggccccaagatcccttctaaagatcccaaattttgggtgctggtggtggttggtggagtcctggcttgctatagcttgctagtaacagtggcctttattattttctgggtgaggagtaagaggagcaggctcctgcacagtgactacatgaacatgactccccgccgccccgggcccacccgcaagcattaccagccctatgccccaccacgcgacttcgcagcctatcgctccagagtgaagttcagcaggagcgcagacgcccccgcgtaccagcagggccagaaccagctctataacgagctcaatctaggacgaagagaggagtacgatgttttggacaagagacgtggccgggaccctgagatggggggaaagccgagaaggaagaaccctcaggaaggcctgtacaatgaactgcagaaagataagatggcggaggcctacagtgagattgggatgaaaggcgagcgccggaggggcaaggggcacgatggcctttaccagggtctcagtacagccaccaaggacacctacgacgcccttcacatgcaggccctgccccctcgcggaccgcagtgtactaattatgctctcttgaaattggctggagatgttgagagcaatcccgggcccatgcggatcagcaagccccacctgcggagcatcagcatccagtgctacctgtgcctgctgctgaacagccacttcctgaccgaggccggcatccacgtgttcatcctgggctgcttcagcgccggactgcccaagaccgaggccaactgggtgaacgtgatcagcgacctgaagaagatcgaggacctgatccagagcatgcacatcgacgccaccctgtacaccgagagcgacgtgcaccccagctgcaaggtgaccgccatgaagtgctttctgctggaactgcaggtgatcagcctggaaagcggcgacgccagcatccacgacaccgtggagaacctgatcatcctggccaacaacagcctgagcagcaacggcaacgtgaccgagagcggctgcaaagagtgcgaggaactggaagagaagaacatcaaagagtttctgcagagcttcgtgcacatcgtgcagatgttcatcaacaccagctgacgcgtcatcatcgatccggattagtccaatttgttaaagacaggatatcagtggtccaggctctagttttgactcaacaatatcaccagctgaagcctatagagtacgagccatagataaaataaaagattttatttagtctccagaaaaaggggggaatgaaagaccccacctgtaggtttggcaagctagcttaagtaacgccattttgcaaggcatggaaaaatacataactgagaatagagaagttcagatcaaggtcaggaacagatggaacagctgaatatgggccaaacaggatatctgtggtaagcagttcctgccccggctcagggccaagaacagatggaacagctgaatatgggccaaacaggatatctgtggtaagcagttcctgccccggctcagggccaagaacagatggtccccagatgcggtccagccctcagcagtttctagagaaccatcagatgtttccagggtgccccaaggacctgaaatgaccctgtgccttatttgaactaaccaatcagttcgcttctcgcttctgttcgcgcgcttctgctccccgagctcaataaaagagcccacaacccctcactcggggcgccagtcctccgattgactgagtcgcccgggtacccgtgtatccaataaaccctcttgcagttgcatccgacttgtggtctcgctgttccttgggagggtctcctctgagtgattgactacccgtcagcgggggtctttcacacatgcagcatgtatcaaaattaatttggttttttttcttaagtatttacattaaatggccatagtacttaaagttacattggcttccttgaaataaacatggagtattcagaatgtgtcataaatatttctaattttaagatagtatctccattggctttctactttttcttttatttttttttgtcctctgtcttccatttgttgttgttgttgtttgtttgtttgtttgttggttggttggttaatttttttttaaagatcctacactatagttcaagctagactattagctactctgtaacccagggtgaccttgaagtcatgggtagcctgctgttttagccttcccacatctaagattacaggtatgagctatcatttttggtatattgattgattgattgattgatgtgtgtgtgtgtgattgtgtttgtgtgtgtgactgtgaaaatgtgtgtatgggtgtgtgtgaatgtgtgtatgtatgtgtgtgtgtgagtgtgtgtgtgtgtgtgtgcatgtgtgtgtgtgtgactgtgtctatgtgtatgactgtgtgtgtgtgtgtgtgtgtgtgtgtgtgtgtgtgtgtgtgtgtgttgtgaaaaaatattctatggtagtgagagccaacgctccggctcaggtgtcaggttggtttttgagacagagtctttcacttagcttggaattcactggccgtcgttttacaacgtcgtgactgggaaaaccctggcgttacccaacttaatcgccttgcagcacatccccctttcgccagctggcgtaatagcgaagaggcccgcaccgatcgcccttcccaacagttgcgcagcctgaatggcgaatggcgcctgatgcggtattttctccttacgcatctgtgcggtatttcacaccgcatatggtgcactctcagtacaatctgctctgatgccgcatagttaagccagccccgacacccgccaacacccgctgacgcgccctgacgggcttgtctgctcccggcatccgcttacagacaagctgtgaccgtctccgggagctgcatgtgtcagaggttttcaccgtcatcaccgaaacgcgcgagacgaaagggcctcgtgatacgcctatttttataggttaatgtcatgataataatggtttcttagacgtcaggtggcacttttcggggaaatgtgcgcggaacccctatttgtttatttttctaaatacattcaaatatgtatccgctcatgagacaataaccctgataaatgcttcaataatattgaaaaaggaagagtatgagtattcaacatttccgtgtcgcccttattcccttttttgcggcattttgccttcctgtttttgctcacccagaaacgctggtgaaagtaaaagatgctgaagatcagttgggtgcacgagtgggttacatcgaactggatctcaacagcggtaagatccttgagagttttcgccccgaagaacgttttccaatgatgagcacttttaaagttctgctatgtggcgcggtattatcccgtattgacgccgggcaagagcaactcggtcgccgcatacactattctcagaatgacttggttgagtactcaccagtcacagaaaagcatcttacggatggcatgacagtaagagaattatgcagtgctgccataaccatgagtgataacactgcggccaacttacttctgacaacgatcggaggaccgaaggagctaaccgcttttttgcacaacatgggggatcatgtaactcgccttgatcgttgggaaccggagctgaatgaagccataccaaacgacgagcgtgacaccacgatgcctgtagcaatggcaacaacgttgcgcaaactattaactggcgaactacttactctagcttcccggcaacaattaatagactggatggaggcggataaagttgcaggaccacttctgcgctcggcccttccggctggctggtttattgctgataaatctggagccggtgagcgtgggtctcgcggtatcattgcagcactggggccagatggtaagccctcccgtatcgtagttatctacacgacggggagtcaggcaactatggatgaacgaaatagacagatcgctgagataggtgcctcactgattaagcattggtaactgtcagaccaagtttactcatatatactttagattgatttaaaacttcatttttaatttaaaaggatctaggtgaagatcctttttgataatctcatgaccaaaatcccttaacgtgagttttcgttccactgagcgtcagaccccgtagaaaagatcaaaggatcttcttgagatcctttttttctgcgcgtaatctgctgcttgcaaacaaaaaaaccaccgctaccagcggtggtttgtttgccggatcaagagctaccaactctttttccgaaggtaactggcttcagcagagcgcagataccaaatactgttcttctagtgtagccgtagttaggccaccacttcaagaactctgtagcaccgcctacatacctcgctctgctaatcctgttaccagtggctgctgccagtggcgataagtcgtgtcttaccgggttggactcaagacgatagttaccggataaggcgcagcggtcgggctgaacggggggttcgtgcacacagcccagcttggagcgaacgacctacaccgaactgagatacctacagcgtgagctatgagaaagcgccacgcttcccgaagggagaaaggcggacaggtatccggtaagcggcagggtcggaacaggagagcgcacgagggagcttccagggggaaacgcctggtatctttatagtcctgtcgggtttcgccacctctgacttgagcgtcgatttttgtgatgctcgtcaggggggcggagcctatggaaaaacgccagcaacgcggcctttttacggttcctggccttttgctggccttttgctcacatgttctttcctgcgttatcccctgattctgtggataaccgtattaccgcctttgagtgagctgataccgctcgccgcagccgaacgaccgagcgcagcgagtcagtgagcgaggaagcggaagagcgcccaatacgcaaaccgcctctccccgcgcgttggccgattcattaatgcagctggcacgacaggtttcccgactggaaagcgggcagtgagcgcaacgcaattaatgtgagttagctcactcattaggcaccccaggctttacactttatgcttccggctcgtatgttgtgtggaattgtgagcggataacaatttcacacaggaaacagctatgaccatgattacgccaagctttgctcttaggagtttcctaatacatcccaaactcaaatatataaagcatttgacttgttctatgccctagggggcggggggaagctaagccagctttttttaacatttaaaatgttaattccattttaaatgcacagatgtttttatttcataagggtttcaatgtgcatgaatgctgcaatattcctgttaccaaagctagtataaataaaaatagataaacgtggaaattacttagagtttctgtcattaacgtttccttcctcagttgacaacataaatgcgctgctgagcaagccagtttgcatctgtcaggatcaatttcccattatgccagtcatattaattactagtcaattagttgatttttatttttgacatatacatgtg

SEQ ID NO: 40 - DNA, 10604 bp, synthetic construct
  misc_feature 1..10604: note = pSFG4-CD123-Ev3-CAR
  source 1..10604: mol_type = other DNA
aatgaaagaccccacctgtaggtttggcaagctagcttaagtaacgccattttgcaaggcatggaaaaatacataactgagaatagaaaagttcagatcaaggtcaggaacagatggaacagctgaatatgggccaaacaggatatctgtggtaagcagttcctgccccggctcagggccaagaacagatggaacagctgaatatgggccaaacaggatatctgtggtaagcagttcctgccccggctcagggccaagaacagatggtccccagatgcggtccagccctcagcagtttctagagaaccatcagatgtttccagggtgccccaaggacctgaaatgaccctgtgccttatttgaactaaccaatcagttcgcttctcgcttctgttcgcgcgcttatgctccccgagctcaataaaagagcccacaacccctcactcggggcgccagtcctccgattgactgagtcgcccgggtacccgtgtatccaataaaccctcttgcagttgcatccgacttgtggtctcgctgttccttgggagggtctcctctgagtgattgactacccgtcagcgggggtctttcatttgggggctcgtccgggatcgggagacccctgcccagggaccaccgacccaccaccgggaggtaagctggccagcaacttatctgtgtctgtccgattgtctagtgtctatgactgattttatgcgcctgcgtcggtactagttagctaactagctctgtatctggcggacccgtggtggaactgacgagttcggaacacccggccgcaaccctgggagacgtcccagggacttcgggggccgtttttgtggcccgacctgagtcctaaaatcccgatcgtttaggactctttggtgcaccccccttagaggagggatatgtggttctggtaggagacgagaacctaaaacagttcccgcctccgtctgaatttttgctttcggtttgggaccgaagccgcgccgcgcgtcttgtctgctgcagcatcgttctgtgttgtctctgtctgactgtgtttctgtatttgtctgaaaatatgggcccgggctagcctgttaccactcccttaagtttgaccttaggtcactggaaagatgtcgagcggatcgctcacaaccagtcggtagatgtcaagaagagacgttgggttaccttctgctctgcagaatggccaacctttaacgtcggatggccgcgagacggcacctttaaccgagacctcatcacccaggttaagatcaaggtcttttcacctggcccgcatggacacccagaccaggtggggtacatcgtgacctgggaagccttggcttttgacccccctccctgggtcaagccctttgtacaccctaagcctccgcctcctcttcctccatccgccccgtctctcccccttgaacctcctcgttcgaccccgcctcgatcctccctttatccagccctcactccttctctaggcgcccccatatggccatatgagatcttatatggggcacccccgccccttgtaaacttccctgaccctgacatgacaagagttactaacagcccctctctccaagctcacttacaggctctctacttagtccagcacgaagtctggagacctctggcggcagcctaccaagaacaactggaccgaccggtggtacctcacccttaccgagtcggcgacacagtgtgggtccgccgacaccagactaagaacctagaacctcgctggaaaggaccttacacagtcctgctgaccacccccaccgccctcaaagtagacggcatcgcagcttggatacacgccgcccacgtgaaggctgccgaccccgggggtggaccatcctctagactgccatgctcgagggagtgcaggtggaaaccatctccccaggagacgggcgcaccttccccaagcgcggccagacctgcgtggtgcactacaccgggatgcttgaagatggaaagaaagttgattcctcccgggacagaaacaagccctttaagtttatgctaggcaagcaggaggtgatccgaggctgggaagaaggggttgcccagatgagtgtgggtcagagagccaaactgactatatctccagattatgcctatggtgccactgggcacccaggcatcatcccaccacatgccactctcgtcttcgatgtggagcttctaaaactggaatctggcggtggatccggagtcgacggatttggtgatgtcggtgctcttgagagtttgaggggaaatgcagatttggcttacatcctgagcatggagccctgtggccactgcctcattatcaacaatgtgaacttctgccgtgagtccgggctccgcacccgcactggctccaacatcgactgtgagaagttgcggcgtcgcttctcctcgctgcatttcatggtggaggtgaagggcgacctgactgccaagaaaatggtgctggctttgctggagctggcgcagcaggaccacggtgctctggactgctgcgtggtggtcattctctctcacggctgtcaggccagccacctgcagttcccaggggctgtctacggcacagatggatgccctgtgtcggtcgagaagattgtgaacatcttcaatgggaccagctgccccagcctgggagggaagcccaagctctttttcatccaggcctgtggtggggagcagaaagaccatgggtttgaggtggcctccacttcccctgaagacgagtcccctggcagtaaccccgagccagatgccaccccgttccaggaaggtttgaggaccttcgaccagctggacgccatatctagtttgcccacacccagtgacatctttgtgtcctactctactttcccaggttttgtttcctggagggaccccaagagtggctcctggtacgttgagaccctggacgacatctttgagcagtgggctcactctgaagacctgcagtccctcctgcttagggtcgctaatgctgtttcggtgaaagggatttataaacagatgcctggttgctttaatttcctccggaaaaaacttttctttaaaacatcagctagcagagccgagggcaggggaagtcttctaacatgcggggacgtggaggaaaatcccgggcccatggagtttggactgtcatggctttttctggttgctatattgaaaggtgtccaatgcagtagagacgtacaaataactcaatcccctagttacttggctgcgtcaccaggagagaccataacaattaactgtagagcgagcaaatctattagcaaggaccttgcatggtaccaggaaaagcccggaaaaacgaataaacttcttatatactctggctcaactttgcaaagtggaattccgtcaagatttagtggtagcgggtctggaaccgacttcacattgactataagttccttggagccggaggattttgcgatgtattattgccagcaacataataaatatccctatactttcgggggaggaactaaattggagataaagggttcaacttctgggtctggtaaacctggcagcggcgaaggtagcacaaaagggcaagtccaactccagcagcccggcgcggaactcgtgcgacctggcgcttcagttaagctgagctgcaaggcctcaggatacaccttcacaagctactggatgaattgggtgaagcagaggcctgatcaaggactcgaatggataggtagaattgatccctacgactccgagacgcattataaccagaaatttaaggataaggcgattcttaccgtggacaaaagttcttcaacggcatatatgcaactgagcagtttgacatcagaagacagtgctgtttattactgcgcgagaggtaactgggatgactactggggccagggcactaccttggttaccgtgtcaagctacgtcaccgtctcttcacaggatcccgccctggaagagaagaaaggcaattacgtcgtgaccgaccacggcagctgtgtgcgggcttgtggcgccgatagctacgagatggaagaggacggcgtgcggaagtgcaagaagtgcgagggcccctgcagaaaagtgtgcaacggcatcggcatcggagagttcaaggatagcctgagcatcaacgccaccaacatcaagcacttcaagaactgcaccagcatcagcggcgacctgcacatcctgcccgtggcctttagaggcgacagcttcacccacacccccccactggatccccaggaactggacatcctgaaaaccgtgaaagagatcacaggctttctgctgattcaggcctggcccgagaaccggacagacctgcacgccttcgagaacctggaaatcatcagaggccggaccaagcagcacggccagttttctctggccgtggtgtccctgaacatcaccagcctgggcctgcggagcctgaaagaaatcagcgacggcgacgtgatcatctccggcaacaagaacctgtgctacgccaacaccatcaattggaagaagctgttcggcacctccggccagaaaacaaagatcatctctaaccggggcgagaacagctgcaaagccaccggacaagtgtgccacgccctgtgtagccctgagggctgttggggacccgagcccagagattgcgtgtcctgccggaatgtgtccagaggccgcgagtgcgtggacaagtgcaacctgctggaaggcgagccccgcgagtttgtggaaaacagcgagtgcatccagtgccaccccgagtgtctgccccaggccatgaacattacctgcaccggcagaggccccgacaactgtatccagtgcgcccactacatcgacggcccccactgcgtgaaaacctgtccagctggcgtgatgggagagaacaacaccctcgtgtggaagtacgccgacgccggccatgtgtgccacctgtgtcaccccaattgcacctacggctgtaccggccctggcctggaaggctgtcctaccaacggccccaagatcccttctaaagatcccaaattttgggtgctggtggtggttggtggagtcctggcttgctatagcttgctagtaacagtggcctttattattttctgggtgaggagtaagaggagcaggctcctgcacagtgactacatgaacatgactccccgccgccccgggcccacccgcaagcattaccagccctatgccccaccacgcgacttcgcagcctatcgctccagagtgaagttcagcaggagcgcagacgcccccgcgtaccagcagggccagaaccagctctataacgagctcaatctaggacgaagagaggagtacgatgttttggacaagagacgtggccgggaccctgagatggggggaaagccgagaaggaagaaccctcaggaaggcctgtacaatgaactgcagaaagataagatggcggaggcctacagtgagattgggatgaaaggcgagcgccggaggggcaaggggcacgatggcctttaccagggtctcagtacagccaccaaggacacctacgacgcccttcacatgcaggccctgccccctcgcggaccgcagtgtactaattatgctctcttgaaattggctggagatgttgagagcaatcccgggcccatgcggatcagcaagccccacctgcggagcatcagcatccagtgctacctgtgcctgctgctgaacagccacttcctgaccgaggccggcatccacgtgttcatcctgggctgcttcagcgccggactgcccaagaccgaggccaactgggtgaacgtgatcagcgacctgaagaagatcgaggacctgatccagagcatgcacatcgacgccaccctgtacaccgagagcgacgtgcaccccagctgcaaggtgaccgccatgaagtgctttctgctggaactgcaggtgatcagcctggaaagcggcgacgccagcatccacgacaccgtggagaacctgatcatcctggccaacaacagcctgagcagcaacggcaacgtgaccgagagcggctgcaaagagtgcgaggaactggaagagaagaacatcaaagagtttctgcagagcttcgtgcacatcgtgcagatgttcatcaacaccagctgacgcgtcatcatcgatccggattagtccaatttgttaaagacaggatatcagtggtccaggctctagttttgactcaacaatatcaccagctgaagcctatagagtacgagccatagataaaataaaagattttatttagtctccagaaaaaggggggaatgaaagaccccacctgtaggtttggcaagctagcttaagtaacgccattttgcaaggcatggaaaaatacataactgagaatagagaagttcagatcaaggtcaggaacagatggaacagctgaatatgggccaaacaggatatctgtggtaagcagttcctgccccggctcagggccaagaacagatggaacagctgaatatgggccaaacaggatatctgtggtaagcagttcctgccccggctcagggccaagaacagatggtccccagatgcggtccagccctcagcagtttctagagaaccatcagatgtttccagggtgccccaaggacctgaaatgaccctgtgccttatttgaactaaccaatcagttcgcttctcgcttctgttcgcgcgcttctgctccccgagctcaataaaagagcccacaacccctcactcggggcgccagtcctccgattgactgagtcgcccgggtacccgtgtatccaataaaccctcttgcagttgcatccgacttgtggtctcgctgttccttgggagggtctcctctgagtgattgactacccgtcagcgggggtctttcacacatgcagcatgtatcaaaattaatttggttttttttcttaagtatttacattaaatggccatagtacttaaagttacattggcttccttgaaataaacatggagtattcagaatgtgtcataaatatttctaattttaagatagtatctccattggctttctactttttcttttatttttttttgtcctctgtcttccatttgttgttgttgttgtttgtttgtttgtttgttggttggttggttaatttttttttaaagatcctacactatagttcaagctagactattagctactctgtaacccagggtgaccttgaagtcatgggtagcctgctgttttagccttcccacatctaagattacaggtatgagctatcatttttggtatattgattgattgattgattgatgtgtgtgtgtgtgattgtgtttgtgtgtgtgactgtgaaaatgtgtgtatgggtgtgtgtgaatgtgtgtatgtatgtgtgtgtgtgagtgtgtgtgtgtgtgtgtgcatgtgtgtgtgtgtgactgtgtctatgtgtatgactgtgtgtgtgtgtgtgtgtgtgtgtgtgtgtgtgtgtgtgtgtgtgttgtgaaaaaatattctatggtagtgagagccaacgctccggctcaggtgtcaggttggtttttgagacagagtctttcacttagcttggaattcactggccgtcgttttacaacgtcgtgactgggaaaaccctggcgttacccaacttaatcgccttgcagcacatccccctttcgccagctggcgtaatagcgaagaggcccgcaccgatcgcccttcccaacagttgcgcagcctgaatggcgaatggcgcctgatgcggtattttctccttacgcatctgtgcggtatttcacaccgcatatggtgcactctcagtacaatctgctctgatgccgcatagttaagccagccccgacacccgccaacacccgctgacgcgccctgacgggcttgtctgctcccggcatccgcttacagacaagctgtgaccgtctccgggagctgcatgtgtcagaggttttcaccgtcatcaccgaaacgcgcgagacgaaagggcctcgtgatacgcctatttttataggttaatgtcatgataataatggtttcttagacgtcaggtggcacttttcggggaaatgtgcgcggaacccctatttgtttatttttctaaatacattcaaatatgtatccgctcatgagacaataaccctgataaatgcttcaataatattgaaaaaggaagagtatgagtattcaacatttccgtgtcgcccttattcccttttttgcggcattttgccttcctgtttttgctcacccagaaacgctggtgaaagtaaaagatgctgaagatcagttgggtgcacgagtgggttacatcgaactggatctcaacagcggtaagatccttgagagttttcgccccgaagaacgttttccaatgatgagcacttttaaagttctgctatgtggcgcggtattatcccgtattgacgccgggcaagagcaactcggtcgccgcatacactattctcagaatgacttggttgagtactcaccagtcacagaaaagcatcttacggatggcatgacagtaagagaattatgcagtgctgccataaccatgagtgataacactgcggccaacttacttctgacaacgatcggaggaccgaaggagctaaccgcttttttgcacaacatgggggatcatgtaactcgccttgatcgttgggaaccggagctgaatgaagccataccaaacgacgagcgtgacaccacgatgcctgtagcaatggcaacaacgttgcgcaaactattaactggcgaactacttactctagcttcccggcaacaattaatagactggatggaggcggataaagttgcaggaccacttctgcgctcggcccttccggctggctggtttattgctgataaatctggagccggtgagcgtgggtctcgcggtatcattgcagcactggggccagatggtaagccctcccgtatcgtagttatctacacgacggggagtcaggcaactatggatgaacgaaatagacagatcgctgagataggtgcctcactgattaagcattggtaactgtcagaccaagtttactcatatatactttagattgatttaaaacttcatttttaatttaaaaggatctaggtgaagatcctttttgataatctcatgaccaaaatcccttaacgtgagttttcgttccactgagcgtcagaccccgtagaaaagatcaaaggatcttcttgagatcctttttttctgcgcgtaatctgctgcttgcaaacaaaaaaaccaccgctaccagcggtggtttgtttgccggatcaagagctaccaactctttttccgaaggtaactggcttcagcagagcgcagataccaaatactgttcttctagtgtagccgtagttaggccaccacttcaagaactctgtagcaccgcctacatacctcgctctgctaatcctgttaccagtggctgctgccagtggcgataagtcgtgtcttaccgggttggactcaagacgatagttaccggataaggcgcagcggtcgggctgaacggggggttcgtgcacacagcccagcttggagcgaacgacctacaccgaactgagatacctacagcgtgagctatgagaaagcgccacgcttcccgaagggagaaaggcggacaggtatccggtaagcggcagggtcggaacaggagagcgcacgagggagcttccagggggaaacgcctggtatctttatagtcctgtcgggtttcgccacctctgacttgagcgtcgatttttgtgatgctcgtcaggggggcggagcctatggaaaaacgccagcaacgcggcctttttacggttcctggccttttgctggccttttgctcacatgttctttcctgcgttatcccctgattctgtggataaccgtattaccgcctttgagtgagctgataccgctcgccgcagccgaacgaccgagcgcagcgagtcagtgagcgaggaagcggaagagcgcccaatacgcaaaccgcctctccccgcgcgttggccgattcattaatgcagctggcacgacaggtttcccgactggaaagcgggcagtgagcgcaacgcaattaatgtgagttagctcactcattaggcaccccaggctttacactttatgcttccggctcgtatgttgtgtggaattgtgagcggataacaatttcacacaggaaacagctatgaccatgattacgccaagctttgctcttaggagtttcctaatacatcccaaactcaaatatataaagcatttgacttgttctatgccctagggggcggggggaagctaagccagctttttttaacatttaaaatgttaattccattttaaatgcacagatgtttttatttcataagggtttcaatgtgcatgaatgctgcaatattcctgttaccaaagctagtataaataaaaatagataaacgtggaaattacttagagtttctgtcattaacgtttccttcctcagttgacaacataaatgcgctgctgagcaagccagtttgcatctgtcaggatcaatttcccattatgccagtcatattaattactagtcaattagttgatttttatttttgacatatacatgtg

SEQ ID NO: 41 - DNA, 10604 bp, synthetic construct
  misc_feature 1..10604: note = pSFG4-hCD123-Ev3-CAR
  source 1..10604: mol_type = other DNA
aatgaaagaccccacctgtaggtttggcaagctagcttaagtaacgccattttgcaaggcatggaaaaatacataactgagaatagaaaagttcagatcaaggtcaggaacagatggaacagctgaatatgggccaaacaggatatctgtggtaagcagttcctgccccggctcagggccaagaacagatggaacagctgaatatgggccaaacaggatatctgtggtaagcagttcctgccccggctcagggccaagaacagatggtccccagatgcggtccagccctcagcagtttctagagaaccatcagatgtttccagggtgccccaaggacctgaaatgaccctgtgccttatttgaactaaccaatcagttcgcttctcgcttctgttcgcgcgcttatgctccccgagctcaataaaagagcccacaacccctcactcggggcgccagtcctccgattgactgagtcgcccgggtacccgtgtatccaataaaccctcttgcagttgcatccgacttgtggtctcgctgttccttgggagggtctcctctgagtgattgactacccgtcagcgggggtctttcatttgggggctcgtccgggatcgggagacccctgcccagggaccaccgacccaccaccgggaggtaagctggccagcaacttatctgtgtctgtccgattgtctagtgtctatgactgattttatgcgcctgcgtcggtactagttagctaactagctctgtatctggcggacccgtggtggaactgacgagttcggaacacccggccgcaaccctgggagacgtcccagggacttcgggggccgtttttgtggcccgacctgagtcctaaaatcccgatcgtttaggactctttggtgcaccccccttagaggagggatatgtggttctggtaggagacgagaacctaaaacagttcccgcctccgtctgaatttttgctttcggtttgggaccgaagccgcgccgcgcgtcttgtctgctgcagcatcgttctgtgttgtctctgtctgactgtgtttctgtatttgtctgaaaatatgggcccgggctagcctgttaccactcccttaagtttgaccttaggtcactggaaagatgtcgagcggatcgctcacaaccagtcggtagatgtcaagaagagacgttgggttaccttctgctctgcagaatggccaacctttaacgtcggatggccgcgagacggcacctttaaccgagacctcatcacccaggttaagatcaaggtcttttcacctggcccgcatggacacccagaccaggtggggtacatcgtgacctgggaagccttggcttttgacccccctccctgggtcaagccctttgtacaccctaagcctccgcctcctcttcctccatccgccccgtctctcccccttgaacctcctcgttcgaccccgcctcgatcctccctttatccagccctcactccttctctaggcgcccccatatggccatatgagatcttatatggggcacccccgccccttgtaaacttccctgaccctgacatgacaagagttactaacagcccctctctccaagctcacttacaggctctctacttagtccagcacgaagtctggagacctctggcggcagcctaccaagaacaactggaccgaccggtggtacctcacccttaccgagtcggcgacacagtgtgggtccgccgacaccagactaagaacctagaacctcgctggaaaggaccttacacagtcctgctgaccacccccaccgccctcaaagtagacggcatcgcagcttggatacacgccgcccacgtgaaggctgccgaccccgggggtggaccatcctctagactgccatgctcgagggagtgcaggtggaaaccatctccccaggagacgggcgcaccttccccaagcgcggccagacctgcgtggtgcactacaccgggatgcttgaagatggaaagaaagttgattcctcccgggacagaaacaagccctttaagtttatgctaggcaagcaggaggtgatccgaggctgggaagaaggggttgcccagatgagtgtgggtcagagagccaaactgactatatctccagattatgcctatggtgccactgggcacccaggcatcatcccaccacatgccactctcgtcttcgatgtggagcttctaaaactggaatctggcggtggatccggagtcgacggatttggtgatgtcggtgctcttgagagtttgaggggaaatgcagatttggcttacatcctgagcatggagccctgtggccactgcctcattatcaacaatgtgaacttctgccgtgagtccgggctccgcacccgcactggctccaacatcgactgtgagaagttgcggcgtcgcttctcctcgctgcatttcatggtggaggtgaagggcgacctgactgccaagaaaatggtgctggctttgctggagctggcgcagcaggaccacggtgctctggactgctgcgtggtggtcattctctctcacggctgtcaggccagccacctgcagttcccaggggctgtctacggcacagatggatgccctgtgtcggtcgagaagattgtgaacatcttcaatgggaccagctgccccagcctgggagggaagcccaagctctttttcatccaggcctgtggtggggagcagaaagaccatgggtttgaggtggcctccacttcccctgaagacgagtcccctggcagtaaccccgagccagatgccaccccgttccaggaaggtttgaggaccttcgaccagctggacgccatatctagtttgcccacacccagtgacatctttgtgtcctactctactttcccaggttttgtttcctggagggaccccaagagtggctcctggtacgttgagaccctggacgacatctttgagcagtgggctcactctgaagacctgcagtccctcctgcttagggtcgctaatgctgtttcggtgaaagggatttataaacagatgcctggttgctttaatttcctccggaaaaaacttttctttaaaacatcagctagcagagccgagggcaggggaagtcttctaacatgcggggacgtggaggaaaatcccgggcccatggaattcgggctttcatggttgttcctcgttgcgatacttaaaggcgttcagtgcagtagagacattcagatgacccaaagccctagtagcctctccgccagtgtgggtgaccgcgtgactattacgtgccgagcaagcaagagtattagcaaagatttggcatggtaccagcagaaaccaggcaaggtccctaagttgcttatatatagcgggtctacactccaatctggagtgccggatcgcttctcaggttccggatcaggaaccgatttcactcttacaatttcctctctgcaaccggaggacgtggcaacatactattgccagcagcataacaaatatccctatactttcggtcaaggtacaaaagtagaaataaaacgaggttccacctccgggagtgggaagcccggctccggcgaaggatccaccaaaggcgaggtacagctcgttgaaagcgggggcggtctcgtccaaccaggagggtctcttcgactttcttgtgctgcaagtgggtacacgtttacttcctattggatgaattgggttcggcaagcccccggtaaagggcttgaatggatagggaggatagacccctacgattctgagacgcattataatcagaaattcaaagataagttcataataagcagagacaatgcaaaaaatagtttgtacctccagatgaatagtcttcgggcagaagacacagcggtatattactgtgctcggggtaactgggatgattactggggtcagggaactctggttactgtgtctagctacgtcaccgtctcttcacaggatcccgccctggaagagaagaaaggcaattacgtcgtgaccgaccacggcagctgtgtgcgggcttgtggcgccgatagctacgagatggaagaggacggcgtgcggaagtgcaagaagtgcgagggcccctgcagaaaagtgtgcaacggcatcggcatcggagagttcaaggatagcctgagcatcaacgccaccaacatcaagcacttcaagaactgcaccagcatcagcggcgacctgcacatcctgcccgtggcctttagaggcgacagcttcacccacacccccccactggatccccaggaactggacatcctgaaaaccgtgaaagagatcacaggctttctgctgattcaggcctggcccgagaaccggacagacctgcacgccttcgagaacctggaaatcatcagaggccggaccaagcagcacggccagttttctctggccgtggtgtccctgaacatcaccagcctgggcctgcggagcctgaaagaaatcagcgacggcgacgtgatcatctccggcaacaagaacctgtgctacgccaacaccatcaattggaagaagctgttcggcacctccggccagaaaacaaagatcatctctaaccggggcgagaacagctgcaaagccaccggacaagtgtgccacgccctgtgtagccctgagggctgttggggacccgagcccagagattgcgtgtcctgccggaatgtgtccagaggccgcgagtgcgtggacaagtgcaacctgctggaaggcgagccccgcgagtttgtggaaaacagcgagtgcatccagtgccaccccgagtgtctgccccaggccatgaacattacctgcaccggcagaggccccgacaactgtatccagtgcgcccactacatcgacggcccccactgcgtgaaaacctgtccagctggcgtgatgggagagaacaacaccctcgtgtggaagtacgccgacgccggccatgtgtgccacctgtgtcaccccaattgcacctacggctgtaccggccctggcctggaaggctgtcctaccaacggccccaagatcccttctaaagatcccaaattttgggtgctggtggtggttggtggagtcctggcttgctatagcttgctagtaacagtggcctttattattttctgggtgaggagtaagaggagcaggctcctgcacagtgactacatgaacatgactccccgccgccccgggcccacccgcaagcattaccagccctatgccccaccacgcgacttcgcagcctatcgctccagagtgaagttcagcaggagcgcagacgcccccgcgtaccagcagggccagaaccagctctataacgagctcaatctaggacgaagagaggagtacgatgttttggacaagagacgtggccgggaccctgagatggggggaaagccgagaaggaagaaccctcaggaaggcctgtacaatgaactgcagaaagataagatggcggaggcctacagtgagattgggatgaaaggcgagcgccggaggggcaaggggcacgatggcctttaccagggtctcagtacagccaccaaggacacctacgacgcccttcacatgcaggccctgccccctcgcggaccgcagtgtactaattatgctctcttgaaattggctggagatgttgagagcaatcccgggcccatgcggatcagcaagccccacctgcggagcatcagcatccagtgctacctgtgcctgctgctgaacagccacttcctgaccgaggccggcatccacgtgttcatcctgggctgcttcagcgccggactgcccaagaccgaggccaactgggtgaacgtgatcagcgacctgaagaagatcgaggacctgatccagagcatgcacatcgacgccaccctgtacaccgagagcgacgtgcaccccagctgcaaggtgaccgccatgaagtgctttctgctggaactgcaggtgatcagcctggaaagcggcgacgccagcatccacgacaccgtggagaacctgatcatcctggccaacaacagcctgagcagcaacggcaacgtgaccgagagcggctgcaaagagtgcgaggaactggaagagaagaacatcaaagagtttctgcagagcttcgtgcacatcgtgcagatgttcatcaacaccagctgacgcgtcatcatcgatccggattagtccaatttgttaaagacaggatatcagtggtccaggctctagttttgactcaacaatatcaccagctgaagcctatagagtacgagccatagataaaataaaagattttatttagtctccagaaaaaggggggaatgaaagaccccacctgtaggtttggcaagctagcttaagtaacgccattttgcaaggcatggaaaaatacataactgagaatagagaagttcagatcaaggtcaggaacagatggaacagctgaatatgggccaaacaggatatctgtggtaagcagttcctgccccggctcagggccaagaacagatggaacagctgaatatgggccaaacaggatatctgtggtaagcagttcctgccccggctcagggccaagaacagatggtccccagatgcggtccagccctcagcagtttctagagaaccatcagatgtttccagggtgccccaaggacctgaaatgaccctgtgccttatttgaactaaccaatcagttcgcttctcgcttctgttcgcgcgcttctgctccccgagctcaataaaagagcccacaacccctcactcggggcgccagtcctccgattgactgagtcgcccgggtacccgtgtatccaataaaccctcttgcagttgcatccgacttgtggtctcgctgttccttgggagggtctcctctgagtgattgactacccgtcagcgggggtctttcacacatgcagcatgtatcaaaattaatttggttttttttcttaagtatttacattaaatggccatagtacttaaagttacattggcttccttgaaataaacatggagtattcagaatgtgtcataaatatttctaattttaagatagtatctccattggctttctactttttcttttatttttttttgtcctctgtcttccatttgttgttgttgttgtttgtttgtttgtttgttggttggttggttaatttttttttaaagatcctacactatagttcaagctagactattagctactctgtaacccagggtgaccttgaagtcatgggtagcctgctgttttagccttcccacatctaagattacaggtatgagctatcatttttggtatattgattgattgattgattgatgtgtgtgtgtgtgattgtgtttgtgtgtgtgactgtgaaaatgtgtgtatgggtgtgtgtgaatgtgtgtatgtatgtgtgtgtgtgagtgtgtgtgtgtgtgtgtgcatgtgtgtgtgtgtgactgtgtctatgtgtatgactgtgtgtgtgtgtgtgtgtgtgtgtgtgtgtgtgtgtgtgtgtgtgttgtgaaaaaatattctatggtagtgagagccaacgctccggctcaggtgtcaggttggtttttgagacagagtctttcacttagcttggaattcactggccgtcgttttacaacgtcgtgactgggaaaaccctggcgttacccaacttaatcgccttgcagcacatccccctttcgccagctggcgtaatagcgaagaggcccgcaccgatcgcccttcccaacagttgcgcagcctgaatggcgaatggcgcctgatgcggtattttctccttacgcatctgtgcggtatttcacaccgcatatggtgcactctcagtacaatctgctctgatgccgcatagttaagccagccccgacacccgccaacacccgctgacgcgccctgacgggcttgtctgctcccggcatccgcttacagacaagctgtgaccgtctccgggagctgcatgtgtcagaggttttcaccgtcatcaccgaaacgcgcgagacgaaagggcctcgtgatacgcctatttttataggttaatgtcatgataataatggtttcttagacgtcaggtggcacttttcggggaaatgtgcgcggaacccctatttgtttatttttctaaatacattcaaatatgtatccgctcatgagacaataaccctgataaatgcttcaataatattgaaaaaggaagagtatgagtattcaacatttccgtgtcgcccttattcccttttttgcggcattttgccttcctgtttttgctcacccagaaacgctggtgaaagtaaaagatgctgaagatcagttgggtgcacgagtgggttacatcgaactggatctcaacagcggtaagatccttgagagttttcgccccgaagaacgttttccaatgatgagcacttttaaagttctgctatgtggcgcggtattatcccgtattgacgccgggcaagagcaactcggtcgccgcatacactattctcagaatgacttggttgagtactcaccagtcacagaaaagcatcttacggatggcatgacagtaagagaattatgcagtgctgccataaccatgagtgataacactgcggccaacttacttctgacaacgatcggaggaccgaaggagctaaccgcttttttgcacaacatgggggatcatgtaactcgccttgatcgttgggaaccggagctgaatgaagccataccaaacgacgagcgtgacaccacgatgcctgtagcaatggcaacaacgttgcgcaaactattaactggcgaactacttactctagcttcccggcaacaattaatagactggatggaggcggataaagttgcaggaccacttctgcgctcggcccttccggctggctggtttattgctgataaatctggagccggtgagcgtgggtctcgcggtatcattgcagcactggggccagatggtaagccctcccgtatcgtagttatctacacgacggggagtcaggcaactatggatgaacgaaatagacagatcgctgagataggtgcctcactgattaagcattggtaactgtcagaccaagtttactcatatatactttagattgatttaaaacttcatttttaatttaaaaggatctaggtgaagatcctttttgataatctcatgaccaaaatcccttaacgtgagttttcgttccactgagcgtcagaccccgtagaaaagatcaaaggatcttcttgagatcctttttttctgcgcgtaatctgctgcttgcaaacaaaaaaaccaccgctaccagcggtggtttgtttgccggatcaagagctaccaactctttttccgaaggtaactggcttcagcagagcgcagataccaaatactgttcttctagtgtagccgtagttaggccaccacttcaagaactctgtagcaccgcctacatacctcgctctgctaatcctgttaccagtggctgctgccagtggcgataagtcgtgtcttaccgggttggactcaagacgatagttaccggataaggcgcagcggtcgggctgaacggggggttcgtgcacacagcccagcttggagcgaacgacctacaccgaactgagatacctacagcgtgagctatgagaaagcgccacgcttcccgaagggagaaaggcggacaggtatccggtaagcggcagggtcggaacaggagagcgcacgagggagcttccagggggaaacgcctggtatctttatagtcctgtcgggtttcgccacctctgacttgagcgtcgatttttgtgatgctcgtcaggggggcggagcctatggaaaaacgccagcaacgcggcctttttacggttcctggccttttgctggccttttgctcacatgttctttcctgcgttatcccctgattctgtggataaccgtattaccgcctttgagtgagctgataccgctcgccgcagccgaacgaccgagcgcagcgagtcagtgagcgaggaagcggaagagcgcccaatacgcaaaccgcctctccccgcgcgttggccgattcattaatgcagctggcacgacaggtttcccgactggaaagcgggcagtgagcgcaacgcaattaatgtgagttagctcactcattaggcaccccaggctttacactttatgcttccggctcgtatgttgtgtggaattgtgagcggataacaatttcacacaggaaacagctatgaccatgattacgccaagctttgctcttaggagtttcctaatacatcccaaactcaaatatataaagcatttgacttgttctatgccctagggggcggggggaagctaagccagctttttttaacatttaaaatgttaattccattttaaatgcacagatgtttttatttcataagggtttcaatgtgcatgaatgctgcaatattcctgttaccaaagctagtataaataaaaatagataaacgtggaaattacttagagtttctgtcattaacgtttccttcctcagttgacaacataaatgcgctgctgagcaagccagtttgcatctgtcaggatcaatttcccattatgccagtcatattaattactagtcaattagttgatttttatttttgacatatacatgtg

SEQ ID NO: 42 - DNA, 10610 bp, synthetic construct
  misc_feature 1..10610: note = pSFG4-Meso-Ev3-CAR
  source 1..10610: mol_type = other DNA
aatgaaagaccccacctgtaggtttggcaagctagcttaagtaacgccattttgcaaggcatggaaaaatacataactgagaatagaaaagttcagatcaaggtcaggaacagatggaacagctgaatatgggccaaacaggatatctgtggtaagcagttcctgccccggctcagggccaagaacagatggaacagctgaatatgggccaaacaggatatctgtggtaagcagttcctgccccggctcagggccaagaacagatggtccccagatgcggtccagccctcagcagtttctagagaaccatcagatgtttccagggtgccccaaggacctgaaatgaccctgtgccttatttgaactaaccaatcagttcgcttctcgcttctgttcgcgcgcttatgctccccgagctcaataaaagagcccacaacccctcactcggggcgccagtcctccgattgactgagtcgcccgggtacccgtgtatccaataaaccctcttgcagttgcatccgacttgtggtctcgctgttccttgggagggtctcctctgagtgattgactacccgtcagcgggggtctttcatttgggggctcgtccgggatcgggagacccctgcccagggaccaccgacccaccaccgggaggtaagctggccagcaacttatctgtgtctgtccgattgtctagtgtctatgactgattttatgcgcctgcgtcggtactagttagctaactagctctgtatctggcggacccgtggtggaactgacgagttcggaacacccggccgcaaccctgggagacgtcccagggacttcgggggccgtttttgtggcccgacctgagtcctaaaatcccgatcgtttaggactctttggtgcaccccccttagaggagggatatgtggttctggtaggagacgagaacctaaaacagttcccgcctccgtctgaatttttgctttcggtttgggaccgaagccgcgccgcgcgtcttgtctgctgcagcatcgttctgtgttgtctctgtctgactgtgtttctgtatttgtctgaaaatatgggcccgggctagcctgttaccactcccttaagtttgaccttaggtcactggaaagatgtcgagcggatcgctcacaaccagtcggtagatgtcaagaagagacgttgggttaccttctgctctgcagaatggccaacctttaacgtcggatggccgcgagacggcacctttaaccgagacctcatcacccaggttaagatcaaggtcttttcacctggcccgcatggacacccagaccaggtggggtacatcgtgacctgggaagccttggcttttgacccccctccctgggtcaagccctttgtacaccctaagcctccgcctcctcttcctccatccgccccgtctctcccccttgaacctcctcgttcgaccccgcctcgatcctccctttatccagccctcactccttctctaggcgcccccatatggccatatgagatcttatatggggcacccccgccccttgtaaacttccctgaccctgacatgacaagagttactaacagcccctctctccaagctcacttacaggctctctacttagtccagcacgaagtctggagacctctggcggcagcctaccaagaacaactggaccgaccggtggtacctcacccttaccgagtcggcgacacagtgtgggtccgccgacaccagactaagaacctagaacctcgctggaaaggaccttacacagtcctgctgaccacccccaccgccctcaaagtagacggcatcgcagcttggatacacgccgcccacgtgaaggctgccgaccccgggggtggaccatcctctagactgccatgctcgagggagtgcaggtggaaaccatctccccaggagacgggcgcaccttccccaagcgcggccagacctgcgtggtgcactacaccgggatgcttgaagatggaaagaaagttgattcctcccgggacagaaacaagccctttaagtttatgctaggcaagcaggaggtgatccgaggctgggaagaaggggttgcccagatgagtgtgggtcagagagccaaactgactatatctccagattatgcctatggtgccactgggcacccaggcatcatcccaccacatgccactctcgtcttcgatgtggagcttctaaaactggaatctggcggtggatccggagtcgacggatttggtgatgtcggtgctcttgagagtttgaggggaaatgcagatttggcttacatcctgagcatggagccctgtggccactgcctcattatcaacaatgtgaacttctgccgtgagtccgggctccgcacccgcactggctccaacatcgactgtgagaagttgcggcgtcgcttctcctcgctgcatttcatggtggaggtgaagggcgacctgactgccaagaaaatggtgctggctttgctggagctggcgcagcaggaccacggtgctctggactgctgcgtggtggtcattctctctcacggctgtcaggccagccacctgcagttcccaggggctgtctacggcacagatggatgccctgtgtcggtcgagaagattgtgaacatcttcaatgggaccagctgccccagcctgggagggaagcccaagctctttttcatccaggcctgtggtggggagcagaaagaccatgggtttgaggtggcctccacttcccctgaagacgagtcccctggcagtaaccccgagccagatgccaccccgttccaggaaggtttgaggaccttcgaccagctggacgccatatctagtttgcccacacccagtgacatctttgtgtcctactctactttcccaggttttgtttcctggagggaccccaagagtggctcctggtacgttgagaccctggacgacatctttgagcagtgggctcactctgaagacctgcagtccctcctgcttagggtcgctaatgctgtttcggtgaaagggatttataaacagatgcctggttgctttaatttcctccggaaaaaacttttctttaaaacatcagctagcagagccgagggcaggggaagtcttctaacatgcggggacgtggaggaaaatcccgggcccatggagttcggccttagctggctgttccttgtggccatactcaagggcgtccagtgtagtcgcgatatagagctgacgcaaagcccggcaattatgtcagcaagtccaggagaaaaggtgactatgacttgttccgcaagcagttctgtaagttacatgcactggtaccagcaaaaaagtggaactagccctaagcggtggatctatgacacgtctaaattggcctctggtgtccccggacgattttcaggttcaggaagtggaaacagttactctcttactataagtagcgtcgaggcggaggatgacgccacctactactgccagcagtggagcgggtaccccctcaccttcggggccgggaccaagttggagattaaaggatcaacatccgggagcggaaagccggggtcaggtgagggctcaacaaaagggcaggtacagctccagcaaagtgggcccgagctggaaaaaccgggtgcgagtgtcaaactttcttgtaaggccagcggttactctttcacgggttatacaatgaattgggtgaaacagtcccacggcaagagcctcgaatggataggtctcatcacaccatacaacggagcttcctcctataatcagaagttccggggaaaggcaaccctcactgtagacaagtcttcctcaacagcatatatggatctcctgtcactcacgtccgaagacagcgcggtttatttttgtgcgagagggggttatgacgggcgcgggttcgactactggggtcaaggcactacagtaacggtaagcagctacgtcaccgtctcttcacaggatcccgccctggaagagaagaaaggcaattacgtcgtgaccgaccacggcagctgtgtgcgggcttgtggcgccgatagctacgagatggaagaggacggcgtgcggaagtgcaagaagtgcgagggcccctgcagaaaagtgtgcaacggcatcggcatcggagagttcaaggatagcctgagcatcaacgccaccaacatcaagcacttcaagaactgcaccagcatcagcggcgacctgcacatcctgcccgtggcctttagaggcgacagcttcacccacacccccccactggatccccaggaactggacatcctgaaaaccgtgaaagagatcacaggctttctgctgattcaggcctggcccgagaaccggacagacctgcacgccttcgagaacctggaaatcatcagaggccggaccaagcagcacggccagttttctctggccgtggtgtccctgaacatcaccagcctgggcctgcggagcctgaaagaaatcagcgacggcgacgtgatcatctccggcaacaagaacctgtgctacgccaacaccatcaattggaagaagctgttcggcacctccggccagaaaacaaagatcatctctaaccggggcgagaacagctgcaaagccaccggacaagtgtgccacgccctgtgtagccctgagggctgttggggacccgagcccagagattgcgtgtcctgccggaatgtgtccagaggccgcgagtgcgtggacaagtgcaacctgctggaaggcgagccccgcgagtttgtggaaaacagcgagtgcatccagtgccaccccgagtgtctgccccaggccatgaacattacctgcaccggcagaggccccgacaactgtatccagtgcgcccactacatcgacggcccccactgcgtgaaaacctgtccagctggcgtgatgggagagaacaacaccctcgtgtggaagtacgccgacgccggccatgtgtgccacctgtgtcaccccaattgcacctacggctgtaccggccctggcctggaaggctgtcctaccaacggccccaagatcccttctaaagatcccaaattttgggtgctggtggtggttggtggagtcctggcttgctatagcttgctagtaacagtggcctttattattttctgggtgaggagtaagaggagcaggctcctgcacagtgactacatgaacatgactccccgccgccccgggcccacccgcaagcattaccagccctatgccccaccacgcgacttcgcagcctatcgctccagagtgaagttcagcaggagcgcagacgcccccgcgtaccagcagggccagaaccagctctataacgagctcaatctaggacgaagagaggagtacgatgttttggacaagagacgtggccgggaccctgagatggggggaaagccgagaaggaagaaccctcaggaaggcctgtacaatgaactgcagaaagataagatggcggaggcctacagtgagattgggatgaaaggcgagcgccggaggggcaaggggcacgatggcctttaccagggtctcagtacagccaccaaggacacctacgacgcccttcacatgcaggccctgccccctcgcggaccgcagtgtactaattatgctctcttgaaattggctggagatgttgagagcaatcccgggcccatgcggatcagcaagccccacctgcggagcatcagcatccagtgctacctgtgcctgctgctgaacagccacttcctgaccgaggccggcatccacgtgttcatcctgggctgcttcagcgccggactgcccaagaccgaggccaactgggtgaacgtgatcagcgacctgaagaagatcgaggacctgatccagagcatgcacatcgacgccaccctgtacaccgagagcgacgtgcaccccagctgcaaggtgaccgccatgaagtgctttctgctggaactgcaggtgatcagcctggaaagcggcgacgccagcatccacgacaccgtggagaacctgatcatcctggccaacaacagcctgagcagcaacggcaacgtgaccgagagcggctgcaaagagtgcgaggaactggaagagaagaacatcaaagagtttctgcagagcttcgtgcacatcgtgcagatgttcatcaacaccagctgacgcgtcatcatcgatccggattagtccaatttgttaaagacaggatatcagtggtccaggctctagttttgactcaacaatatcaccagctgaagcctatagagtacgagccatagataaaataaaagattttatttagtctccagaaaaaggggggaatgaaagaccccacctgtaggtttggcaagctagcttaagtaacgccattttgcaaggcatggaaaaatacataactgagaatagagaagttcagatcaaggtcaggaacagatggaacagctgaatatgggccaaacaggatatctgtggtaagcagttcctgccccggctcagggccaagaacagatggaacagctgaatatgggccaaacaggatatctgtggtaagcagttcctgccccggctcagggccaagaacagatggtccccagatgcggtccagccctcagcagtttctagagaaccatcagatgtttccagggtgccccaaggacctgaaatgaccctgtgccttatttgaactaaccaatcagttcgcttctcgcttctgttcgcgcgcttctgctccccgagctcaataaaagagcccacaacccctcactcggggcgccagtcctccgattgactgagtcgcccgggtacccgtgtatccaataaaccctcttgcagttgcatccgacttgtggtctcgctgttccttgggagggtctcctctgagtgattgactacccgtcagcgggggtctttcacacatgcagcatgtatcaaaattaatttggttttttttcttaagtatttacattaaatggccatagtacttaaagttacattggcttccttgaaataaacatggagtattcagaatgtgtcataaatatttctaattttaagatagtatctccattggctttctactttttcttttatttttttttgtcctctgtcttccatttgttgttgttgttgtttgtttgtttgtttgttggttggttggttaatttttttttaaagatcctacactatagttcaagctagactattagctactctgtaacccagggtgaccttgaagtcatgggtagcctgctgttttagccttcccacatctaagattacaggtatgagctatcatttttggtatattgattgattgattgattgatgtgtgtgtgtgtgattgtgtttgtgtgtgtgactgtgaaaatgtgtgtatgggtgtgtgtgaatgtgtgtatgtatgtgtgtgtgtgagtgtgtgtgtgtgtgtgtgcatgtgtgtgtgtgtgactgtgtctatgtgtatgactgtgtgtgtgtgtgtgtgtgtgtgtgtgtgtgtgtgtgtgtgtgtgttgtgaaaaaatattctatggtagtgagagccaacgctccggctcaggtgtcaggttggtttttgagacagagtctttcacttagcttggaattcactggccgtcgttttacaacgtcgtgactgggaaaaccctggcgttacccaacttaatcgccttgcagcacatccccctttcgccagctggcgtaatagcgaagaggcccgcaccgatcgcccttcccaacagttgcgcagcctgaatggcgaatggcgcctgatgcggtattttctccttacgcatctgtgcggtatttcacaccgcatatggtgcactctcagtacaatctgctctgatgccgcatagttaagccagccccgacacccgccaacacccgctgacgcgccctgacgggcttgtctgctcccggcatccgcttacagacaagctgtgaccgtctccgggagctgcatgtgtcagaggttttcaccgtcatcaccgaaacgcgcgagacgaaagggcctcgtgatacgcctatttttataggttaatgtcatgataataatggtttcttagacgtcaggtggcacttttcggggaaatgtgcgcggaacccctatttgtttatttttctaaatacattcaaatatgtatccgctcatgagacaataaccctgataaatgcttcaataatattgaaaaaggaagagtatgagtattcaacatttccgtgtcgcccttattcccttttttgcggcattttgccttcctgtttttgctcacccagaaacgctggtgaaagtaaaagatgctgaagatcagttgggtgcacgagtgggttacatcgaactggatctcaacagcggtaagatccttgagagttttcgccccgaagaacgttttccaatgatgagcacttttaaagttctgctatgtggcgcggtattatcccgtattgacgccgggcaagagcaactcggtcgccgcatacactattctcagaatgacttggttgagtactcaccagtcacagaaaagcatcttacggatggcatgacagtaagagaattatgcagtgctgccataaccatgagtgataacactgcggccaacttacttctgacaacgatcggaggaccgaaggagctaaccgcttttttgcacaacatgggggatcatgtaactcgccttgatcgttgggaaccggagctgaatgaagccataccaaacgacgagcgtgacaccacgatgcctgtagcaatggcaacaacgttgcgcaaactattaactggcgaactacttactctagcttcccggcaacaattaatagactggatggaggcggataaagttgcaggaccacttctgcgctcggcccttccggctggctggtttattgctgataaatctggagccggtgagcgtgggtctcgcggtatcattgcagcactggggccagatggtaagccctcccgtatcgtagttatctacacgacggggagtcaggcaactatggatgaacgaaatagacagatcgctgagataggtgcctcactgattaagcattggtaactgtcagaccaagtttactcatatatactttagattgatttaaaacttcatttttaatttaaaaggatctaggtgaagatcctttttgataatctcatgaccaaaatcccttaacgtgagttttcgttccactgagcgtcagaccccgtagaaaagatcaaaggatcttcttgagatcctttttttctgcgcgtaatctgctgcttgcaaacaaaaaaaccaccgctaccagcggtggtttgtttgccggatcaagagctaccaactctttttccgaaggtaactggcttcagcagagcgcagataccaaatactgttcttctagtgtagccgtagttaggccaccacttcaagaactctgtagcaccgcctacatacctcgctctgctaatcctgttaccagtggctgctgccagtggcgataagtcgtgtcttaccgggttggactcaagacgatagttaccggataaggcgcagcggtcgggctgaacggggggttcgtgcacacagcccagcttggagcgaacgacctacaccgaactgagatacctacagcgtgagctatgagaaagcgccacgcttcccgaagggagaaaggcggacaggtatccggtaagcggcagggtcggaacaggagagcgcacgagggagcttccagggggaaacgcctggtatctttatagtcctgtcgggtttcgccacctctgacttgagcgtcgatttttgtgatgctcgtcaggggggcggagcctatggaaaaacgccagcaacgcggcctttttacggttcctggccttttgctggccttttgctcacatgttctttcctgcgttatcccctgattctgtggataaccgtattaccgcctttgagtgagctgataccgctcgccgcagccgaacgaccgagcgcagcgagtcagtgagcgaggaagcggaagagcgcccaatacgcaaaccgcctctccccgcgcgttggccgattcattaatgcagctggcacgacaggtttcccgactggaaagcgggcagtgagcgcaacgcaattaatgtgagttagctcactcattaggcaccccaggctttacactttatgcttccggctcgtatgttgtgtggaattgtgagcggataacaatttcacacaggaaacagctatgaccatgattacgccaagctttgctcttaggagtttcctaatacatcccaaactcaaatatataaagcatttgacttgttctatgccctagggggcggggggaagctaagccagctttttttaacatttaaaatgttaattccattttaaatgcacagatgtttttatttcataagggtttcaatgtgcatgaatgctgcaatattcctgttaccaaagctagtataaataaaaatagataaacgtggaaattacttagagtttctgtcattaacgtttccttcctcagttgacaacataaatgcgctgctgagcaagccagtttgcatctgtcaggatcaatttcccattatgccagtcatattaattactagtcaattagttgatttttatttttgacatatacatgtg

SEQ ID NO: 43 - DNA, 10595 bp, synthetic construct
  misc_feature 1..10595: note = pSFG4-hMeso-Ev3-CAR
  source 1..10595: mol_type = other DNA
aatgaaagaccccacctgtaggtttggcaagctagcttaagtaacgccattttgcaaggcatggaaaaatacataactgagaatagaaaagttcagatcaaggtcaggaacagatggaacagctgaatatgggccaaacaggatatctgtggtaagcagttcctgccccggctcagggccaagaacagatggaacagctgaatatgggccaaacaggatatctgtggtaagcagttcctgccccggctcagggccaagaacagatggtccccagatgcggtccagccctcagcagtttctagagaaccatcagatgtttccagggtgccccaaggacctgaaatgaccctgtgccttatttgaactaaccaatcagttcgcttctcgcttctgttcgcgcgcttatgctccccgagctcaataaaagagcccacaacccctcactcggggcgccagtcctccgattgactgagtcgcccgggtacccgtgtatccaataaaccctcttgcagttgcatccgacttgtggtctcgctgttccttgggagggtctcctctgagtgattgactacccgtcagcgggggtctttcatttgggggctcgtccgggatcgggagacccctgcccagggaccaccgacccaccaccgggaggtaagctggccagcaacttatctgtgtctgtccgattgtctagtgtctatgactgattttatgcgcctgcgtcggtactagttagctaactagctctgtatctggcggacccgtggtggaactgacgagttcggaacacccggccgcaaccctgggagacgtcccagggacttcgggggccgtttttgtggcccgacctgagtcctaaaatcccgatcgtttaggactctttggtgcaccccccttagaggagggatatgtggttctggtaggagacgagaacctaaaacagttcccgcctccgtctgaatttttgctttcggtttgggaccgaagccgcgccgcgcgtcttgtctgctgcagcatcgttctgtgttgtctctgtctgactgtgtttctgtatttgtctgaaaatatgggcccgggctagcctgttaccactcccttaagtttgaccttaggtcactggaaagatgtcgagcggatcgctcacaaccagtcggtagatgtcaagaagagacgttgggttaccttctgctctgcagaatggccaacctttaacgtcggatggccgcgagacggcacctttaaccgagacctcatcacccaggttaagatcaaggtcttttcacctggcccgcatggacacccagaccaggtggggtacatcgtgacctgggaagccttggcttttgacccccctccctgggtcaagccctttgtacaccctaagcctccgcctcctcttcctccatccgccccgtctctcccccttgaacctcctcgttcgaccccgcctcgatcctccctttatccagccctcactccttctctaggcgcccccatatggccatatgagatcttatatggggcacccccgccccttgtaaacttccctgaccctgacatgacaagagttactaacagcccctctctccaagctcacttacaggctctctacttagtccagcacgaagtctggagacctctggcggcagcctaccaagaacaactggaccgaccggtggtacctcacccttaccgagtcggcgacacagtgtgggtccgccgacaccagactaagaacctagaacctcgctggaaaggaccttacacagtcctgctgaccacccccaccgccctcaaagtagacggcatcgcagcttggatacacgccgcccacgtgaaggctgccgaccccgggggtggaccatcctctagactgccatgctcgagggagtgcaggtggaaaccatctccccaggagacgggcgcaccttccccaagcgcggccagacctgcgtggtgcactacaccgggatgcttgaagatggaaagaaagttgattcctcccgggacagaaacaagccctttaagtttatgctaggcaagcaggaggtgatccgaggctgggaagaaggggttgcccagatgagtgtgggtcagagagccaaactgactatatctccagattatgcctatggtgccactgggcacccaggcatcatcccaccacatgccactctcgtcttcgatgtggagcttctaaaactggaatctggcggtggatccggagtcgacggatttggtgatgtcggtgctcttgagagtttgaggggaaatgcagatttggcttacatcctgagcatggagccctgtggccactgcctcattatcaacaatgtgaacttctgccgtgagtccgggctccgcacccgcactggctccaacatcgactgtgagaagttgcggcgtcgcttctcctcgctgcatttcatggtggaggtgaagggcgacctgactgccaagaaaatggtgctggctttgctggagctggcgcagcaggaccacggtgctctggactgctgcgtggtggtcattctctctcacggctgtcaggccagccacctgcagttcccaggggctgtctacggcacagatggatgccctgtgtcggtcgagaagattgtgaacatcttcaatgggaccagctgccccagcctgggagggaagcccaagctctttttcatccaggcctgtggtggggagcagaaagaccatgggtttgaggtggcctccacttcccctgaagacgagtcccctggcagtaaccccgagccagatgccaccccgttccaggaaggtttgaggaccttcgaccagctggacgccatatctagtttgcccacacccagtgacatctttgtgtcctactctactttcccaggttttgtttcctggagggaccccaagagtggctcctggtacgttgagaccctggacgacatctttgagcagtgggctcactctgaagacctgcagtccctcctgcttagggtcgctaatgctgtttcggtgaaagggatttataaacagatgcctggttgctttaatttcctccggaaaaaacttttctttaaaacatcagctagcagagccgagggcaggggaagtcttctaacatgcggggacgtggaggaaaatcccgggcccatggagttcggcctttcttggctgtttttggtcgcaatattgaagggcgttcagtgttcaagggacatacagatgacgcagtcacctagctctctttcagcctctgtgggagaccgcgttacaattacgtgttctgcttctagttcagtgtcttacatgcattggtaccagcaaaaacccggcaaggttccaaagctccttatatacgatacgtccaaactggcttcaggcgtgccagacaggtttagtggatctgggagcggcactgacttcacacttacaatatccagtctgcaacccgaagatgttgcgacatactattgtcagcaatggagcggctatccgctcaccggacaggggacaaaagtggagataaagcggggctccaccagtggttccgggaagcctggtagtggtgagggttctacgaaaggcgaagtgcagttggtggagtctggtggcgggcttgttcaacccggtggttctctcaggcttagctgtgcagcctctgggtacacaatgaattgggtaaggcaagcgcctggaaagggccttgagtggatcggtttgataaccccatacaacggagcttcaagttacaaccaaaagttccgcgggaagtttattataagcagggataacgcaaagaacagcctctatcttcaaatgaactcactccgggctgaagacacagccgtctattattgtgcccgggggggctacgacggacgagggttcgattactggggtcagggcacactcgtgaccgtgtcaagctacgtcaccgtctcttcacaggatcccgccctggaagagaagaaaggcaattacgtcgtgaccgaccacggcagctgtgtgcgggcttgtggcgccgatagctacgagatggaagaggacggcgtgcggaagtgcaagaagtgcgagggcccctgcagaaaagtgtgcaacggcatcggcatcggagagttcaaggatagcctgagcatcaacgccaccaacatcaagcacttcaagaactgcaccagcatcagcggcgacctgcacatcctgcccgtggcctttagaggcgacagcttcacccacacccccccactggatccccaggaactggacatcctgaaaaccgtgaaagagatcacaggctttctgctgattcaggcctggcccgagaaccggacagacctgcacgccttcgagaacctggaaatcatcagaggccggaccaagcagcacggccagttttctctggccgtggtgtccctgaacatcaccagcctgggcctgcggagcctgaaagaaatcagcgacggcgacgtgatcatctccggcaacaagaacctgtgctacgccaacaccatcaattggaagaagctgttcggcacctccggccagaaaacaaagatcatctctaaccggggcgagaacagctgcaaagccaccggacaagtgtgccacgccctgtgtagccctgagggctgttggggacccgagcccagagattgcgtgtcctgccggaatgtgtccagaggccgcgagtgcgtggacaagtgcaacctgctggaaggcgagccccgcgagtttgtggaaaacagcgagtgcatccagtgccaccccgagtgtctgccccaggccatgaacattacctgcaccggcagaggccccgacaactgtatccagtgcgcccactacatcgacggcccccactgcgtgaaaacctgtccagctggcgtgatgggagagaacaacaccctcgtgtggaagtacgccgacgccggccatgtgtgccacctgtgtcaccccaattgcacctacggctgtaccggccctggcctggaaggctgtcctaccaacggccccaagatcccttctaaagatcccaaattttgggtgctggtggtggttggtggagtcctggcttgctatagcttgctagtaacagtggcctttattattttctgggtgaggagtaagaggagcaggctcctgcacagtgactacatgaacatgactccccgccgccccgggcccacccgcaagcattaccagccctatgccccaccacgcgacttcgcagcctatcgctccagagtgaagttcagcaggagcgcagacgcccccgcgtaccagcagggccagaaccagctctataacgagctcaatctaggacgaagagaggagtacgatgttttggacaagagacgtggccgggaccctgagatggggggaaagccgagaaggaagaaccctcaggaaggcctgtacaatgaactgcagaaagataagatggcggaggcctacagtgagattgggatgaaaggcgagcgccggaggggcaaggggcacgatggcctttaccagggtctcagtacagccaccaaggacacctacgacgcccttcacatgcaggccctgccccctcgcggaccgcagtgtactaattatgctctcttgaaattggctggagatgttgagagcaatcccgggcccatgcggatcagcaagccccacctgcggagcatcagcatccagtgctacctgtgcctgctgctgaacagccacttcctgaccgaggccggcatccacgtgttcatcctgggctgcttcagcgccggactgcccaagaccgaggccaactgggtgaacgtgatcagcgacctgaagaagatcgaggacctgatccagagcatgcacatcgacgccaccctgtacaccgagagcgacgtgcaccccagctgcaaggtgaccgccatgaagtgctttctgctggaactgcaggtgatcagcctggaaagcggcgacgccagcatccacgacaccgtggagaacctgatcatcctggccaacaacagcctgagcagcaacggcaacgtgaccgagagcggctgcaaagagtgcgaggaactggaagagaagaacatcaaagagtttctgcagagcttcgtgcacatcgtgcagatgttcatcaacaccagctgacgcgtcatcatcgatccggattagtccaatttgttaaagacaggatatcagtggtccaggctctagttttgactcaacaatatcaccagctgaagcctatagagtacgagccatagataaaataaaagattttatttagtctccagaaaaaggggggaatgaaagaccccacctgtaggtttggcaagctagcttaagtaacgccattttgcaaggcatggaaaaatacataactgagaatagagaagttcagatcaaggtcaggaacagatggaacagctgaatatgggccaaacaggatatctgtggtaagcagttcctgccccggctcagggccaagaacagatggaacagctgaatatgggccaaacaggatatctgtggtaagcagttcctgccccggctcagggccaagaacagatggtccccagatgcggtccagccctcagcagtttctagagaaccatcagatgtttccagggtgccccaaggacctgaaatgaccctgtgccttatttgaactaaccaatcagttcgcttctcgcttctgttcgcgcgcttctgctccccgagctcaataaaagagcccacaacccctcactcggggcgccagtcctccgattgactgagtcgcccgggtacccgtgtatccaataaaccctcttgcagttgcatccgacttgtggtctcgctgttccttgggagggtctcctctgagtgattgactacccgtcagcgggggtctttcacacatgcagcatgtatcaaaattaatttggttttttttcttaagtatttacattaaatggccatagtacttaaagttacattggcttccttgaaataaacatggagtattcagaatgtgtcataaatatttctaattttaagatagtatctccattggctttctactttttcttttatttttttttgtcctctgtcttccatttgttgttgttgttgtttgtttgtttgtttgttggttggttggttaatttttttttaaagatcctacactatagttcaagctagactattagctactctgtaacccagggtgaccttgaagtcatgggtagcctgctgttttagccttcccacatctaagattacaggtatgagctatcatttttggtatattgattgattgattgattgatgtgtgtgtgtgtgattgtgtttgtgtgtgtgactgtgaaaatgtgtgtatgggtgtgtgtgaatgtgtgtatgtatgtgtgtgtgtgagtgtgtgtgtgtgtgtgtgcatgtgtgtgtgtgtgactgtgtctatgtgtatgactgtgtgtgtgtgtgtgtgtgtgtgtgtgtgtgtgtgtgtgtgtgtgttgtgaaaaaatattctatggtagtgagagccaacgctccggctcaggtgtcaggttggtttttgagacagagtctttcacttagcttggaattcactggccgtcgttttacaacgtcgtgactgggaaaaccctggcgttacccaacttaatcgccttgcagcacatccccctttcgccagctggcgtaatagcgaagaggcccgcaccgatcgcccttcccaacagttgcgcagcctgaatggcgaatggcgcctgatgcggtattttctccttacgcatctgtgcggtatttcacaccgcatatggtgcactctcagtacaatctgctctgatgccgcatagttaagccagccccgacacccgccaacacccgctgacgcgccctgacgggcttgtctgctcccggcatccgcttacagacaagctgtgaccgtctccgggagctgcatgtgtcagaggttttcaccgtcatcaccgaaacgcgcgagacgaaagggcctcgtgatacgcctatttttataggttaatgtcatgataataatggtttcttagacgtcaggtggcacttttcggggaaatgtgcgcggaacccctatttgtttatttttctaaatacattcaaatatgtatccgctcatgagacaataaccctgataaatgcttcaataatattgaaaaaggaagagtatgagtattcaacatttccgtgtcgcccttattcccttttttgcggcattttgccttcctgtttttgctcacccagaaacgctggtgaaagtaaaagatgctgaagatcagttgggtgcacgagtgggttacatcgaactggatctcaacagcggtaagatccttgagagttttcgccccgaagaacgttttccaatgatgagcacttttaaagttctgctatgtggcgcggtattatcccgtattgacgccgggcaagagcaactcggtcgccgcatacactattctcagaatgacttggttgagtactcaccagtcacagaaaagcatcttacggatggcatgacagtaagagaattatgcagtgctgccataaccatgagtgataacactgcggccaacttacttctgacaacgatcggaggaccgaaggagctaaccgcttttttgcacaacatgggggatcatgtaactcgccttgatcgttgggaaccggagctgaatgaagccataccaaacgacgagcgtgacaccacgatgcctgtagcaatggcaacaacgttgcgcaaactattaactggcgaactacttactctagcttcccggcaacaattaatagactggatggaggcggataaagttgcaggaccacttctgcgctcggcccttccggctggctggtttattgctgataaatctggagccggtgagcgtgggtctcgcggtatcattgcagcactggggccagatggtaagccctcccgtatcgtagttatctacacgacggggagtcaggcaactatggatgaacgaaatagacagatcgctgagataggtgcctcactgattaagcattggtaactgtcagaccaagtttactcatatatactttagattgatttaaaacttcatttttaatttaaaaggatctaggtgaagatcctttttgataatctcatgaccaaaatcccttaacgtgagttttcgttccactgagcgtcagaccccgtagaaaagatcaaaggatcttcttgagatcctttttttctgcgcgtaatctgctgcttgcaaacaaaaaaaccaccgctaccagcggtggtttgtttgccggatcaagagctaccaactctttttccgaaggtaactggcttcagcagagcgcagataccaaatactgttcttctagtgtagccgtagttaggccaccacttcaagaactctgtagcaccgcctacatacctcgctctgctaatcctgttaccagtggctgctgccagtggcgataagtcgtgtcttaccgggttggactcaagacgatagttaccggataaggcgcagcggtcgggctgaacggggggttcgtgcacacagcccagcttggagcgaacgacctacaccgaactgagatacctacagcgtgagctatgagaaagcgccacgcttcccgaagggagaaaggcggacaggtatccggtaagcggcagggtcggaacaggagagcgcacgagggagcttccagggggaaacgcctggtatctttatagtcctgtcgggtttcgccacctctgacttgagcgtcgatttttgtgatgctcgtcaggggggcggagcctatggaaaaacgccagcaacgcggcctttttacggttcctggccttttgctggccttttgctcacatgttctttcctgcgttatcccctgattctgtggataaccgtattaccgcctttgagtgagctgataccgctcgccgcagccgaacgaccgagcgcagcgagtcagtgagcgaggaagcggaagagcgcccaatacgcaaaccgcctctccccgcgcgttggccgattcattaatgcagctggcacgacaggtttcccgactggaaagcgggcagtgagcgcaacgcaattaatgtgagttagctcactcattaggcaccccaggctttacactttatgcttccggctcgtatgttgtgtggaattgtgagcggataacaatttcacacaggaaacagctatgaccatgattacgccaagctttgctcttaggagtttcctaatacatcccaaactcaaatatataaagcatttgacttgttctatgccctagggggcggggggaagctaagccagctttttttaacatttaaaatgttaattccattttaaatgcacagatgtttttatttcataagggtttcaatgtgcatgaatgctgcaatattcctgttaccaaagctagtataaataaaaatagataaacgtggaaattacttagagtttctgtcattaacgtttccttcctcagttgacaacataaatgcgctgctgagcaagccagtttgcatctgtcaggatcaatttcccattatgccagtcatattaattactagtcaattagttgatttttatttttgacatatacatgtg

SEQ ID NO: 44 - DNA, 10613 bp, synthetic construct
  misc_feature 1..10613: note = pSFG4-ROR1-Ev3-CAR
  source 1..10613: mol_type = other DNA
aatgaaagaccccacctgtaggtttggcaagctagcttaagtaacgccattttgcaaggcatggaaaaatacataactgagaatagaaaagttcagatcaaggtcaggaacagatggaacagctgaatatgggccaaacaggatatctgtggtaagcagttcctgccccggctcagggccaagaacagatggaacagctgaatatgggccaaacaggatatctgtggtaagcagttcctgccccggctcagggccaagaacagatggtccccagatgcggtccagccctcagcagtttctagagaaccatcagatgtttccagggtgccccaaggacctgaaatgaccctgtgccttatttgaactaaccaatcagttcgcttctcgcttctgttcgcgcgcttatgctccccgagctcaataaaagagcccacaacccctcactcggggcgccagtcctccgattgactgagtcgcccgggtacccgtgtatccaataaaccctcttgcagttgcatccgacttgtggtctcgctgttccttgggagggtctcctctgagtgattgactacccgtcagcgggggtctttcatttgggggctcgtccgggatcgggagacccctgcccagggaccaccgacccaccaccgggaggtaagctggccagcaacttatctgtgtctgtccgattgtctagtgtctatgactgattttatgcgcctgcgtcggtactagttagctaactagctctgtatctggcggacccgtggtggaactgacgagttcggaacacccggccgcaaccctgggagacgtcccagggacttcgggggccgtttttgtggcccgacctgagtcctaaaatcccgatcgtttaggactctttggtgcaccccccttagaggagggatatgtggttctggtaggagacgagaacctaaaacagttcccgcctccgtctgaatttttgctttcggtttgggaccgaagccgcgccgcgcgtcttgtctgctgcagcatcgttctgtgttgtctctgtctgactgtgtttctgtatttgtctgaaaatatgggcccgggctagcctgttaccactcccttaagtttgaccttaggtcactggaaagatgtcgagcggatcgctcacaaccagtcggtagatgtcaagaagagacgttgggttaccttctgctctgcagaatggccaacctttaacgtcggatggccgcgagacggcacctttaaccgagacctcatcacccaggttaagatcaaggtcttttcacctggcccgcatggacacccagaccaggtggggtacatcgtgacctgggaagccttggcttttgacccccctccctgggtcaagccctttgtacaccctaagcctccgcctcctcttcctccatccgccccgtctctcccccttgaacctcctcgttcgaccccgcctcgatcctccctttatccagccctcactccttctctaggcgcccccatatggccatatgagatcttatatggggcacccccgccccttgtaaacttccctgaccctgacatgacaagagttactaacagcccctctctccaagctcacttacaggctctctacttagtccagcacgaagtctggagacctctggcggcagcctaccaagaacaactggaccgaccggtggtacctcacccttaccgagtcggcgacacagtgtgggtccgccgacaccagactaagaacctagaacctcgctggaaaggaccttacacagtcctgctgaccacccccaccgccctcaaagtagacggcatcgcagcttggatacacgccgcccacgtgaaggctgccgaccccgggggtggaccatcctctagactgccatgctcgagggagtgcaggtggaaaccatctccccaggagacgggcgcaccttccccaagcgcggccagacctgcgtggtgcactacaccgggatgcttgaagatggaaagaaagttgattcctcccgggacagaaacaagccctttaagtttatgctaggcaagcaggaggtgatccgaggctgggaagaaggggttgcccagatgagtgtgggtcagagagccaaactgactatatctccagattatgcctatggtgccactgggcacccaggcatcatcccaccacatgccactctcgtcttcgatgtggagcttctaaaactggaatctggcggtggatccggagtcgacggatttggtgatgtcggtgctcttgagagtttgaggggaaatgcagatttggcttacatcctgagcatggagccctgtggccactgcctcattatcaacaatgtgaacttctgccgtgagtccgggctccgcacccgcactggctccaacatcgactgtgagaagttgcggcgtcgcttctcctcgctgcatttcatggtggaggtgaagggcgacctgactgccaagaaaatggtgctggctttgctggagctggcgcagcaggaccacggtgctctggactgctgcgtggtggtcattctctctcacggctgtcaggccagccacctgcagttcccaggggctgtctacggcacagatggatgccctgtgtcggtcgagaagattgtgaacatcttcaatgggaccagctgccccagcctgggagggaagcccaagctctttttcatccaggcctgtggtggggagcagaaagaccatgggtttgaggtggcctccacttcccctgaagacgagtcccctggcagtaaccccgagccagatgccaccccgttccaggaaggtttgaggaccttcgaccagctggacgccatatctagtttgcccacacccagtgacatctttgtgtcctactctactttcccaggttttgtttcctggagggaccccaagagtggctcctggtacgttgagaccctggacgacatctttgagcagtgggctcactctgaagacctgcagtccctcctgcttagggtcgctaatgctgtttcggtgaaagggatttataaacagatgcctggttgctttaatttcctccggaaaaaacttttctttaaaacatcagctagcagagccgagggcaggggaagtcttctaacatgcggggacgtggaggaaaatcccgggcccatggagttcggtcttagctggctgttcctcgtggcaatcctcaagggagtacaatgcagcagagatattaagatgacgcagtccccctcttctatgtacgcgagtctgggagagagggtaaccattacatgtaaggcgtctcccgatataaactcatatctgagctggtttcaacaaaagccgggcaagagtccgaagacactcatttaccgagcaaaccgcctggtagacggtgtgccttccagattctctggcggtggcagcgggcaagactactcactcaccataaattcacttgaatacgaggatatgggtatatactactgcttgcaatatgatgagtttccatatacttttggcggcggaactaaacttgaaatgaaagggagcacgtctggttccggcaagcctggttcaggagagggtagcaccaaaggggaagtcaaactcgtcgaaagtggtggtggcttggtgaaacccggcggatctctgaaactcagttgtgccgcttctggttttacatttagctcctacgcgatgagttgggtcaggcaaataccagagaagagacttgagtgggtcgctagtattagcaggggagggaccacctactatccagactctgtgaaaggtagattcactatctctagagacaacgtacgcaatatcctgtatctccaaatgagctcattgaggagcgaggatacggctatgtactattgtggccgatacgactatgatggatactatgcgatggattactggggccaaggcacttctgtaacagtttctagctacgtcaccgtctcttcacaggatcccgccctggaagagaagaaaggcaattacgtcgtgaccgaccacggcagctgtgtgcgggcttgtggcgccgatagctacgagatggaagaggacggcgtgcggaagtgcaagaagtgcgagggcccctgcagaaaagtgtgcaacggcatcggcatcggagagttcaaggatagcctgagcatcaacgccaccaacatcaagcacttcaagaactgcaccagcatcagcggcgacctgcacatcctgcccgtggcctttagaggcgacagcttcacccacacccccccactggatccccaggaactggacatcctgaaaaccgtgaaagagatcacaggctttctgctgattcaggcctggcccgagaaccggacagacctgcacgccttcgagaacctggaaatcatcagaggccggaccaagcagcacggccagttttctctggccgtggtgtccctgaacatcaccagcctgggcctgcggagcctgaaagaaatcagcgacggcgacgtgatcatctccggcaacaagaacctgtgctacgccaacaccatcaattggaagaagctgttcggcacctccggccagaaaacaaagatcatctctaaccggggcgagaacagctgcaaagccaccggacaagtgtgccacgccctgtgtagccctgagggctgttggggacccgagcccagagattgcgtgtcctgccggaatgtgtccagaggccgcgagtgcgtggacaagtgcaacctgctggaaggcgagccccgcgagtttgtggaaaacagcgagtgcatccagtgccaccccgagtgtctgccccaggccatgaacattacctgcaccggcagaggccccgacaactgtatccagtgcgcccactacatcgacggcccccactgcgtgaaaacctgtccagctggcgtgatgggagagaacaacaccctcgtgtggaagtacgccgacgccggccatgtgtgccacctgtgtcaccccaattgcacctacggctgtaccggccctggcctggaaggctgtcctaccaacggccccaagatcccttctaaagatcccaaattttgggtgctggtggtggttggtggagtcctggcttgctatagcttgctagtaacagtggcctttattattttctgggtgaggagtaagaggagcaggctcctgcacagtgactacatgaacatgactccccgccgccccgggcccacccgcaagcattaccagccctatgccccaccacgcgacttcgcagcctatcgctccagagtgaagttcagcaggagcgcagacgcccccgcgtaccagcagggccagaaccagctctataacgagctcaatctaggacgaagagaggagtacgatgttttggacaagagacgtggccgggaccctgagatggggggaaagccgagaaggaagaaccctcaggaaggcctgtacaatgaactgcagaaagataagatggcggaggcctacagtgagattgggatgaaaggcgagcgccggaggggcaaggggcacgatggcctttaccagggtctcagtacagccaccaaggacacctacgacgcccttcacatgcaggccctgccccctcgcggaccgcagtgtactaattatgctctcttgaaattggctggagatgttgagagcaatcccgggcccatgcggatcagcaagccccacctgcggagcatcagcatccagtgctacctgtgcctgctgctgaacagccacttcctgaccgaggccggcatccacgtgttcatcctgggctgcttcagcgccggactgcccaagaccgaggccaactgggtgaacgtgatcagcgacctgaagaagatcgaggacctgatccagagcatgcacatcgacgccaccctgtacaccgagagcgacgtgcaccccagctgcaaggtgaccgccatgaagtgctttctgctggaactgcaggtgatcagcctggaaagcggcgacgccagcatccacgacaccgtggagaacctgatcatcctggccaacaacagcctgagcagcaacggcaacgtgaccgagagcggctgcaaagagtgcgaggaactggaagagaagaacatcaaagagtttctgcagagcttcgtgcacatcgtgcagatgttcatcaacaccagctgacgcgtcatcatcgatccggattagtccaatttgttaaagacaggatatcagtggtccaggctctagttttgactcaacaatatcaccagctgaagcctatagagtacgagccatagataaaataaaagattttatttagtctccagaaaaaggggggaatgaaagaccccacctgtaggtttggcaagctagcttaagtaacgccattttgcaaggcatggaaaaatacataactgagaatagagaagttcagatcaaggtcaggaacagatggaacagctgaatatgggccaaacaggatatctgtggtaagcagttcctgccccggctcagggccaagaacagatggaacagctgaatatgggccaaacaggatatctgtggtaagcagttcctgccccggctcagggccaagaacagatggtccccagatgcggtccagccctcagcagtttctagagaaccatcagatgtttccagggtgccccaaggacctgaaatgaccctgtgccttatttgaactaaccaatcagttcgcttctcgcttctgttcgcgcgcttctgctccccgagctcaataaaagagcccacaacccctcactcggggcgccagtcctccgattgactgagtcgcccgggtacccgtgtatccaataaaccctcttgcagttgcatccgacttgtggtctcgctgttccttgggagggtctcctctgagtgattgactacccgtcagcgggggtctttcacacatgcagcatgtatcaaaattaatttggttttttttcttaagtatttacattaaatggccatagtacttaaagttacattggcttccttgaaataaacatggagtattcagaatgtgtcataaatatttctaattttaagatagtatctccattggctttctactttttcttttatttttttttgtcctctgtcttccatttgttgttgttgttgtttgtttgtttgtttgttggttggttggttaatttttttttaaagatcctacactatagttcaagctagactattagctactctgtaacccagggtgaccttgaagtcatgggtagcctgctgttttagccttcccacatctaagattacaggtatgagctatcatttttggtatattgattgattgattgattgatgtgtgtgtgtgtgattgtgtttgtgtgtgtgactgtgaaaatgtgtgtatgggtgtgtgtgaatgtgtgtatgtatgtgtgtgtgtgagtgtgtgtgtgtgtgtgtgcatgtgtgtgtgtgtgactgtgtctatgtgtatgactgtgtgtgtgtgtgtgtgtgtgtgtgtgtgtgtgtgtgtgtgtgtgttgtgaaaaaatattctatggtagtgagagccaacgctccggctcaggtgtcaggttggtttttgagacagagtctttcacttagcttggaattcactggccgtcgttttacaacgtcgtgactgggaaaaccctggcgttacccaacttaatcgccttgcagcacatccccctttcgccagctggcgtaatagcgaagaggcccgcaccgatcgcccttcccaacagttgcgcagcctgaatggcgaatggcgcctgatgcggtattttctccttacgcatctgtgcggtatttcacaccgcatatggtgcactctcagtacaatctgctctgatgccgcatagttaagccagccccgacacccgccaacacccgctgacgcgccctgacgggcttgtctgctcccggcatccgcttacagacaagctgtgaccgtctccgggagctgcatgtgtcagaggttttcaccgtcatcaccgaaacgcgcgagacgaaagggcctcgtgatacgcctatttttataggttaatgtcatgataataatggtttcttagacgtcaggtggcacttttcggggaaatgtgcgcggaacccctatttgtttatttttctaaatacattcaaatatgtatccgctcatgagacaataaccctgataaatgcttcaataatattgaaaaaggaagagtatgagtattcaacatttccgtgtcgcccttattcccttttttgcggcattttgccttcctgtttttgctcacccagaaacgctggtgaaagtaaaagatgctgaagatcagttgggtgcacgagtgggttacatcgaactggatctcaacagcggtaagatccttgagagttttcgccccgaagaacgttttccaatgatgagcacttttaaagttctgctatgtggcgcggtattatcccgtattgacgccgggcaagagcaactcggtcgccgcatacactattctcagaatgacttggttgagtactcaccagtcacagaaaagcatcttacggatggcatgacagtaagagaattatgcagtgctgccataaccatgagtgataacactgcggccaacttacttctgacaacgatcggaggaccgaaggagctaaccgcttttttgcacaacatgggggatcatgtaactcgccttgatcgttgggaaccggagctgaatgaagccataccaaacgacgagcgtgacaccacgatgcctgtagcaatggcaacaacgttgcgcaaactattaactggcgaactacttactctagcttcccggcaacaattaatagactggatggaggcggataaagttgcaggaccacttctgcgctcggcccttccggctggctggtttattgctgataaatctggagccggtgagcgtgggtctcgcggtatcattgcagcactggggccagatggtaagccctcccgtatcgtagttatctacacgacggggagtcaggcaactatggatgaacgaaatagacagatcgctgagataggtgcctcactgattaagcattggtaactgtcagaccaagtttactcatatatactttagattgatttaaaacttcatttttaatttaaaaggatctaggtgaagatcctttttgataatctcatgaccaaaatcccttaacgtgagttttcgttccactgagcgtcagaccccgtagaaaagatcaaaggatcttcttgagatcctttttttctgcgcgtaatctgctgcttgcaaacaaaaaaaccaccgctaccagcggtggtttgtttgccggatcaagagctaccaactctttttccgaaggtaactggcttcagcagagcgcagataccaaatactgttcttctagtgtagccgtagttaggccaccacttcaagaactctgtagcaccgcctacatacctcgctctgctaatcctgttaccagtggctgctgccagtggcgataagtcgtgtcttaccgggttggactcaagacgatagttaccggataaggcgcagcggtcgggctgaacggggggttcgtgcacacagcccagcttggagcgaacgacctacaccgaactgagatacctacagcgtgagctatgagaaagcgccacgcttcccgaagggagaaaggcggacaggtatccggtaagcggcagggtcggaacaggagagcgcacgagggagcttccagggggaaacgcctggtatctttatagtcctgtcgggtttcgccacctctgacttgagcgtcgatttttgtgatgctcgtcaggggggcggagcctatggaaaaacgccagcaacgcggcctttttacggttcctggccttttgctggccttttgctcacatgttctttcctgcgttatcccctgattctgtggataaccgtattaccgcctttgagtgagctgataccgctcgccgcagccgaacgaccgagcgcagcgagtcagtgagcgaggaagcggaagagcgcccaatacgcaaaccgcctctccccgcgcgttggccgattcattaatgcagctggcacgacaggtttcccgactggaaagcgggcagtgagcgcaacgcaattaatgtgagttagctcactcattaggcaccccaggctttacactttatgcttccggctcgtatgttgtgtggaattgtgagcggataacaatttcacacaggaaacagctatgaccatgattacgccaagctttgctcttaggagtttcctaatacatcccaaactcaaatatataaagcatttgacttgttctatgccctagggggcggggggaagctaagccagctttttttaacatttaaaatgttaattccattttaaatgcacagatgtttttatttcataagggtttcaatgtgcatgaatgctgcaatattcctgttaccaaagctagtataaataaaaatagataaacgtggaaattacttagagtttctgtcattaacgtttccttcctcagttgacaacataaatgcgctgctgagcaagccagtttgcatctgtcaggatcaatttcccattatgccagtcatattaattactagtcaattagttgatttttatttttgacatatacatgtg

SEQ ID NO: 45 - DNA, 10616 bp, synthetic construct
  misc_feature 1..10616: note = pSFG4-hROR1-Ev3-CAR
  source 1..10616: mol_type = other DNA
aatgaaagaccccacctgtaggtttggcaagctagcttaagtaacgccattttgcaaggcatggaaaaatacataactgagaatagaaaagttcagatcaaggtcaggaacagatggaacagctgaatatgggccaaacaggatatctgtggtaagcagttcctgccccggctcagggccaagaacagatggaacagctgaatatgggccaaacaggatatctgtggtaagcagttcctgccccggctcagggccaagaacagatggtccccagatgcggtccagccctcagcagtttctagagaaccatcagatgtttccagggtgccccaaggacctgaaatgaccctgtgccttatttgaactaaccaatcagttcgcttctcgcttctgttcgcgcgcttatgctccccgagctcaataaaagagcccacaacccctcactcggggcgccagtcctccgattgactgagtcgcccgggtacccgtgtatccaataaaccctcttgcagttgcatccgacttgtggtctcgctgttccttgggagggtctcctctgagtgattgactacccgtcagcgggggtctttcatttgggggctcgtccgggatcgggagacccctgcccagggaccaccgacccaccaccgggaggtaagctggccagcaacttatctgtgtctgtccgattgtctagtgtctatgactgattttatgcgcctgcgtcggtactagttagctaactagctctgtatctggcggacccgtggtggaactgacgagttcggaacacccggccgcaaccctgggagacgtcccagggacttcgggggccgtttttgtggcccgacctgagtcctaaaatcccgatcgtttaggactctttggtgcaccccccttagaggagggatatgtggttctggtaggagacgagaacctaaaacagttcccgcctccgtctgaatttttgctttcggtttgggaccgaagccgcgccgcgcgtcttgtctgctgcagcatcgttctgtgttgtctctgtctgactgtgtttctgtatttgtctgaaaatatgggcccgggctagcctgttaccactcccttaagtttgaccttaggtcactggaaagatgtcgagcggatcgctcacaaccagtcggtagatgtcaagaagagacgttgggttaccttctgctctgcagaatggccaacctttaacgtcggatggccgcgagacggcacctttaaccgagacctcatcacccaggttaagatcaaggtcttttcacctggcccgcatggacacccagaccaggtggggtacatcgtgacctgggaagccttggcttttgacccccctccctgggtcaagccctttgtacaccctaagcctccgcctcctcttcctccatccgccccgtctctcccccttgaacctcctcgttcgaccccgcctcgatcctccctttatccagccctcactccttctctaggcgcccccatatggccatatgagatcttatatggggcacccccgccccttgtaaacttccctgaccctgacatgacaagagttactaacagcccctctctccaagctcacttacaggctctctacttagtccagcacgaagtctggagacctctggcggcagcctaccaagaacaactggaccgaccggtggtacctcacccttaccgagtcggcgacacagtgtgggtccgccgacaccagactaagaacctagaacctcgctggaaaggaccttacacagtcctgctgaccacccccaccgccctcaaagtagacggcatcgcagcttggatacacgccgcccacgtgaaggctgccgaccccgggggtggaccatcctctagactgccatgctcgagggagtgcaggtggaaaccatctccccaggagacgggcgcaccttccccaagcgcggccagacctgcgtggtgcactacaccgggatgcttgaagatggaaagaaagttgattcctcccgggacagaaacaagccctttaagtttatgctaggcaagcaggaggtgatccgaggctgggaagaaggggttgcccagatgagtgtgggtcagagagccaaactgactatatctccagattatgcctatggtgccactgggcacccaggcatcatcccaccacatgccactctcgtcttcgatgtggagcttctaaaactggaatctggcggtggatccggagtcgacggatttggtgatgtcggtgctcttgagagtttgaggggaaatgcagatttggcttacatcctgagcatggagccctgtggccactgcctcattatcaacaatgtgaacttctgccgtgagtccgggctccgcacccgcactggctccaacatcgactgtgagaagttgcggcgtcgcttctcctcgctgcatttcatggtggaggtgaagggcgacctgactgccaagaaaatggtgctggctttgctggagctggcgcagcaggaccacggtgctctggactgctgcgtggtggtcattctctctcacggctgtcaggccagccacctgcagttcccaggggctgtctacggcacagatggatgccctgtgtcggtcgagaagattgtgaacatcttcaatgggaccagctgccccagcctgggagggaagcccaagctctttttcatccaggcctgtggtggggagcagaaagaccatgggtttgaggtggcctccacttcccctgaagacgagtcccctggcagtaaccccgagccagatgccaccccgttccaggaaggtttgaggaccttcgaccagctggacgccatatctagtttgcccacacccagtgacatctttgtgtcctactctactttcccaggttttgtttcctggagggaccccaagagtggctcctggtacgttgagaccctggacgacatctttgagcagtgggctcactctgaagacctgcagtccctcctgcttagggtcgctaatgctgtttcggtgaaagggatttataaacagatgcctggttgctttaatttcctccggaaaaaacttttctttaaaacatcagctagcagagccgagggcaggggaagtcttctaacatgcggggacgtggaggaaaatcccgggcccatggagttcggacttagttggcttttcctcgtcgccatactcaaaggtgtacaatgctcacgcgatatacaaatgacgcagagtccatcctcactgtctgcctcagtaggcgacagggtcacaataacctgtaaagcaagcccggatatcaactcttacctcagttggttccaacagaaaccaggaaaggtgccgaagttgttgatttaccgcgcaaaccgcctcgttgacggcgtgccagataggttttctggcagcgggagcggcactgactttacgctcactatatcaagcctgcagccggaggacgtagcaacttactattgcctccaatacgacgaattcccttacacgttcgggcaaggaactaaagttgaaataaaaagaggaagcacaagtggttctggaaaacccggttccggtgagggcagtaccaaaggagaggtgcagttggtagagtctggtgggggtttggtgcaacccggagggtctctgaggttgtcttgcgcggcatccggctttactttttcctcatatgcgatgtcatgggtacgacaggccccaggcaagggactggagtggatcgcatctatttcacgaggagggacgacatattacccggattcagtgaagggcaaattcataatttcacgcgataacgccaagaactccctctacctgcaaatgaacagtcttagagcggaagatacggctgtgtattactgtgcgcgatatgactacgatggatattacgcgatggattattggggacaaggtacactggtaaccgtttccagctacgtcaccgtctcttcacaggatcccgccctggaagagaagaaaggcaattacgtcgtgaccgaccacggcagctgtgtgcgggcttgtggcgccgatagctacgagatggaagaggacggcgtgcggaagtgcaagaagtgcgagggcccctgcagaaaagtgtgcaacggcatcggcatcggagagttcaaggatagcctgagcatcaacgccaccaacatcaagcacttcaagaactgcaccagcatcagcggcgacctgcacatcctgcccgtggcctttagaggcgacagcttcacccacacccccccactggatccccaggaactggacatcctgaaaaccgtgaaagagatcacaggctttctgctgattcaggcctggcccgagaaccggacagacctgcacgccttcgagaacctggaaatcatcagaggccggaccaagcagcacggccagttttctctggccgtggtgtccctgaacatcaccagcctgggcctgcggagcctgaaagaaatcagcgacggcgacgtgatcatctccggcaacaagaacctgtgctacgccaacaccatcaattggaagaagctgttcggcacctccggccagaaaacaaagatcatctctaaccggggcgagaacagctgcaaagccaccggacaagtgtgccacgccctgtgtagccctgagggctgttggggacccgagcccagagattgcgtgtcctgccggaatgtgtccagaggccgcgagtgcgtggacaagtgcaacctgctggaaggcgagccccgcgagtttgtggaaaacagcgagtgcatccagtgccaccccgagtgtctgccccaggccatgaacattacctgcaccggcagaggccccgacaactgtatccagtgcgcccactacatcgacggcccccactgcgtgaaaacctgtccagctggcgtgatgggagagaacaacaccctcgtgtggaagtacgccgacgccggccatgtgtgccacctgtgtcaccccaattgcacctacggctgtaccggccctggcctggaaggctgtcctaccaacggccccaagatcccttctaaagatcccaaattttgggtgctggtggtggttggtggagtcctggcttgctatagcttgctagtaacagtggcctttattattttctgggtgaggagtaagaggagcaggctcctgcacagtgactacatgaacatgactccccgccgccccgggcccacccgcaagcattaccagccctatgccccaccacgcgacttcgcagcctatcgctccagagtgaagttcagcaggagcgcagacgcccccgcgtaccagcagggccagaaccagctctataacgagctcaatctaggacgaagagaggagtacgatgttttggacaagagacgtggccgggaccctgagatggggggaaagccgagaaggaagaaccctcaggaaggcctgtacaatgaactgcagaaagataagatggcggaggcctacagtgagattgggatgaaaggcgagcgccggaggggcaaggggcacgatggcctttaccagggtctcagtacagccaccaaggacacctacgacgcccttcacatgcaggccctgccccctcgcggaccgcagtgtactaattatgctctcttgaaattggctggagatgttgagagcaatcccgggcccatgcggatcagcaagccccacctgcggagcatcagcatccagtgctacctgtgcctgctgctgaacagccacttcctgaccgaggccggcatccacgtgttcatcctgggctgcttcagcgccggactgcccaagaccgaggccaactgggtgaacgtgatcagcgacctgaagaagatcgaggacctgatccagagcatgcacatcgacgccaccctgtacaccgagagcgacgtgcaccccagctgcaaggtgaccgccatgaagtgctttctgctggaactgcaggtgatcagcctggaaagcggcgacgccagcatccacgacaccgtggagaacctgatcatcctggccaacaacagcctgagcagcaacggcaacgtgaccgagagcggctgcaaagagtgcgaggaactggaagagaagaacatcaaagagtttctgcagagcttcgtgcacatcgtgcagatgttcatcaacaccagctgacgcgtcatcatcgatccggattagtccaatttgttaaagacaggatatcagtggtccaggctctagttttgactcaacaatatcaccagctgaagcctatagagtacgagccatagataaaataaaagattttatttagtctccagaaaaaggggggaatgaaagaccccacctgtaggtttggcaagctagcttaagtaacgccattttgcaaggcatggaaaaatacataactgagaatagagaagttcagatcaaggtcaggaacagatggaacagctgaatatgggccaaacaggatatctgtggtaagcagttcctgccccggctcagggccaagaacagatggaacagctgaatatgggccaaacaggatatctgtggtaagcagttcctgccccggctcagggccaagaacagatggtccccagatgcggtccagccctcagcagtttctagagaaccatcagatgtttccagggtgccccaaggacctgaaatgaccctgtgccttatttgaactaaccaatcagttcgcttctcgcttctgttcgcgcgcttctgctccccgagctcaataaaagagcccacaacccctcactcggggcgccagtcctccgattgactgagtcgcccgggtacccgtgtatccaataaaccctcttgcagttgcatccgacttgtggtctcgctgttccttgggagggtctcctctgagtgattgactacccgtcagcgggggtctttcacacatgcagcatgtatcaaaattaatttggttttttttcttaagtatttacattaaatggccatagtacttaaagttacattggcttccttgaaataaacatggagtattcagaatgtgtcataaatatttctaattttaagatagtatctccattggctttctactttttcttttatttttttttgtcctctgtcttccatttgttgttgttgttgtttgtttgtttgtttgttggttggttggttaatttttttttaaagatcctacactatagttcaagctagactattagctactctgtaacccagggtgaccttgaagtcatgggtagcctgctgttttagccttcccacatctaagattacaggtatgagctatcatttttggtatattgattgattgattgattgatgtgtgtgtgtgtgattgtgtttgtgtgtgtgactgtgaaaatgtgtgtatgggtgtgtgtgaatgtgtgtatgtatgtgtgtgtgtgagtgtgtgtgtgtgtgtgtgcatgtgtgtgtgtgtgactgtgtctatgtgtatgactgtgtgtgtgtgtgtgtgtgtgtgtgtgtgtgtgtgtgtgtgtgtgttgtgaaaaaatattctatggtagtgagagccaacgctccggctcaggtgtcaggttggtttttgagacagagtctttcacttagcttggaattcactggccgtcgttttacaacgtcgtgactgggaaaaccctggcgttacccaacttaatcgccttgcagcacatccccctttcgccagctggcgtaatagcgaagaggcccgcaccgatcgcccttcccaacagttgcgcagcctgaatggcgaatggcgcctgatgcggtattttctccttacgcatctgtgcggtatttcacaccgcatatggtgcactctcagtacaatctgctctgatgccgcatagttaagccagccccgacacccgccaacacccgctgacgcgccctgacgggcttgtctgctcccggcatccgcttacagacaagctgtgaccgtctccgggagctgcatgtgtcagaggttttcaccgtcatcaccgaaacgcgcgagacgaaagggcctcgtgatacgcctatttttataggttaatgtcatgataataatggtttcttagacgtcaggtggcacttttcggggaaatgtgcgcggaacccctatttgtttatttttctaaatacattcaaatatgtatccgctcatgagacaataaccctgataaatgcttcaataatattgaaaaaggaagagtatgagtattcaacatttccgtgtcgcccttattcccttttttgcggcattttgccttcctgtttttgctcacccagaaacgctggtgaaagtaaaagatgctgaagatcagttgggtgcacgagtgggttacatcgaactggatctcaacagcggtaagatccttgagagttttcgccccgaagaacgttttccaatgatgagcacttttaaagttctgctatgtggcgcggtattatcccgtattgacgccgggcaagagcaactcggtcgccgcatacactattctcagaatgacttggttgagtactcaccagtcacagaaaagcatcttacggatggcatgacagtaagagaattatgcagtgctgccataaccatgagtgataacactgcggccaacttacttctgacaacgatcggaggaccgaaggagctaaccgcttttttgcacaacatgggggatcatgtaactcgccttgatcgttgggaaccggagctgaatgaagccataccaaacgacgagcgtgacaccacgatgcctgtagcaatggcaacaacgttgcgcaaactattaactggcgaactacttactctagcttcccggcaacaattaatagactggatggaggcggataaagttgcaggaccacttctgcgctcggcccttccggctggctggtttattgctgataaatctggagccggtgagcgtgggtctcgcggtatcattgcagcactggggccagatggtaagccctcccgtatcgtagttatctacacgacggggagtcaggcaactatggatgaacgaaatagacagatcgctgagataggtgcctcactgattaagcattggtaactgtcagaccaagtttactcatatatactttagattgatttaaaacttcatttttaatttaaaaggatctaggtgaagatcctttttgataatctcatgaccaaaatcccttaacgtgagttttcgttccactgagcgtcagaccccgtagaaaagatcaaaggatcttcttgagatcctttttttctgcgcgtaatctgctgcttgcaaacaaaaaaaccaccgctaccagcggtggtttgtttgccggatcaagagctaccaactctttttccgaaggtaactggcttcagcagagcgcagataccaaatactgttcttctagtgtagccgtagttaggccaccacttcaagaactctgtagcaccgcctacatacctcgctctgctaatcctgttaccagtggctgctgccagtggcgataagtcgtgtcttaccgggttggactcaagacgatagttaccggataaggcgcagcggtcgggctgaacggggggttcgtgcacacagcccagcttggagcgaacgacctacaccgaactgagatacctacagcgtgagctatgagaaagcgccacgcttcccgaagggagaaaggcggacaggtatccggtaagcggcagggtcggaacaggagagcgcacgagggagcttccagggggaaacgcctggtatctttatagtcctgtcgggtttcgccacctctgacttgagcgtcgatttttgtgatgctcgtcaggggggcggagcctatggaaaaacgccagcaacgcggcctttttacggttcctggccttttgctggccttttgctcacatgttctttcctgcgttatcccctgattctgtggataaccgtattaccgcctttgagtgagctgataccgctcgccgcagccgaacgaccgagcgcagcgagtcagtgagcgaggaagcggaagagcgcccaatacgcaaaccgcctctccccgcgcgttggccgattcattaatgcagctggcacgacaggtttcccgactggaaagcgggcagtgagcgcaacgcaattaatgtgagttagctcactcattaggcaccccaggctttacactttatgcttccggctcgtatgttgtgtggaattgtgagcggataacaatttcacacaggaaacagctatgaccatgattacgccaagctttgctcttaggagtttcctaatacatcccaaactcaaatatataaagcatttgacttgttctatgccctagggggcggggggaagctaagccagctttttttaacatttaaaatgttaattccattttaaatgcacagatgtttttatttcataagggtttcaatgtgcatgaatgctgcaatattcctgttaccaaagctagtataaataaaaatagataaacgtggaaattacttagagtttctgtcattaacgtttccttcctcagttgacaacataaatgcgctgctgagcaagccagtttgcatctgtcaggatcaatttcccattatgccagtcatattaattactagtcaattagttgatttttatttttgacatatacatgtg

SEQ ID NO: 46 - DNA, 10610 bp, synthetic construct
  misc_feature 1..10610: note = pSFG4-CD5-Ev3-CAR
  source 1..10610: mol_type = other DNA
aatgaaagaccccacctgtaggtttggcaagctagcttaagtaacgccattttgcaaggcatggaaaaatacataactgagaatagaaaagttcagatcaaggtcaggaacagatggaacagctgaatatgggccaaacaggatatctgtggtaagcagttcctgccccggctcagggccaagaacagatggaacagctgaatatgggccaaacaggatatctgtggtaagcagttcctgccccggctcagggccaagaacagatggtccccagatgcggtccagccctcagcagtttctagagaaccatcagatgtttccagggtgccccaaggacctgaaatgaccctgtgccttatttgaactaaccaatcagttcgcttctcgcttctgttcgcgcgcttatgctccccgagctcaataaaagagcccacaacccctcactcggggcgccagtcctccgattgactgagtcgcccgggtacccgtgtatccaataaaccctcttgcagttgcatccgacttgtggtctcgctgttccttgggagggtctcctctgagtgattgactacccgtcagcgggggtctttcatttgggggctcgtccgggatcgggagacccctgcccagggaccaccgacccaccaccgggaggtaagctggccagcaacttatctgtgtctgtccgattgtctagtgtctatgactgattttatgcgcctgcgtcggtactagttagctaactagctctgtatctggcggacccgtggtggaactgacgagttcggaacacccggccgcaaccctgggagacgtcccagggacttcgggggccgtttttgtggcccgacctgagtcctaaaatcccgatcgtttaggactctttggtgcaccccccttagaggagggatatgtggttctggtaggagacgagaacctaaaacagttcccgcctccgtctgaatttttgctttcggtttgggaccgaagccgcgccgcgcgtcttgtctgctgcagcatcgttctgtgttgtctctgtctgactgtgtttctgtatttgtctgaaaatatgggcccgggctagcctgttaccactcccttaagtttgaccttaggtcactggaaagatgtcgagcggatcgctcacaaccagtcggtagatgtcaagaagagacgttgggttaccttctgctctgcagaatggccaacctttaacgtcggatggccgcgagacggcacctttaaccgagacctcatcacccaggttaagatcaaggtcttttcacctggcccgcatggacacccagaccaggtggggtacatcgtgacctgggaagccttggcttttgacccccctccctgggtcaagccctttgtacaccctaagcctccgcctcctcttcctccatccgccccgtctctcccccttgaacctcctcgttcgaccccgcctcgatcctccctttatccagccctcactccttctctaggcgcccccatatggccatatgagatcttatatggggcacccccgccccttgtaaacttccctgaccctgacatgacaagagttactaacagcccctctctccaagctcacttacaggctctctacttagtccagcacgaagtctggagacctctggcggcagcctaccaagaacaactggaccgaccggtggtacctcacccttaccgagtcggcgacacagtgtgggtccgccgacaccagactaagaacctagaacctcgctggaaaggaccttacacagtcctgctgaccacccccaccgccctcaaagtagacggcatcgcagcttggatacacgccgcccacgtgaaggctgccgaccccgggggtggaccatcctctagactgccatgctcgagggagtgcaggtggaaaccatctccccaggagacgggcgcaccttccccaagcgcggccagacctgcgtggtgcactacaccgggatgcttgaagatggaaagaaagttgattcctcccgggacagaaacaagccctttaagtttatgctaggcaagcaggaggtgatccgaggctgggaagaaggggttgcccagatgagtgtgggtcagagagccaaactgactatatctccagattatgcctatggtgccactgggcacccaggcatcatcccaccacatgccactctcgtcttcgatgtggagcttctaaaactggaatctggcggtggatccggagtcgacggatttggtgatgtcggtgctcttgagagtttgaggggaaatgcagatttggcttacatcctgagcatggagccctgtggccactgcctcattatcaacaatgtgaacttctgccgtgagtccgggctccgcacccgcactggctccaacatcgactgtgagaagttgcggcgtcgcttctcctcgctgcatttcatggtggaggtgaagggcgacctgactgccaagaaaatggtgctggctttgctggagctggcgcagcaggaccacggtgctctggactgctgcgtggtggtcattctctctcacggctgtcaggccagccacctgcagttcccaggggctgtctacggcacagatggatgccctgtgtcggtcgagaagattgtgaacatcttcaatgggaccagctgccccagcctgggagggaagcccaagctctttttcatccaggcctgtggtggggagcagaaagaccatgggtttgaggtggcctccacttcccctgaagacgagtcccctggcagtaaccccgagccagatgccaccccgttccaggaaggtttgaggaccttcgaccagctggacgccatatctagtttgcccacacccagtgacatctttgtgtcctactctactttcccaggttttgtttcctggagggaccccaagagtggctcctggtacgttgagaccctggacgacatctttgagcagtgggctcactctgaagacctgcagtccctcctgcttagggtcgctaatgctgtttcggtgaaagggatttataaacagatgcctggttgctttaatttcctccggaaaaaacttttctttaaaacatcagctagcagagccgagggcaggggaagtcttctaacatgcggggacgtggaggaaaatcccgggcccatggagttcggcttgagttggttgttccttgtggcgatactcaaaggcgttcaatgtagccgagacataaaaatgacccagtctccgtcatctatgtatgcaagcctcggcgagcgagtgaccatcacgtgcaaggcgagtcaagatataaacagctacttgtcatggttccaacaaaaaccagggaaatcacctaagaccctgatctatagagccaatcgcctggttgacggtgtcccctcccgctttagcggctccggaagcggtcaagattactctctcacaatttcttccttggattatgaagacatggggatctactattgtcaacagtatgacgaatccccgtggactttcggtggcggtaccaaattggaaataaagggctctacaagcggctcaggaaaacctggatcaggcgaagggtctacgaagggccagatacaactcgttcaaagtgggccagaactcaaaaaaccgggagaaacagtgaaaatttcttgtaaggcatcaggatacacattcacaaactacgggatgaattgggtcaaacaagcacccggaaaggggctgcgctggatggggtggatcaacacacatactggggaacctacttacgcagacgatttcaagggcagattcgccttttctttggagacctccgcctctactgcatacttgcagataaacaacctgaagaatgaagataccgccacctacttctgtacgcgcaggggctacgattggtattttgatgtatggggggcaggcaccactgttactgtgtcaagctacgtcaccgtctcttcacaggatcccgccctggaagagaagaaaggcaattacgtcgtgaccgaccacggcagctgtgtgcgggcttgtggcgccgatagctacgagatggaagaggacggcgtgcggaagtgcaagaagtgcgagggcccctgcagaaaagtgtgcaacggcatcggcatcggagagttcaaggatagcctgagcatcaacgccaccaacatcaagcacttcaagaactgcaccagcatcagcggcgacctgcacatcctgcccgtggcctttagaggcgacagcttcacccacacccccccactggatccccaggaactggacatcctgaaaaccgtgaaagagatcacaggctttctgctgattcaggcctggcccgagaaccggacagacctgcacgccttcgagaacctggaaatcatcagaggccggaccaagcagcacggccagttttctctggccgtggtgtccctgaacatcaccagcctgggcctgcggagcctgaaagaaatcagcgacggcgacgtgatcatctccggcaacaagaacctgtgctacgccaacaccatcaattggaagaagctgttcggcacctccggccagaaaacaaagatcatctctaaccggggcgagaacagctgcaaagccaccggacaagtgtgccacgccctgtgtagccctgagggctgttggggacccgagcccagagattgcgtgtcctgccggaatgtgtccagaggccgcgagtgcgtggacaagtgcaacctgctggaaggcgagccccgcgagtttgtggaaaacagcgagtgcatccagtgccaccccgagtgtctgccccaggccatgaacattacctgcaccggcagaggccccgacaactgtatccagtgcgcccactacatcgacggcccccactgcgtgaaaacctgtccagctggcgtgatgggagagaacaacaccctcgtgtggaagtacgccgacgccggccatgtgtgccacctgtgtcaccccaattgcacctacggctgtaccggccctggcctggaaggctgtcctaccaacggccccaagatcccttctaaagatcccaaattttgggtgctggtggtggttggtggagtcctggcttgctatagcttgctagtaacagtggcctttattattttctgggtgaggagtaagaggagcaggctcctgcacagtgactacatgaacatgactccccgccgccccgggcccacccgcaagcattaccagccctatgccccaccacgcgacttcgcagcctatcgctccagagtgaagttcagcaggagcgcagacgcccccgcgtaccagcagggccagaaccagctctataacgagctcaatctaggacgaagagaggagtacgatgttttggacaagagacgtggccgggaccctgagatggggggaaagccgagaaggaagaaccctcaggaaggcctgtacaatgaactgcagaaagataagatggcggaggcctacagtgagattgggatgaaaggcgagcgccggaggggcaaggggcacgatggcctttaccagggtctcagtacagccaccaaggacacctacgacgcccttcacatgcaggccctgccccctcgcggaccgcagtgtactaattatgctctcttgaaattggctggagatgttgagagcaatcccgggcccatgcggatcagcaagccccacctgcggagcatcagcatccagtgctacctgtgcctgctgctgaacagccacttcctgaccgaggccggcatccacgtgttcatcctgggctgcttcagcgccggactgcccaagaccgaggccaactgggtgaacgtgatcagcgacctgaagaagatcgaggacctgatccagagcatgcacatcgacgccaccctgtacaccgagagcgacgtgcaccccagctgcaaggtgaccgccatgaagtgctttctgctggaactgcaggtgatcagcctggaaagcggcgacgccagcatccacgacaccgtggagaacctgatcatcctggccaacaacagcctgagcagcaacggcaacgtgaccgagagcggctgcaaagagtgcgaggaactggaagagaagaacatcaaagagtttctgcagagcttcgtgcacatcgtgcagatgttcatcaacaccagctgacgcgtcatcatcgatccggattagtccaatttgttaaagacaggatatcagtggtccaggctctagttttgactcaacaatatcaccagctgaagcctatagagtacgagccatagataaaataaaagattttatttagtctccagaaaaaggggggaatgaaagaccccacctgtaggtttggcaagctagcttaagtaacgccattttgcaaggcatggaaaaatacataactgagaatagagaagttcagatcaaggtcaggaacagatggaacagctgaatatgggccaaacaggatatctgtggtaagcagttcctgccccggctcagggccaagaacagatggaacagctgaatatgggccaaacaggatatctgtggtaagcagttcctgccccggctcagggccaagaacagatggtccccagatgcggtccagccctcagcagtttctagagaaccatcagatgtttccagggtgccccaaggacctgaaatgaccctgtgccttatttgaactaaccaatcagttcgcttctcgcttctgttcgcgcgcttctgctccccgagctcaataaaagagcccacaacccctcactcggggcgccagtcctccgattgactgagtcgcccgggtacccgtgtatccaataaaccctcttgcagttgcatccgacttgtggtctcgctgttccttgggagggtctcctctgagtgattgactacccgtcagcgggggtctttcacacatgcagcatgtatcaaaattaatttggttttttttcttaagtatttacattaaatggccatagtacttaaagttacattggcttccttgaaataaacatggagtattcagaatgtgtcataaatatttctaattttaagatagtatctccattggctttctactttttcttttatttttttttgtcctctgtcttccatttgttgttgttgttgtttgtttgtttgtttgttggttggttggttaatttttttttaaagatcctacactatagttcaagctagactattagctactctgtaacccagggtgaccttgaagtcatgggtagcctgctgttttagccttcccacatctaagattacaggtatgagctatcatttttggtatattgattgattgattgattgatgtgtgtgtgtgtgattgtgtttgtgtgtgtgactgtgaaaatgtgtgtatgggtgtgtgtgaatgtgtgtatgtatgtgtgtgtgtgagtgtgtgtgtgtgtgtgtgcatgtgtgtgtgtgtgactgtgtctatgtgtatgactgtgtgtgtgtgtgtgtgtgtgtgtgtgtgtgtgtgtgtgtgtgtgttgtgaaaaaatattctatggtagtgagagccaacgctccggctcaggtgtcaggttggtttttgagacagagtctttcacttagcttggaattcactggccgtcgttttacaacgtcgtgactgggaaaaccctggcgttacccaacttaatcgccttgcagcacatccccctttcgccagctggcgtaatagcgaagaggcccgcaccgatcgcccttcccaacagttgcgcagcctgaatggcgaatggcgcctgatgcggtattttctccttacgcatctgtgcggtatttcacaccgcatatggtgcactctcagtacaatctgctctgatgccgcatagttaagccagccccgacacccgccaacacccgctgacgcgccctgacgggcttgtctgctcccggcatccgcttacagacaagctgtgaccgtctccgggagctgcatgtgtcagaggttttcaccgtcatcaccgaaacgcgcgagacgaaagggcctcgtgatacgcctatttttataggttaatgtcatgataataatggtttcttagacgtcaggtggcacttttcggggaaatgtgcgcggaacccctatttgtttatttttctaaatacattcaaatatgtatccgctcatgagacaataaccctgataaatgcttcaataatattgaaaaaggaagagtatgagtattcaacatttccgtgtcgcccttattcccttttttgcggcattttgccttcctgtttttgctcacccagaaacgctggtgaaagtaaaagatgctgaagatcagttgggtgcacgagtgggttacatcgaactggatctcaacagcggtaagatccttgagagttttcgccccgaagaacgttttccaatgatgagcacttttaaagttctgctatgtggcgcggtattatcccgtattgacgccgggcaagagcaactcggtcgccgcatacactattctcagaatgacttggttgagtactcaccagtcacagaaaagcatcttacggatggcatgacagtaagagaattatgcagtgctgccataaccatgagtgataacactgcggccaacttacttctgacaacgatcggaggaccgaaggagctaaccgcttttttgcacaacatgggggatcatgtaactcgccttgatcgttgggaaccggagctgaatgaagccataccaaacgacgagcgtgacaccacgatgcctgtagcaatggcaacaacgttgcgcaaactattaactggcgaactacttactctagcttcccggcaacaattaatagactggatggaggcggataaagttgcaggaccacttctgcgctcggcccttccggctggctggtttattgctgataaatctggagccggtgagcgtgggtctcgcggtatcattgcagcactggggccagatggtaagccctcccgtatcgtagttatctacacgacggggagtcaggcaactatggatgaacgaaatagacagatcgctgagataggtgcctcactgattaagcattggtaactgtcagaccaagtttactcatatatactttagattgatttaaaacttcatttttaatttaaaaggatctaggtgaagatcctttttgataatctcatgaccaaaatcccttaacgtgagttttcgttccactgagcgtcagaccccgtagaaaagatcaaaggatcttcttgagatcctttttttctgcgcgtaatctgctgcttgcaaacaaaaaaaccaccgctaccagcggtggtttgtttgccggatcaagagctaccaactctttttccgaaggtaactggcttcagcagagcgcagataccaaatactgttcttctagtgtagccgtagttaggccaccacttcaagaactctgtagcaccgcctacatacctcgctctgctaatcctgttaccagtggctgctgccagtggcgataagtcgtgtcttaccgggttggactcaagacgatagttaccggataaggcgcagcggtcgggctgaacggggggttcgtgcacacagcccagcttggagcgaacgacctacaccgaactgagatacctacagcgtgagctatgagaaagcgccacgcttcccgaagggagaaaggcggacaggtatccggtaagcggcagggtcggaacaggagagcgcacgagggagcttccagggggaaacgcctggtatctttatagtcctgtcgggtttcgccacctctgacttgagcgtcgatttttgtgatgctcgtcaggggggcggagcctatggaaaaacgccagcaacgcggcctttttacggttcctggccttttgctggccttttgctcacatgttctttcctgcgttatcccctgattctgtggataaccgtattaccgcctttgagtgagctgataccgctcgccgcagccgaacgaccgagcgcagcgagtcagtgagcgaggaagcggaagagcgcccaatacgcaaaccgcctctccccgcgcgttggccgattcattaatgcagctggcacgacaggtttcccgactggaaagcgggcagtgagcgcaacgcaattaatgtgagttagctcactcattaggcaccccaggctttacactttatgcttccggctcgtatgttgtgtggaattgtgagcggataacaatttcacacaggaaacagctatgaccatgattacgccaagctttgctcttaggagtttcctaatacatcccaaactcaaatatataaagcatttgacttgttctatgccctagggggcggggggaagctaagccagctttttttaacatttaaaatgttaattccattttaaatgcacagatgtttttatttcataagggtttcaatgtgcatgaatgctgcaatattcctgttaccaaagctagtataaataaaaatagataaacgtggaaattacttagagtttctgtcattaacgtttccttcctcagttgacaacataaatgcgctgctgagcaagccagtttgcatctgtcaggatcaatttcccattatgccagtcatattaattactagtcaattagttgatttttatttttgacatatacatgtg

SEQ ID NO: 47 - DNA, 10610 bp, synthetic construct
  misc_feature 1..10610: note = pSFG4-hCD5-Ev3-CAR
  source 1..10610: mol_type = other DNA
aatgaaagaccccacctgtaggtttggcaagctagcttaagtaacgccattttgcaaggcatggaaaaatacataactgagaatagaaaagttcagatcaaggtcaggaacagatggaacagctgaatatgggccaaacaggatatctgtggtaagcagttcctgccccggctcagggccaagaacagatggaacagctgaatatgggccaaacaggatatctgtggtaagcagttcctgccccggctcagggccaagaacagatggtccccagatgcggtccagccctcagcagtttctagagaaccatcagatgtttccagggtgccccaaggacctgaaatgaccctgtgccttatttgaactaaccaatcagttcgcttctcgcttctgttcgcgcgcttatgctccccgagctcaataaaagagcccacaacccctcactcggggcgccagtcctccgattgactgagtcgcccgggtacccgtgtatccaataaaccctcttgcagttgcatccgacttgtggtctcgctgttccttgggagggtctcctctgagtgattgactacccgtcagcgggggtctttcatttgggggctcgtccgggatcgggagacccctgcccagggaccaccgacccaccaccgggaggtaagctggccagcaacttatctgtgtctgtccgattgtctagtgtctatgactgattttatgcgcctgcgtcggtactagttagctaactagctctgtatctggcggacccgtggtggaactgacgagttcggaacacccggccgcaaccctgggagacgtcccagggacttcgggggccgtttttgtggcccgacctgagtcctaaaatcccgatcgtttaggactctttggtgcaccccccttagaggagggatatgtggttctggtaggagacgagaacctaaaacagttcccgcctccgtctgaatttttgctttcggtttgggaccgaagccgcgccgcgcgtcttgtctgctgcagcatcgttctgtgttgtctctgtctgactgtgtttctgtatttgtctgaaaatatgggcccgggctagcctgttaccactcccttaagtttgaccttaggtcactggaaagatgtcgagcggatcgctcacaaccagtcggtagatgtcaagaagagacgttgggttaccttctgctctgcagaatggccaacctttaacgtcggatggccgcgagacggcacctttaaccgagacctcatcacccaggttaagatcaaggtcttttcacctggcccgcatggacacccagaccaggtggggtacatcgtgacctgggaagccttggcttttgacccccctccctgggtcaagccctttgtacaccctaagcctccgcctcctcttcctccatccgccccgtctctcccccttgaacctcctcgttcgaccccgcctcgatcctccctttatccagccctcactccttctctaggcgcccccatatggccatatgagatcttatatggggcacccccgccccttgtaaacttccctgaccctgacatgacaagagttactaacagcccctctctccaagctcacttacaggctctctacttagtccagcacgaagtctggagacctctggcggcagcctaccaagaacaactggaccgaccggtggtacctcacccttaccgagtcggcgacacagtgtgggtccgccgacaccagactaagaacctagaacctcgctggaaaggaccttacacagtcctgctgaccacccccaccgccctcaaagtagacggcatcgcagcttggatacacgccgcccacgtgaaggctgccgaccccgggggtggaccatcctctagactgccatgctcgagggagtgcaggtggaaaccatctccccaggagacgggcgcaccttccccaagcgcggccagacctgcgtggtgcactacaccgggatgcttgaagatggaaagaaagttgattcctcccgggacagaaacaagccctttaagtttatgctaggcaagcaggaggtgatccgaggctgggaagaaggggttgcccagatgagtgtgggtcagagagccaaactgactatatctccagattatgcctatggtgccactgggcacccaggcatcatcccaccacatgccactctcgtcttcgatgtggagcttctaaaactggaatctggcggtggatccggagtcgacggatttggtgatgtcggtgctcttgagagtttgaggggaaatgcagatttggcttacatcctgagcatggagccctgtggccactgcctcattatcaacaatgtgaacttctgccgtgagtccgggctccgcacccgcactggctccaacatcgactgtgagaagttgcggcgtcgcttctcctcgctgcatttcatggtggaggtgaagggcgacctgactgccaagaaaatggtgctggctttgctggagctggcgcagcaggaccacggtgctctggactgctgcgtggtggtcattctctctcacggctgtcaggccagccacctgcagttcccaggggctgtctacggcacagatggatgccctgtgtcggtcgagaagattgtgaacatcttcaatgggaccagctgccccagcctgggagggaagcccaagctctttttcatccaggcctgtggtggggagcagaaagaccatgggtttgaggtggcctccacttcccctgaagacgagtcccctggcagtaaccccgagccagatgccaccccgttccaggaaggtttgaggaccttcgaccagctggacgccatatctagtttgcccacacccagtgacatctttgtgtcctactctactttcccaggttttgtttcctggagggaccccaagagtggctcctggtacgttgagaccctggacgacatctttgagcagtgggctcactctgaagacctgcagtccctcctgcttagggtcgctaatgctgtttcggtgaaagggatttataaacagatgcctggttgctttaatttcctccggaaaaaacttttctttaaaacatcagctagcagagccgagggcaggggaagtcttctaacatgcggggacgtggaggaaaatcccgggcccatggagttcggtctcagttggctgtttttggttgctatcttgaagggcgtccaatgcagccgggacatccagatgacccagtctccctctagcatgtcagcgagtcttggtgatcgagtgacgattacctgcagagcctctcaagatataaacagctatctttcatggttccaacagaagccggggaagtccccaaaaactctcatatacagggcgaatcgactcgtagacggtgtgccttcaaggttttccgggagtggtagtggcacagattacacacttacaatctcttcattgcagtatgaggatttcgggatctactactgtcaacagtacgacgaatccccatggacgtttgggggcgggaccaaacttgagataaaagggagcacatctggaagtggtaaacctgggtcaggggagggttccacaaaaggacaaattcaacttgtccaaagcggtcctggtcttaagaagcctggagggtctgtcaggataagttgtgcggcatccggctacaccttcaccaactatgggatgaactgggtgaaacaagcgcctgggaaaggtcttcgatggatgggctggattaatacccacactggagagcccacttacgctgatgatttcaaaggacgatttaccttctccttggatacttccaagagtaccgcgtacttgcaaatcaacagtctccgggctgaagacacggccacatacttctgtacgcggagagggtatgactggtattttgatgtgtggggtcagggaacaaccgtgactgtttcaagctacgtcaccgtctcttcacaggatcccgccctggaagagaagaaaggcaattacgtcgtgaccgaccacggcagctgtgtgcgggcttgtggcgccgatagctacgagatggaagaggacggcgtgcggaagtgcaagaagtgcgagggcccctgcagaaaagtgtgcaacggcatcggcatcggagagttcaaggatagcctgagcatcaacgccaccaacatcaagcacttcaagaactgcaccagcatcagcggcgacctgcacatcctgcccgtggcctttagaggcgacagcttcacccacacccccccactggatccccaggaactggacatcctgaaaaccgtgaaagagatcacaggctttctgctgattcaggcctggcccgagaaccggacagacctgcacgccttcgagaacctggaaatcatcagaggccggaccaagcagcacggccagttttctctggccgtggtgtccctgaacatcaccagcctgggcctgcggagcctgaaagaaatcagcgacggcgacgtgatcatctccggcaacaagaacctgtgctacgccaacaccatcaattggaagaagctgttcggcacctccggccagaaaacaaagatcatctctaaccggggcgagaacagctgcaaagccaccggacaagtgtgccacgccctgtgtagccctgagggctgttggggacccgagcccagagattgcgtgtcctgccggaatgtgtccagaggccgcgagtgcgtggacaagtgcaacctgctggaaggcgagccccgcgagtttgtggaaaacagcgagtgcatccagtgccaccccgagtgtctgccccaggccatgaacattacctgcaccggcagaggccccgacaactgtatccagtgcgcccactacatcgacggcccccactgcgtgaaaacctgtccagctggcgtgatgggagagaacaacaccctcgtgtggaagtacgccgacgccggccatgtgtgccacctgtgtcaccccaattgcacctacggctgtaccggccctggcctggaaggctgtcctaccaacggccccaagatcccttctaaagatcccaaattttgggtgctggtggtggttggtggagtcctggcttgctatagcttgctagtaacagtggcctttattattttctgggtgaggagtaagaggagcaggctcctgcacagtgactacatgaacatgactccccgccgccccgggcccacccgcaagcattaccagccctatgccccaccacgcgacttcgcagcctatcgctccagagtgaagttcagcaggagcgcagacgcccccgcgtaccagcagggccagaaccagctctataacgagctcaatctaggacgaagagaggagtacgatgttttggacaagagacgtggccgggaccctgagatggggggaaagccgagaaggaagaaccctcaggaaggcctgtacaatgaactgcagaaagataagatggcggaggcctacagtgagattgggatgaaaggcgagcgccggaggggcaaggggcacgatggcctttaccagggtctcagtacagccaccaaggacacctacgacgcccttcacatgcaggccctgccccctcgcggaccgcagtgtactaattatgctctcttgaaattggctggagatgttgagagcaatcccgggcccatgcggatcagcaagccccacctgcggagcatcagcatccagtgctacctgtgcctgctgctgaacagccacttcctgaccgaggccggcatccacgtgttcatcctgggctgcttcagcgccggactgcccaagaccgaggccaactgggtgaacgtgatcagcgacctgaagaagatcgaggacctgatccagagcatgcacatcgacgccaccctgtacaccgagagcgacgtgcaccccagctgcaaggtgaccgccatgaagtgctttctgctggaactgcaggtgatcagcctggaaagcggcgacgccagcatccacgacaccgtggagaacctgatcatcctggccaacaacagcctgagcagcaacggcaacgtgaccgagagcggctgcaaagagtgcgaggaactggaagagaagaacatcaaagagtttctgcagagcttcgtgcacatcgtgcagatgttcatcaacaccagctgacgcgtcatcatcgatccggattagtccaatttgttaaagacaggatatcagtggtccaggctctagttttgactcaacaatatcaccagctgaagcctatagagtacgagccatagataaaataaaagattttatttagtctccagaaaaaggggggaatgaaagaccccacctgtaggtttggcaagctagcttaagtaacgccattttgcaaggcatggaaaaatacataactgagaatagagaagttcagatcaaggtcaggaacagatggaacagctgaatatgggccaaacaggatatctgtggtaagcagttcctgccccggctcagggccaagaacagatggaacagctgaatatgggccaaacaggatatctgtggtaagcagttcctgccccggctcagggccaagaacagatggtccccagatgcggtccagccctcagcagtttctagagaaccatcagatgtttccagggtgccccaaggacctgaaatgaccctgtgccttatttgaactaaccaatcagttcgcttctcgcttctgttcgcgcgcttctgctccccgagctcaataaaagagcccacaacccctcactcggggcgccagtcctccgattgactgagtcgcccgggtacccgtgtatccaataaaccctcttgcagttgcatccgacttgtggtctcgctgttccttgggagggtctcctctgagtgattgactacccgtcagcgggggtctttcacacatgcagcatgtatcaaaattaatttggttttttttcttaagtatttacattaaatggccatagtacttaaagttacattggcttccttgaaataaacatggagtattcagaatgtgtcataaatatttctaattttaagatagtatctccattggctttctactttttcttttatttttttttgtcctctgtcttccatttgttgttgttgttgtttgtttgtttgtttgttggttggttggttaatttttttttaaagatcctacactatagttcaagctagactattagctactctgtaacccagggtgaccttgaagtcatgggtagcctgctgttttagccttcccacatctaagattacaggtatgagctatcatttttggtatattgattgattgattgattgatgtgtgtgtgtgtgattgtgtttgtgtgtgtgactgtgaaaatgtgtgtatgggtgtgtgtgaatgtgtgtatgtatgtgtgtgtgtgagtgtgtgtgtgtgtgtgtgcatgtgtgtgtgtgtgactgtgtctatgtgtatgactgtgtgtgtgtgtgtgtgtgtgtgtgtgtgtgtgtgtgtgtgtgtgttgtgaaaaaatattctatggtagtgagagccaacgctccggctcaggtgtcaggttggtttttgagacagagtctttcacttagcttggaattcactggccgtcgttttacaacgtcgtgactgggaaaaccctggcgttacccaacttaatcgccttgcagcacatccccctttcgccagctggcgtaatagcgaagaggcccgcaccgatcgcccttcccaacagttgcgcagcctgaatggcgaatggcgcctgatgcggtattttctccttacgcatctgtgcggtatttcacaccgcatatggtgcactctcagtacaatctgctctgatgccgcatagttaagccagccccgacacccgccaacacccgctgacgcgccctgacgggcttgtctgctcccggcatccgcttacagacaagctgtgaccgtctccgggagctgcatgtgtcagaggttttcaccgtcatcaccgaaacgcgcgagacgaaagggcctcgtgatacgcctatttttataggttaatgtcatgataataatggtttcttagacgtcaggtggcacttttcggggaaatgtgcgcggaacccctatttgtttatttttctaaatacattcaaatatgtatccgctcatgagacaataaccctgataaatgcttcaataatattgaaaaaggaagagtatgagtattcaacatttccgtgtcgcccttattcccttttttgcggcattttgccttcctgtttttgctcacccagaaacgctggtgaaagtaaaagatgctgaagatcagttgggtgcacgagtgggttacatcgaactggatctcaacagcggtaagatccttgagagttttcgccccgaagaacgttttccaatgatgagcacttttaaagttctgctatgtggcgcggtattatcccgtattgacgccgggcaagagcaactcggtcgccgcatacactattctcagaatgacttggttgagtactcaccagtcacagaaaagcatcttacggatggcatgacagtaagagaattatgcagtgctgccataaccatgagtgataacactgcggccaacttacttctgacaacgatcggaggaccgaaggagctaaccgcttttttgcacaacatgggggatcatgtaactcgccttgatcgttgggaaccggagctgaatgaagccataccaaacgacgagcgtgacaccacgatgcctgtagcaatggcaacaacgttgcgcaaactattaactggcgaactacttactctagcttcccggcaacaattaatagactggatggaggcggataaagttgcaggaccacttctgcgctcggcccttccggctggctggtttattgctgataaatctggagccggtgagcgtgggtctcgcggtatcattgcagcactggggccagatggtaagccctcccgtatcgtagttatctacacgacggggagtcaggcaactatggatgaacgaaatagacagatcgctgagataggtgcctcactgattaagcattggtaactgtcagaccaagtttactcatatatactttagattgatttaaaacttcatttttaatttaaaaggatctaggtgaagatcctttttgataatctcatgaccaaaatcccttaacgtgagttttcgttccactgagcgtcagaccccgtagaaaagatcaaaggatcttcttgagatcctttttttctgcgcgtaatctgctgcttgcaaacaaaaaaaccaccgctaccagcggtggtttgtttgccggatcaagagctaccaactctttttccgaaggtaactggcttcagcagagcgcagataccaaatactgttcttctagtgtagccgtagttaggccaccacttcaagaactctgtagcaccgcctacatacctcgctctgctaatcctgttaccagtggctgctgccagtggcgataagtcgtgtcttaccgggttggactcaagacgatagttaccggataaggcgcagcggtcgggctgaacggggggttcgtgcacacagcccagcttggagcgaacgacctacaccgaactgagatacctacagcgtgagctatgagaaagcgccacgcttcccgaagggagaaaggcggacaggtatccggtaagcggcagggtcggaacaggagagcgcacgagggagcttccagggggaaacgcctggtatctttatagtcctgtcgggtttcgccacctctgacttgagcgtcgatttttgtgatgctcgtcaggggggcggagcctatggaaaaacgccagcaacgcggcctttttacggttcctggccttttgctggccttttgctcacatgttctttcctgcgttatcccctgattctgtggataaccgtattaccgcctttgagtgagctgataccgctcgccgcagccgaacgaccgagcgcagcgagtcagtgagcgaggaagcggaagagcgcccaatacgcaaaccgcctctccccgcgcgttggccgattcattaatgcagctggcacgacaggtttcccgactggaaagcgggcagtgagcgcaacgcaattaatgtgagttagctcactcattaggcaccccaggctttacactttatgcttccggctcgtatgttgtgtggaattgtgagcggataacaatttcacacaggaaacagctatgaccatgattacgccaagctttgctcttaggagtttcctaatacatcccaaactcaaatatataaagcatttgacttgttctatgccctagggggcggggggaagctaagccagctttttttaacatttaaaatgttaattccattttaaatgcacagatgtttttatttcataagggtttcaatgtgcatgaatgctgcaatattcctgttaccaaagctagtataaataaaaatagataaacgtggaaattacttagagtttctgtcattaacgtttccttcctcagttgacaacataaatgcgctgctgagcaagccagtttgcatctgtcaggatcaatttcccattatgccagtcatattaattactagtcaattagttgatttttatttttgacatatacatgtg

SEQ ID NO: 48 - DNA, 10274 bp, synthetic construct
  misc_feature 1..10274: note = pSFG4-CD19-DAP12-CAR
  source 1..10274: mol_type = other DNA
aatgaaagaccccacctgtaggtttggcaagctagcttaagtaacgccattttgcaaggcatggaaaaatacataactgagaatagaaaagttcagatcaaggtcaggaacagatggaacagctgaatatgggccaaacaggatatctgtggtaagcagttcctgccccggctcagggccaagaacagatggaacagctgaatatgggccaaacaggatatctgtggtaagcagttcctgccccggctcagggccaagaacagatggtccccagatgcggtccagccctcagcagtttctagagaaccatcagatgtttccagggtgccccaaggacctgaaatgaccctgtgccttatttgaactaaccaatcagttcgcttctcgcttctgttcgcgcgcttatgctccccgagctcaataaaagagcccacaacccctcactcggggcgccagtcctccgattgactgagtcgcccgggtacccgtgtatccaataaaccctcttgcagttgcatccgacttgtggtctcgctgttccttgggagggtctcctctgagtgattgactacccgtcagcgggggtctttcatttgggggctcgtccgggatcgggagacccctgcccagggaccaccgacccaccaccgggaggtaagctggccagcaacttatctgtgtctgtccgattgtctagtgtctatgactgattttatgcgcctgcgtcggtactagttagctaactagctctgtatctggcggacccgtggtggaactgacgagttcggaacacccggccgcaaccctgggagacgtcccagggacttcgggggccgtttttgtggcccgacctgagtcctaaaatcccgatcgtttaggactctttggtgcaccccccttagaggagggatatgtggttctggtaggagacgagaacctaaaacagttcccgcctccgtctgaatttttgctttcggtttgggaccgaagccgcgccgcgcgtcttgtctgctgcagcatcgttctgtgttgtctctgtctgactgtgtttctgtatttgtctgaaaatatgggcccgggctagcctgttaccactcccttaagtttgaccttaggtcactggaaagatgtcgagcggatcgctcacaaccagtcggtagatgtcaagaagagacgttgggttaccttctgctctgcagaatggccaacctttaacgtcggatggccgcgagacggcacctttaaccgagacctcatcacccaggttaagatcaaggtcttttcacctggcccgcatggacacccagaccaggtggggtacatcgtgacctgggaagccttggcttttgacccccctccctgggtcaagccctttgtacaccctaagcctccgcctcctcttcctccatccgccccgtctctcccccttgaacctcctcgttcgaccccgcctcgatcctccctttatccagccctcactccttctctaggcgcccccatatggccatatgagatcttatatggggcacccccgccccttgtaaacttccctgaccctgacatgacaagagttactaacagcccctctctccaagctcacttacaggctctctacttagtccagcacgaagtctggagacctctggcggcagcctaccaagaacaactggaccgaccggtggtacctcacccttaccgagtcggcgacacagtgtgggtccgccgacaccagactaagaacctagaacctcgctggaaaggaccttacacagtcctgctgaccacccccaccgccctcaaagtagacggcatcgcagcttggatacacgccgcccacgtgaaggctgccgaccccgggggtggaccatcctctagactgccatgctcgagggagtgcaggtggaaaccatctccccaggagacgggcgcaccttccccaagcgcggccagacctgcgtggtgcactacaccgggatgcttgaagatggaaagaaagttgattcctcccgggacagaaacaagccctttaagtttatgctaggcaagcaggaggtgatccgaggctgggaagaaggggttgcccagatgagtgtgggtcagagagccaaactgactatatctccagattatgcctatggtgccactgggcacccaggcatcatcccaccacatgccactctcgtcttcgatgtggagcttctaaaactggaatctggcggtggatccggagtcgacggatttggtgatgtcggtgctcttgagagtttgaggggaaatgcagatttggcttacatcctgagcatggagccctgtggccactgcctcattatcaacaatgtgaacttctgccgtgagtccgggctccgcacccgcactggctccaacatcgactgtgagaagttgcggcgtcgcttctcctcgctgcatttcatggtggaggtgaagggcgacctgactgccaagaaaatggtgctggctttgctggagctggcgcagcaggaccacggtgctctggactgctgcgtggtggtcattctctctcacggctgtcaggccagccacctgcagttcccaggggctgtctacggcacagatggatgccctgtgtcggtcgagaagattgtgaacatcttcaatgggaccagctgccccagcctgggagggaagcccaagctctttttcatccaggcctgtggtggggagcagaaagaccatgggtttgaggtggcctccacttcccctgaagacgagtcccctggcagtaaccccgagccagatgccaccccgttccaggaaggtttgaggaccttcgaccagctggacgccatatctagtttgcccacacccagtgacatctttgtgtcctactctactttcccaggttttgtttcctggagggaccccaagagtggctcctggtacgttgagaccctggacgacatctttgagcagtgggctcactctgaagacctgcagtccctcctgcttagggtcgctaatgctgtttcggtgaaagggatttataaacagatgcctggttgctttaatttcctccggaaaaaacttttctttaaaacatcagctagcagagccgagggcaggggaagtcttctaacatgcggggacgtggaggaaaatcccgggcccatggagtttgggctgagctggctttttcttgtggctattttaaaaggtgtccagtgctctagagacatccagatgacacagactacatcctccctgtctgcctctctgggagacagagtcaccatcagttgcagggcaagtcaggacattagtaaatatttaaattggtatcagcagaaaccagatggaactgttaaactcctgatctaccatacatcaagattacactcaggagtcccatcaaggttcagtggcagtgggtctggaacagattattctctcaccattagcaacctggagcaagaagatattgccacttacttttgccaacagggtaatacgcttccgtacacgttcggaggggggaccaagctggagctgaaacgtggtggtggtggttctggtggtggtggttctggcggcggcggctccggtggtggtggatccgaggtgcagctgcagcagtctggacctggcctggtggcgccctcacagagcctgtccgtcacatgcactgtctcaggggtctcattacccgactatggtgtaagctggattcgccagcctccacgaaagggtctggagtggctgggagtaatatggggtagtgaaaccacatactataattcagctctcaaatccagactgaccatcatcaaggacaactccaagagccaagttttcttaaaaatgaacagtctgcaaactgatgacacagccatttactactgtgccaaacattattactacggtggtagctatgctatggactactggggccaagggaccacggtcaccgtctcctcgtacgtcaccgtctcttcacaggatcccgccgagcccaaatctcctgacaaaactcacacatgcccaccgtgcccagcacctgaactcctggggggaccgtcagtcttcctcttccccccaaaacccaaggacaccctcatgatctcccggacccctgaggtcacatgcgtggtggtggacgtgagccacgaagaccctgaggtcaagttcaactggtacgtggacggcgtggaggtgcataatgccaagacaaagccgcgggaggagcagtacaacagcacgtaccgtgtggtcagcgtcctcaccgtcctgcaccaggactggctgaatggcaaggagtacaagtgcaaggtctccaacaaagccctcccagcccccatcgagaaaaccatctccaaagccaaagggcagccccgagaaccacaggtgtacaccctgcccccatcccgggatgagctgaccaagaaccaggtcagcctgacctgcctggtcaaaggcttctatcccagcgacatcgccgtggagtgggagagcaatgggcaaccggagaacaactacaagaccacgcctcccgtgctggactccgacggctccttcttcctctacagcaagctcaccgtggacaagagcaggtggcagcaggggaacgtcttctcatgctccgtgatgcatgaggctctgcacaaccactacacgcagaagagcctctccctgtctccgggtaaaaaagatcccaaaggcgtgctggccggaatcgtgatgggcgacctggtgctgacagtgctgatcgccctggctgtgtacttcctgggcagactggtgcccagaggaagaggcgctgccgaagccgccacccggaagcagagaatcaccgagacagagagcccctatcaggaactgcagggccagcggagcgacgtgtacagcgacctgaatacccagcggccctactacaagagagtgaagttcagcaggagcgcagacgcccccgcgtaccagcagggccagaaccagctctataacgagctcaatctaggacgaagagaggagtacgatgttttggacaagagacgtggccgggaccctgagatggggggaaagccgagaaggaagaaccctcaggaaggcctgtacaatgaactgcagaaagataagatggcggaggcctacagtgagattgggatgaaaggcgagcgccggaggggcaaggggcacgatggcctttaccagggtctcagtacagccaccaaggacacctacgacgcccttcacatgcaggccctgccccctcgcggaccgcagtgtactaattatgctctcttgaaattggctggagatgttgagagcaatcccgggcccatgcggatcagcaagccccacctgcggagcatcagcatccagtgctacctgtgcctgctgctgaacagccacttcctgaccgaggccggcatccacgtgttcatcctgggctgcttcagcgccggactgcccaagaccgaggccaactgggtgaacgtgatcagcgacctgaagaagatcgaggacctgatccagagcatgcacatcgacgccaccctgtacaccgagagcgacgtgcaccccagctgcaaggtgaccgccatgaagtgctttctgctggaactgcaggtgatcagcctggaaagcggcgacgccagcatccacgacaccgtggagaacctgatcatcctggccaacaacagcctgagcagcaacggcaacgtgaccgagagcggctgcaaagagtgcgaggaactggaagagaagaacatcaaagagtttctgcagagcttcgtgcacatcgtgcagatgttcatcaacaccagctgacgcgtcatcatcgatccggattagtccaatttgttaaagacaggatatcagtggtccaggctctagttttgactcaacaatatcaccagctgaagcctatagagtacgagccatagataaaataaaagattttatttagtctccagaaaaaggggggaatgaaagaccccacctgtaggtttggcaagctagcttaagtaacgccattttgcaaggcatggaaaaatacataactgagaatagagaagttcagatcaaggtcaggaacagatggaacagctgaatatgggccaaacaggatatctgtggtaagcagttcctgccccggctcagggccaagaacagatggaacagctgaatatgggccaaacaggatatctgtggtaagcagttcctgccccggctcagggccaagaacagatggtccccagatgcggtccagccctcagcagtttctagagaaccatcagatgtttccagggtgccccaaggacctgaaatgaccctgtgccttatttgaactaaccaatcagttcgcttctcgcttctgttcgcgcgcttctgctccccgagctcaataaaagagcccacaacccctcactcggggcgccagtcctccgattgactgagtcgcccgggtacccgtgtatccaataaaccctcttgcagttgcatccgacttgtggtctcgctgttccttgggagggtctcctctgagtgattgactacccgtcagcgggggtctttcacacatgcagcatgtatcaaaattaatttggttttttttcttaagtatttacattaaatggccatagtacttaaagttacattggcttccttgaaataaacatggagtattcagaatgtgtcataaatatttctaattttaagatagtatctccattggctttctactttttcttttatttttttttgtcctctgtcttccatttgttgttgttgttgtttgtttgtttgtttgttggttggttggttaatttttttttaaagatcctacactatagttcaagctagactattagctactctgtaacccagggtgaccttgaagtcatgggtagcctgctgttttagccttcccacatctaagattacaggtatgagctatcatttttggtatattgattgattgattgattgatgtgtgtgtgtgtgattgtgtttgtgtgtgtgactgtgaaaatgtgtgtatgggtgtgtgtgaatgtgtgtatgtatgtgtgtgtgtgagtgtgtgtgtgtgtgtgtgcatgtgtgtgtgtgtgactgtgtctatgtgtatgactgtgtgtgtgtgtgtgtgtgtgtgtgtgtgtgtgtgtgtgtgtgtgttgtgaaaaaatattctatggtagtgagagccaacgctccggctcaggtgtcaggttggtttttgagacagagtctttcacttagcttggaattcactggccgtcgttttacaacgtcgtgactgggaaaaccctggcgttacccaacttaatcgccttgcagcacatccccctttcgccagctggcgtaatagcgaagaggcccgcaccgatcgcccttcccaacagttgcgcagcctgaatggcgaatggcgcctgatgcggtattttctccttacgcatctgtgcggtatttcacaccgcatatggtgcactctcagtacaatctgctctgatgccgcatagttaagccagccccgacacccgccaacacccgctgacgcgccctgacgggcttgtctgctcccggcatccgcttacagacaagctgtgaccgtctccgggagctgcatgtgtcagaggttttcaccgtcatcaccgaaacgcgcgagacgaaagggcctcgtgatacgcctatttttataggttaatgtcatgataataatggtttcttagacgtcaggtggcacttttcggggaaatgtgcgcggaacccctatttgtttatttttctaaatacattcaaatatgtatccgctcatgagacaataaccctgataaatgcttcaataatattgaaaaaggaagagtatgagtattcaacatttccgtgtcgcccttattcccttttttgcggcattttgccttcctgtttttgctcacccagaaacgctggtgaaagtaaaagatgctgaagatcagttgggtgcacgagtgggttacatcgaactggatctcaacagcggtaagatccttgagagttttcgccccgaagaacgttttccaatgatgagcacttttaaagttctgctatgtggcgcggtattatcccgtattgacgccgggcaagagcaactcggtcgccgcatacactattctcagaatgacttggttgagtactcaccagtcacagaaaagcatcttacggatggcatgacagtaagagaattatgcagtgctgccataaccatgagtgataacactgcggccaacttacttctgacaacgatcggaggaccgaaggagctaaccgcttttttgcacaacatgggggatcatgtaactcgccttgatcgttgggaaccggagctgaatgaagccataccaaacgacgagcgtgacaccacgatgcctgtagcaatggcaacaacgttgcgcaaactattaactggcgaactacttactctagcttcccggcaacaattaatagactggatggaggcggataaagttgcaggaccacttctgcgctcggcccttccggctggctggtttattgctgataaatctggagccggtgagcgtgggtctcgcggtatcattgcagcactggggccagatggtaagccctcccgtatcgtagttatctacacgacggggagtcaggcaactatggatgaacgaaatagacagatcgctgagataggtgcctcactgattaagcattggtaactgtcagaccaagtttactcatatatactttagattgatttaaaacttcatttttaatttaaaaggatctaggtgaagatcctttttgataatctcatgaccaaaatcccttaacgtgagttttcgttccactgagcgtcagaccccgtagaaaagatcaaaggatcttcttgagatcctttttttctgcgcgtaatctgctgcttgcaaacaaaaaaaccaccgctaccagcggtggtttgtttgccggatcaagagctaccaactctttttccgaaggtaactggcttcagcagagcgcagataccaaatactgttcttctagtgtagccgtagttaggccaccacttcaagaactctgtagcaccgcctacatacctcgctctgctaatcctgttaccagtggctgctgccagtggcgataagtcgtgtcttaccgggttggactcaagacgatagttaccggataaggcgcagcggtcgggctgaacggggggttcgtgcacacagcccagcttggagcgaacgacctacaccgaactgagatacctacagcgtgagctatgagaaagcgccacgcttcccgaagggagaaaggcggacaggtatccggtaagcggcagggtcggaacaggagagcgcacgagggagcttccagggggaaacgcctggtatctttatagtcctgtcgggtttcgccacctctgacttgagcgtcgatttttgtgatgctcgtcaggggggcggagcctatggaaaaacgccagcaacgcggcctttttacggttcctggccttttgctggccttttgctcacatgttctttcctgcgttatcccctgattctgtggataaccgtattaccgcctttgagtgagctgataccgctcgccgcagccgaacgaccgagcgcagcgagtcagtgagcgaggaagcggaagagcgcccaatacgcaaaccgcctctccccgcgcgttggccgattcattaatgcagctggcacgacaggtttcccgactggaaagcgggcagtgagcgcaacgcaattaatgtgagttagctcactcattaggcaccccaggctttacactttatgcttccggctcgtatgttgtgtggaattgtgagcggataacaatttcacacaggaaacagctatgaccatgattacgccaagctttgctcttaggagtttcctaatacatcccaaactcaaatatataaagcatttgacttgttctatgccctagggggcggggggaagctaagccagctttttttaacatttaaaatgttaattccattttaaatgcacagatgtttttatttcataagggtttcaatgtgcatgaatgctgcaatattcctgttaccaaagctagtataaataaaaatagataaacgtggaaattacttagagtttctgtcattaacgtttccttcctcagttgacaacataaatgcgctgctgagcaagccagtttgcatctgtcaggatcaatttcccattatgccagtcatattaattactagtcaattagttgatttttatttttgacatatacatgtg

SEQ ID NO: 49 - DNA, 9374 bp, synthetic construct
  misc_feature 1..9374: note = pSFG4-CD19-DAP12-Ev3-CAR 2.0
  source 1..9374: mol_type = other DNA
aatgaaagaccccacctgtaggtttggcaagctagcttaagtaacgccattttgcaaggcatggaaaaatacataactgagaatagaaaagttcagatcaaggtcaggaacagatggaacagctgaatatgggccaaacaggatatctgtggtaagcagttcctgccccggctcagggccaagaacagatggaacagctgaatatgggccaaacaggatatctgtggtaagcagttcctgccccggctcagggccaagaacagatggtccccagatgcggtccagccctcagcagtttctagagaaccatcagatgtttccagggtgccccaaggacctgaaatgaccctgtgccttatttgaactaaccaatcagttcgcttctcgcttctgttcgcgcgcttatgctccccgagctcaataaaagagcccacaacccctcactcggggcgccagtcctccgattgactgagtcgcccgggtacccgtgtatccaataaaccctcttgcagttgcatccgacttgtggtctcgctgttccttgggagggtctcctctgagtgattgactacccgtcagcgggggtctttcatttgggggctcgtccgggatcgggagacccctgcccagggaccaccgacccaccaccgggaggtaagctggccagcaacttatctgtgtctgtccgattgtctagtgtctatgactgattttatgcgcctgcgtcggtactagttagctaactagctctgtatctggcggacccgtggtggaactgacgagttcggaacacccggccgcaaccctgggagacgtcccagggacttcgggggccgtttttgtggcccgacctgagtcctaaaatcccgatcgtttaggactctttggtgcaccccccttagaggagggatatgtggttctggtaggagacgagaacctaaaacagttcccgcctccgtctgaatttttgctttcggtttgggaccgaagccgcgccgcgcgtcttgtctgctgcagcatcgttctgtgttgtctctgtctgactgtgtttctgtatttgtctgaaaatatgggcccgggctagcctgttaccactcccttaagtttgaccttaggtcactggaaagatgtcgagcggatcgctcacaaccagtcggtagatgtcaagaagagacgttgggttaccttctgctctgcagaatggccaacctttaacgtcggatggccgcgagacggcacctttaaccgagacctcatcacccaggttaagatcaaggtcttttcacctggcccgcatggacacccagaccaggtggggtacatcgtgacctgggaagccttggcttttgacccccctccctgggtcaagccctttgtacaccctaagcctccgcctcctcttcctccatccgccccgtctctcccccttgaacctcctcgttcgaccccgcctcgatcctccctttatccagccctcactccttctctaggcgcccccatatggccatatgagatcttatatggggcacccccgccccttgtaaacttccctgaccctgacatgacaagagttactaacagcccctctctccaagctcacttacaggctctctacttagtccagcacgaagtctggagacctctggcggcagcctaccaagaacaactggaccgaccggtggtacctcacccttaccgagtcggcgacacagtgtgggtccgccgacaccagactaagaacctagaacctcgctggaaaggaccttacacagtcctgctgaccacccccaccgccctcaaagtagacggcatcgcagcttggatacacgccgcccacgtgaaggctgccgaccccgggggtggaccatcctctagactgccatggagtttgggctgagctggctttttcttgtggctattttaaaaggtgtccagtgctctagagacatccagatgacacagactacatcctccctgtctgcctctctgggagacagagtcaccatcagttgcagggcaagtcaggacattagtaaatatttaaattggtatcagcagaaaccagatggaactgttaaactcctgatctaccatacatcaagattacactcaggagtcccatcaaggttcagtggcagtgggtctggaacagattattctctcaccattagcaacctggagcaagaagatattgccacttacttttgccaacagggtaatacgcttccgtacacgttcggaggggggaccaagctggagctgaaacgtggtggtggtggttctggtggtggtggttctggcggcggcggctccggtggtggtggatccgaggtgcagctgcagcagtctggacctggcctggtggcgccctcacagagcctgtccgtcacatgcactgtctcaggggtctcattacccgactatggtgtaagctggattcgccagcctccacgaaagggtctggagtggctgggagtaatatggggtagtgaaaccacatactataattcagctctcaaatccagactgaccatcatcaaggacaactccaagagccaagttttcttaaaaatgaacagtctgcaaactgatgacacagccatttactactgtgccaaacattattactacggtggtagctatgctatggactactggggccaagggaccacggtcaccgtctcctcgtacgtcaccgtctcttcacaggatcccgccctggaagagaagaaaggcaattacgtcgtgaccgaccacggcagctgtgtgcgggcttgtggcgccgatagctacgagatggaagaggacggcgtgcggaagtgcaagaagtgcgagggcccctgcagaaaagtgtgcaacggcatcggcatcggagagttcaaggatagcctgagcatcaacgccaccaacatcaagcacttcaagaactgcaccagcatcagcggcgacctgcacatcctgcccgtggcctttagaggcgacagcttcacccacacccccccactggatccccaggaactggacatcctgaaaaccgtgaaagagatcacaggctttctgctgattcaggcctggcccgagaaccggacagacctgcacgccttcgagaacctggaaatcatcagaggccggaccaagcagcacggccagttttctctggccgtggtgtccctgaacatcaccagcctgggcctgcggagcctgaaagaaatcagcgacggcgacgtgatcatctccggcaacaagaacctgtgctacgccaacaccatcaattggaagaagctgttcggcacctccggccagaaaacaaagatcatctctaaccggggcgagaacagctgcaaagccaccggacaagtgtgccacgccctgtgtagccctgagggctgttggggacccgagcccagagattgcgtgtcctgccggaatgtgtccagaggccgcgagtgcgtggacaagtgcaacctgctggaaggcgagccccgcgagtttgtggaaaacagcgagtgcatccagtgccaccccgagtgtctgccccaggccatgaacattacctgcaccggcagaggccccgacaactgtatccagtgcgcccactacatcgacggcccccactgcgtgaaaacctgtccagctggcgtgatgggagagaacaacaccctcgtgtggaagtacgccgacgccggccatgtgtgccacctgtgtcaccccaattgcacctacggctgtaccggccctggcctggaaggctgtcctaccaacggccccaagatccctagcaaggatcctaagggagtgctggccggaatcgtgatgggcgacctggtgctgacagtgctgatcgccctggctgtgtacttcctgggcagactggtgcccagaggaagaggcgctgccgaagccgccacccggaagcagagaatcaccgagacagagagcccctatcaggaactgcagggccagcggagcgacgtgtacagcgacctgaatacccagcggccctactacaagagagtgaagttcagcaggagcgcagacgcccccgcgtaccagcagggccagaaccagctctataacgagctcaatctaggacgaagagaggagtacgatgttttggacaagagacgtggccgggaccctgagatggggggaaagccgagaaggaagaaccctcaggaaggcctgtacaatgaactgcagaaagataagatggcggaggcctacagtgagattgggatgaaaggcgagcgccggaggggcaaggggcacgatggcctttaccagggtctcagtacagccaccaaggacacctacgacgcccttcacatgcaggccctgccccctcgcggaccgcagtgtactaattatgctctcttgaaattggctggagatgttgagagcaatcccgggcccatgcggatcagcaagccccacctgcggagcatcagcatccagtgctacctgtgcctgctgctgaacagccacttcctgaccgaggccggcatccacgtgttcatcctgggctgcttcagcgccggactgcccaagaccgaggccaactgggtgaacgtgatcagcgacctgaagaagatcgaggacctgatccagagcatgcacatcgacgccaccctgtacaccgagagcgacgtgcaccccagctgcaaggtgaccgccatgaagtgctttctgctggaactgcaggtgatcagcctggaaagcggcgacgccagcatccacgacaccgtggagaacctgatcatcctggccaacaacagcctgagcagcaacggcaacgtgaccgagagcggctgcaaagagtgcgaggaactggaagagaagaacatcaaagagtttctgcagagcttcgtgcacatcgtgcagatgttcatcaacaccagctgacgcgtcatcatcgatccggattagtccaatttgttaaagacaggatatcagtggtccaggctctagttttgactcaacaatatcaccagctgaagcctatagagtacgagccatagataaaataaaagattttatttagtctccagaaaaaggggggaatgaaagaccccacctgtaggtttggcaagctagcttaagtaacgccattttgcaaggcatggaaaaatacataactgagaatagagaagttcagatcaaggtcaggaacagatggaacagctgaatatgggccaaacaggatatctgtggtaagcagttcctgccccggctcagggccaagaacagatggaacagctgaatatgggccaaacaggatatctgtggtaagcagttcctgccccggctcagggccaagaacagatggtccccagatgcggtccagccctcagcagtttctagagaaccatcagatgtttccagggtgccccaaggacctgaaatgaccctgtgccttatttgaactaaccaatcagttcgcttctcgcttctgttcgcgcgcttctgctccccgagctcaataaaagagcccacaacccctcactcggggcgccagtcctccgattgactgagtcgcccgggtacccgtgtatccaataaaccctcttgcagttgcatccgacttgtggtctcgctgttccttgggagggtctcctctgagtgattgactacccgtcagcgggggtctttcacacatgcagcatgtatcaaaattaatttggttttttttcttaagtatttacattaaatggccatagtacttaaagttacattggcttccttgaaataaacatggagtattcagaatgtgtcataaatatttctaattttaagatagtatctccattggctttctactttttcttttatttttttttgtcctctgtcttccatttgttgttgttgttgtttgtttgtttgtttgttggttggttggttaatttttttttaaagatcctacactatagttcaagctagactattagctactctgtaacccagggtgaccttgaagtcatgggtagcctgctgttttagccttcccacatctaagattacaggtatgagctatcatttttggtatattgattgattgattgattgatgtgtgtgtgtgtgattgtgtttgtgtgtgtgactgtgaaaatgtgtgtatgggtgtgtgtgaatgtgtgtatgtatgtgtgtgtgtgagtgtgtgtgtgtgtgtgtgcatgtgtgtgtgtgtgactgtgtctatgtgtatgactgtgtgtgtgtgtgtgtgtgtgtgtgtgtgtgtgtgtgtgtgtgtgttgtgaaaaaatattctatggtagtgagagccaacgctccggctcaggtgtcaggttggtttttgagacagagtctttcacttagcttggaattcactggccgtcgttttacaacgtcgtgactgggaaaaccctggcgttacccaacttaatcgccttgcagcacatccccctttcgccagctggcgtaatagcgaagaggcccgcaccgatcgcccttcccaacagttgcgcagcctgaatggcgaatggcgcctgatgcggtattttctccttacgcatctgtgcggtatttcacaccgcatatggtgcactctcagtacaatctgctctgatgccgcatagttaagccagccccgacacccgccaacacccgctgacgcgccctgacgggcttgtctgctcccggcatccgcttacagacaagctgtgaccgtctccgggagctgcatgtgtcagaggttttcaccgtcatcaccgaaacgcgcgagacgaaagggcctcgtgatacgcctatttttataggttaatgtcatgataataatggtttcttagacgtcaggtggcacttttcggggaaatgtgcgcggaacccctatttgtttatttttctaaatacattcaaatatgtatccgctcatgagacaataaccctgataaatgcttcaataatattgaaaaaggaagagtatgagtattcaacatttccgtgtcgcccttattcccttttttgcggcattttgccttcctgtttttgctcacccagaaacgctggtgaaagtaaaagatgctgaagatcagttgggtgcacgagtgggttacatcgaactggatctcaacagcggtaagatccttgagagttttcgccccgaagaacgttttccaatgatgagcacttttaaagttctgctatgtggcgcggtattatcccgtattgacgccgggcaagagcaactcggtcgccgcatacactattctcagaatgacttggttgagtactcaccagtcacagaaaagcatcttacggatggcatgacagtaagagaattatgcagtgctgccataaccatgagtgataacactgcggccaacttacttctgacaacgatcggaggaccgaaggagctaaccgcttttttgcacaacatgggggatcatgtaactcgccttgatcgttgggaaccggagctgaatgaagccataccaaacgacgagcgtgacaccacgatgcctgtagcaatggcaacaacgttgcgcaaactattaactggcgaactacttactctagcttcccggcaacaattaatagactggatggaggcggataaagttgcaggaccacttctgcgctcggcccttccggctggctggtttattgctgataaatctggagccggtgagcgtgggtctcgcggtatcattgcagcactggggccagatggtaagccctcccgtatcgtagttatctacacgacggggagtcaggcaactatggatgaacgaaatagacagatcgctgagataggtgcctcactgattaagcattggtaactgtcagaccaagtttactcatatatactttagattgatttaaaacttcatttttaatttaaaaggatctaggtgaagatcctttttgataatctcatgaccaaaatcccttaacgtgagttttcgttccactgagcgtcagaccccgtagaaaagatcaaaggatcttcttgagatcctttttttctgcgcgtaatctgctgcttgcaaacaaaaaaaccaccgctaccagcggtggtttgtttgccggatcaagagctaccaactctttttccgaaggtaactggcttcagcagagcgcagataccaaatactgttcttctagtgtagccgtagttaggccaccacttcaagaactctgtagcaccgcctacatacctcgctctgctaatcctgttaccagtggctgctgccagtggcgataagtcgtgtcttaccgggttggactcaagacgatagttaccggataaggcgcagcggtcgggctgaacggggggttcgtgcacacagcccagcttggagcgaacgacctacaccgaactgagatacctacagcgtgagctatgagaaagcgccacgcttcccgaagggagaaaggcggacaggtatccggtaagcggcagggtcggaacaggagagcgcacgagggagcttccagggggaaacgcctggtatctttatagtcctgtcgggtttcgccacctctgacttgagcgtcgatttttgtgatgctcgtcaggggggcggagcctatggaaaaacgccagcaacgcggcctttttacggttcctggccttttgctggccttttgctcacatgttctttcctgcgttatcccctgattctgtggataaccgtattaccgcctttgagtgagctgataccgctcgccgcagccgaacgaccgagcgcagcgagtcagtgagcgaggaagcggaagagcgcccaatacgcaaaccgcctctccccgcgcgttggccgattcattaatgcagctggcacgacaggtttcccgactggaaagcgggcagtgagcgcaacgcaattaatgtgagttagctcactcattaggcaccccaggctttacactttatgcttccggctcgtatgttgtgtggaattgtgagcggataacaatttcacacaggaaacagctatgaccatgattacgccaagctttgctcttaggagtttcctaatacatcccaaactcaaatatataaagcatttgacttgttctatgccctagggggcggggggaagctaagccagctttttttaacatttaaaatgttaattccattttaaatgcacagatgtttttatttcataagggtttcaatgtgcatgaatgctgcaatattcctgttaccaaagctagtataaataaaaatagataaacgtggaaattacttagagtttctgtcattaacgtttccttcctcagttgacaacataaatgcgctgctgagcaagccagtttgcatctgtcaggatcaatttcccattatgccagtcatattaattactagtcaattagttgatttttatttttgacatatacatgtg

SEQ ID NO: 50 - protein, 1006 aa, synthetic construct
  REGION 1..1006: note = pSFG4-CD19-DAP12-Ev3-CAR 2.0
MEFGLSWLFLVAILKGVQCSRDIQMTQTTSSLSASLGDRVTISCRASQDISKYLNWYQQKPDGTVKLLIYHTSRLHSGVPSRFSGSGSGTDYSLTISNLEQEDIATYFCQQGNTLPYTFGGGTKLELKRGGGGSGGGGSGGGGSGGGGSEVQLQQSGPGLVAPSQSLSVTCTVSGVSLPDYGVSWIRQPPRKGLEWLGVIWGSETTYYNSALKSRLTIIKDNSKSQVFLKMNSLQTDDTAIYYCAKHYYYGGSYAMDYWGQGTTVTVSSYVTVSSQDPALEEKKGNYVVTDHGSCVRACGADSYEMEEDGVRKCKKCEGPCRKVCNGIGIGEFKDSLSINATNIKHFKNCTSISGDLHILPVAFRGDSFTHTPPLDPQELDILKTVKEITGFLLIQAWPENRTDLHAFENLEIIRGRTKQHGQFSLAVVSLNITSLGLRSLKEISDGDVIISGNKNLCYANTINWKKLFGTSGQKTKIISNRGENSCKATGQVCHALCSPEGCWGPEPRDCVSCRNVSRGRECVDKCNLLEGEPREFVENSECIQCHPECLPQAMNITCTGRGPDNCIQCAHYIDGPHCVKTCPAGVMGENNTLVWKYADAGHVCHLCHPNCTYGCTGPGLEGCPTNGPKIPSKDPKGVLAGIVMGDLVLTVLIALAVYFLGRLVPRGRGAAEAATRKQRITETESPYQELQGQRSDVYSDLNTQRPYYKRVKFSRSADAPAYQQGQNQLYNELNLGRREEYDVLDKRRGRDPEMGGKPRRKNPQEGLYNELQKDKMAEAYSEIGMKGERRRGKGHDGLYQGLSTATKDTYDALHMQALPPRGPQCTNYALLKLAGDVESNPGPMRISKPHLRSISIQCYLCLLLNSHFLTEAGIHVFILGCFSAGLPKTEANWVNVISDLKKIEDLIQSMHIDATLYTESDVHPSCKVTAMKCFLLELQVISLESGDASIHDTVENLIILANNSLSSNGNVTESGCKECEELEEKNIKEFLQSFVHIVQMFINTS

SEQ ID NO: 51 - DNA, 219 bp, synthetic construct
  misc_feature 1..219: note = DAP12
  source 1..219: mol_type = other DNA
ggcgtgctggccggaatcgtgatgggcgacctggtgctgacagtgctgatcgccctggctgtgtacttcctgggcagactggtgcccagaggaagaggcgctgccgaagccgccacccggaagcagagaatcaccgagacagagagcccctatcaggaactgcagggccagcggagcgacgtgtacagcgacctgaatacccagcggccctactacaag

SEQ ID NO: 52 - protein, 73 aa, synthetic construct
  REGION 1..73: note = DAP12
GVLAGIVMGDLVLTVLIALAVYFLGRLVPRGRGAAEAATRKQRITETESPYQELQGQRSDVYSDLNTQRPYYK

SEQ ID NO: 53 - DNA, 342 bp, synthetic construct
  misc_feature 1..342: note = CD3zeta
  source 1..342: mol_type = other DNA
agagtgaagttcagcaggagcgcagacgcccccgcgtaccagcagggccagaaccagctctataacgagctcaatctaggacgaagagaggagtacgatgttttggacaagagacgtggccgggaccctgagatggggggaaagccgagaaggaagaaccctcaggaaggcctgtacaatgaactgcagaaagataagatggcggaggcctacagtgagattgggatgaaaggcgagcgccggaggggcaaggggcacgatggcctttaccagggtctcagtacagccaccaaggacacctacgacgcccttcacatgcaggccctgccccctcgcggaccg

SEQ ID NO: 54 - protein, 114 aa, synthetic construct
  REGION 1..114: note = CD3zeta
RVKFSRSADAPAYQQGQNQLYNELNLGRREEYDVLDKRRGRDPEMGGKPRRKNPQEGLYNELQKDKMAEAYSEIGMKGERRRGKGHDGLYQGLSTATKDTYDALHMQALPPRGP

SEQ ID NO: 55 - DNA, 489 bp, synthetic construct
  misc_feature 1..489: note = IL15
  source 1..489: mol_type = other DNA
atgcggatcagcaagccccacctgcggagcatcagcatccagtgctacctgtgcctgctgctgaacagccacttcctgaccgaggccggcatccacgtgttcatcctgggctgcttcagcgccggactgcccaagaccgaggccaactgggtgaacgtgatcagcgacctgaagaagatcgaggacctgatccagagcatgcacatcgacgccaccctgtacaccgagagcgacgtgcaccccagctgcaaggtgaccgccatgaagtgctttctgctggaactgcaggtgatcagcctggaaagcggcgacgccagcatccacgacaccgtggagaacctgatcatcctggccaacaacagcctgagcagcaacggcaacgtgaccgagagcggctgcaaagagtgcgaggaactggaagagaagaacatcaaagagtttctgcagagcttcgtgcacatcgtgcagatgttcatcaacaccagctga

SEQ ID NO: 56 - protein, 162 aa, synthetic construct
  REGION 1..162: note = IL15
MRISKPHLRSISIQCYLCLLLNSHFLTEAGIHVFILGCFSAGLPKTEANWVNVISDLKKIEDLIQSMHIDATLYTESDVHPSCKVTAMKCFLLELQVISLESGDASIHDTVENLIILANNSLSSNGNVTESGCKECEELEEKNIKEFLQSFVHIVQMFINTS

SEQ ID NO: 57 - DNA, 819 bp, synthetic construct
  misc_feature 1..819: note = hCLL-1 scFv
  source 1..819: mol_type = other DNA
atggagtttgggctgagctggctttttcttgtggctattttaaaaggtgtccagtgctcgcgagacatccagatgacccagagccccagcagcctgagcgccagcgtgggcgacagagtgaccatcacctgcagagccagcagcaacgtgatcagcagctacgtgcactggtaccagcagaagcccggcaaggcccccaagctgctgatctacagcaccagcaacctggccagcggcgtgcccagcagattcagcggcagcagaagcggcaccgacttcaccctgaccatcagcagcctgcagcccgaggacttcgccacctactactgccagcagtacagcggctaccccctgaccttcggccagggcaccaaggtggagatcaagagaggtggtggtggttctggtggtggtggttctggcggcggcggctccggtggtggtggatccgaggtgcagctggtggagagcggcggcggcctggtgcagcccggcggcagcctgagactgagctgcgccgccagcggctacagcatcaccagcgcctactactggaactgggtgagacaggcccccggcaagggcctggagtgggtggcctacatcagctacgacggcagaaacaactacaaccccagcctgaagaacagattcaccatcagcgccgacaccagcaagaacaccgcctacctgcagatgaacagcctgagagccgaggacaccgccgtgtactactgcagcagagagggcgactacgacgtgggcaactactacgccatggactactggggccagggcaccctggtgaccgtgagctcg

SEQ ID NO: 58 - protein, 273 aa, synthetic construct
  REGION 1..273: note = hCLL-1 scFv
MEFGLSWLFLVAILKGVQCSRDIQMTQSPSSLSASVGDRVTITCRASSNVISSYVHWYQQKPGKAPKLLIYSTSNLASGVPSRFSGSRSGTDFTLTISSLQPEDFATYYCQQYSGYPLTFGQGTKVEIKRGGGGSGGGGSGGGGSGGGGSEVQLVESGGGLVQPGGSLRLSCAASGYSITSAYYWNWVRQAPGKGLEWVAYISYDGRNNYNPSLKNRFTISADTSKNTAYLQMNSLRAEDTAVYYCSREGDYDVGNYYAMDYWGQGTLVTVSS

SEQ ID NO: 59 - protein, 109 aa, synthetic construct
  REGION 1..109: note = hCLL1 VH
DIQMTQSPSSLSASVGDRVTITCRASSNVISSYVHWYQQKPGKAPKLLIYSTSNLASGVPSRFSGSRSGTDFTLTISSLQPEDFATYYCQQYSGYPLTFGQGTKVEIKR

SEQ ID NO: 60 - protein, 123 aa, synthetic construct
  REGION 1..123: note = hCLL1 VL
EVQLVESGGGLVQPGGSLRLSCAASGYSITSAYYWNWVRQAPGKGLEWVAYISYDGRNNYNPSLKNRFTISADTSKNTAYLQMNSLRAEDTAVYYCSREGDYDVGNYYAMDYWGQGTLVTVSS

SEQ ID NO: 61 - DNA, 804 bp, synthetic construct
  misc_feature 1..804: note = CD99 scFv
  source 1..804: mol_type = other DNA
atggagtttgggctgagctggctttttcttgtggctattttaaaaggtgtccagtgctctagaagcagcgagctgacccaggaccccgccgtgagcgtggccctgggccagaccgtgagaatcacctgccagggcgacagcctgagaagctactacgccagctggtaccagcagaagcccggccaggcccccgtgctggtgatctacggcaagaacaacagacccagcggcatccccgacagattcagcggcagcagcagcggcaacaccgccagcctgaccatcaccggcgcccaggccgaggacgaggccgactactactgcaacagcagcttccccagaaccagcagcgtggtgttcggcggcggcaccaagctgaccgtgctgggcggtggtggtggttctggtggtggtggttctggcggcggcggctccggtggtggtggatccatggccgaggtgcagctggtggagagcggcggcggcctggtgagacccggcggcagcctgagactgagctgcgccgccagcggcttcaccttcagcagctacgccatgagctgggtgagacaggcccccggcaagggcctggagtgggtgagcgccatcagcggcagcggcggcagcacctactacgccgacagcgtgaagggcagattcaccatcagcagagacaacagcaagaacaccctgtacctgcagatgaacagcctgagagccgaggacaccgccgtgtactactgcgccaagagccacaagagattcgactactggggccagggcaccctggtgaccgtgagcaga

SEQ ID NO: 62 - protein, 268 aa, synthetic construct
  REGION 1..268: note = CD99 scFv
MEFGLSWLFLVAILKGVQCSRSSELTQDPAVSVALGQTVRITCQGDSLRSYYASWYQQKPGQAPVLVIYGKNNRPSGIPDRFSGSSSGNTASLTITGAQAEDEADYYCNSSFPRTSSVVFGGGTKLTVLGGGGGSGGGGSGGGGSGGGGSMAEVQLVESGGGLVRPGGSLRLSCAASGFTFSSYAMSWVRQAPGKGLEWVSAISGSGGSTYYADSVKGRFTISRDNSKNTLYLQMNSLRAEDTAVYYCAKSHKRFDYWGQGTLVTVSR

SEQ ID NO: 63 - protein, 108 aa, synthetic construct
  REGION 1..108: note = CD99 VH
SSELTQDPAVSVALGQTVRITCQGDSLRSYYASWYQQKPGQAPVLVIYGKNNRPSGIPDRFSGSSSGNTASLTITGAQAEDEADYYCNSSFPRTSSVVFGGGTKLTVL

SEQ ID NO: 64 - protein, 118 aa, synthetic construct
  REGION 1..118: note = CD99 VL
MAEVQLVESGGGLVRPGGSLRLSCAASGFTFSSYAMSWVRQAPGKGLEWVSAISGSGGSTYYADSVKGRFTISRDNSKNTLYLQMNSLRAEDTAVYYCAKSHKRFDYWGQGTLVTVSR